European Patent Specification EP 3 882 272 B1, published November 6, 2024. Title: Antibody specifically binding to the N-terminal region of lysyl- tRNA synthetase exposed at cell outer membrane. Applicant: Medicinal Bioconvergence Research Center. The sequence listing filed with the application follows.

SEQUENCE LISTING (251 sequences)

SEQ ID NO: 1 - protein, 5 aa, Artificial Sequence
  CDR H1 amino acid
SYDMS

SEQ ID NO: 2 - DNA, 15 bp, Artificial Sequence
  CDR H1 DNA
agttatgatatgagc

SEQ ID NO: 3 - protein, 17 aa, Artificial Sequence
  CDR H2 amino acid
AISYDNGNTYYADSVKG

SEQ ID NO: 4 - DNA, 51 bp, Artificial Sequence
  CDR H2 DNA
gcgatctcttatgataatggtaatacatattacgctgattctgtaaaaggt

SEQ ID NO: 5 - protein, 7 aa, Artificial Sequence
  CDR H3 amino acid
MALDFDY

SEQ ID NO: 6 - DNA, 21 bp, Artificial Sequence
  CDR H3 DNA
atggcgcttgatttcgactac

SEQ ID NO: 7 - protein, 13 aa, Artificial Sequence
  CDR L1 amino acid
TGSSSNIGSNYVT

SEQ ID NO: 8 - DNA, 39 bp, Artificial Sequence
  CDR L1 DNA
actggctcttcatctaatattggcagtaattatgtcacc

SEQ ID NO: 9 - protein, 7 aa, Artificial Sequence
  CDR L2 amino acid
DNSNRPS

SEQ ID NO: 10 - DNA, 21 bp, Artificial Sequence
  CDR L2 DNA
gataatagtaatcggccaagc

SEQ ID NO: 11 - protein, 11 aa, Artificial Sequence
  CDR L3 amino acid
ASWDDSLSAYV

SEQ ID NO: 12 - DNA, 33 bp, Artificial Sequence
  CDR L3 DNA
gcttcttgggatgatagcctgagtgcttatgtc

SEQ ID NO: 13 - protein, 11 aa, Artificial Sequence
  CDR L3 mutant 1 amino acid
ASFSDELGAYV

SEQ ID NO: 14 - DNA, 33 bp, Artificial Sequence
  CDR L3 mutant 1 DNA
gcttcttttagtgatgagttgggggcttatgtc

SEQ ID NO: 15 - protein, 11 aa, Artificial Sequence
  CDR L3 mutant 2 amino acid
SSFSDELGAYV

SEQ ID NO: 16 - DNA, 33 bp, Artificial Sequence
  CDR L3 mutant 2 DNA
tcttcttttagtgatgagttgggggcttatgtc

SEQ ID NO: 17 - protein, 17 aa, Artificial Sequence
  CDR H2 mutant 1 amino acid
AISPQMGRVYYADSVKG

SEQ ID NO: 18 - DNA, 51 bp, Artificial Sequence
  CDR H2 mutant 1 DNA
gcgatctcgccgcagatgggtcgggtgtattacgctgattctgtaaaaggt

SEQ ID NO: 19 - protein, 17 aa, Artificial Sequence
  CDR H2 mutant 2 amino acid
AIDPLGGNIYYADSVKG

SEQ ID NO: 20 - DNA, 51 bp, Artificial Sequence
  CDR H2 mutant 2 DNA
gcgatcgatccgttggggggtaatatttattacgctgattctgtaaaaggt

SEQ ID NO: 21 - protein, 17 aa, Artificial Sequence
  CDR H2 mutant 3 amino acid
AISPYSGRIYYADSVKG

SEQ ID NO: 22 - DNA, 51 bp, Artificial Sequence
  CDR H2 mutant 3 DNA
gcgatctctccgtattcgggtaggatttattacgctgattctgtaaaaggt

SEQ ID NO: 23 - protein, 17 aa, Artificial Sequence
  CDR H2 mutant 4 amino acid
AIGADGGPSYYADSVKG

SEQ ID NO: 24 - DNA, 51 bp, Artificial Sequence
  CDR H2 mutant 4 DNA
gcgatcggggctgatgggggtccgtcttattacgctgattctgtaaaaggt

SEQ ID NO: 25 - protein, 7 aa, Artificial Sequence
  CDR H3 mutant 1 amino acid
LALDFDY

SEQ ID NO: 26 - DNA, 21 bp, Artificial Sequence
  CDR H3 mutant 1 DNA
ctggcgcttgatttcgactac

SEQ ID NO: 27 - protein, 7 aa, Artificial Sequence
  CDR L2 mutant 1 amino acid
SNNQRPS

SEQ ID NO: 28 - DNA, 21 bp, Artificial Sequence
  CDR L2 mutant 1 DNA
agtaataatcagcggccaagc

SEQ ID NO: 29 - protein, 7 aa, Artificial Sequence
  CDR L2 mutant 2 amino acid
RNNQRPS

SEQ ID NO: 30 - DNA, 21 bp, Artificial Sequence
  CDR L2 mutant 2 DNA
cggaataatcagcggccaagc

SEQ ID NO: 31 - protein, 116 aa, Artificial Sequence
  N3 VH
EVQLLESGGGLVQPGGSLRLSCAASGFTFSSYDMSWVRQAPGKGLEWVSAISYDNGNTYYADSVKGRFTISRDNSKNTLYLQMNSLRAEDTAVYYSARMALDFDYWGQGTLVTVSS

SEQ ID NO: 32 - DNA, 348 bp, Artificial Sequence
  N3 VH
gaggtgcagctgttggagtctgggggaggcttggtacagcctggggggtccctgagactctcctgtgcagcctctggattcacctttagcagttatgatatgagctgggtccgccaggctccagggaaggggctggagtgggtctcagcgatctcttatgataatggtaatacatattacgctgattctgtaaaaggtcggttcaccatctccagagacaattccaagaacacgctgtatctgcaaatgaacagcctgagagccgaggacacggccgtgtattactctgcgagaatggcgcttgatttcgactactggggccagggtacactggtcaccgtgagctca

SEQ ID NO: 33 - protein, 110 aa, Artificial Sequence
  N3 VL
QSVLTQPPSASGTPGQRVTISCTGSSSNIGSNYVTWYQQLPGTAPKLLIYDNSNRPSGVPDRFSGSKSGTSASLAISGLRSEDEADYYCASWDDSLSAYVFGGGTKLTVL

SEQ ID NO: 34 - DNA, 330 bp, Artificial Sequence
  N3 VL
cagtctgtgctgactcagccaccctcagcgtctgggacccccgggcagagggtcaccatctcttgtactggctcttcatctaatattggcagtaattatgtcacctggtaccagcagctcccaggaacggcccccaaactcctcatctatgataatagtaatcggccaagcggggtccctgaccgattctctggctccaagtctggcacctcagcctccctggccatcagtgggctccggtccgaggatgaggctgattattactgtgcttcttgggatgatagcctgagtgcttatgtcttcggcggaggcaccaagctgacggtccta

SEQ ID NO: 35 - protein, 116 aa, Artificial Sequence
  N3 VH mutant 1
EVQLLESGGGLVQPGGSLRLSCAASGFTFSSYDMSWVRQAPGKGLEWVSVISSDGGNTYYADSVKGRFTISRDNSKNTLYLQMNSLRAEDTAVYYSARMALDFDYWGQGTLVTVSS

SEQ ID NO: 36 - DNA, 348 bp, Artificial Sequence
  N3 VH mutant 1
gaggtgcagctgttggagtctgggggaggcttggtacagcctggggggtccctgagactctcctgtgcagcctctggattcacctttagcagttatgatatgagctgggtccgccaggctccagggaaggggctggagtgggtctcagtgatctcttctgatggtggtaatacatattacgctgattctgtaaaaggtcggttcaccatctccagagacaattccaagaacacgctgtatctgcaaatgaacagcctgagagccgaggacacggccgtgtattactctgcgagaatggcgcttgatttcgactactggggccagggtacactggtcaccgtgagctca

SEQ ID NO: 37 - protein, 116 aa, Artificial Sequence
  N3 VH mutant 2
EVQLLESGGGLVQPGGSLRLSCAASGFTFSSYDMSWVRQAPGKGLEWVSAISPQMGRVYYADSVKGRFTISRDNSKNTLYLQMNSLRAEDTAVYYCARMALDFDYWGQGTLVTVSS

SEQ ID NO: 38 - DNA, 348 bp, Artificial Sequence
  N3 VH mutant 2
gaggtgcagctgttggagtctgggggaggcttggtacagcctggggggtccctgagactctcctgtgcagcctctggattcacctttagcagttatgatatgagctgggtccgccaggctccagggaaggggctggagtgggtctcagcgatctcgccgcagatgggtcgggtgtattacgctgattctgtaaaaggtcggttcaccatctccagagacaattccaagaacacgctgtatctgcaaatgaacagcctgagagccgaggacacggccgtgtattactgtgcgagaatggcgcttgatttcgactactggggccagggtacactggtcaccgtgagctca

SEQ ID NO: 39 - protein, 116 aa, Artificial Sequence
  N3 VH mutant 3
EVQLLESGGGLVQPGGSLRLSCAASGFTFSSYDMSWVRQAPGKGLEWVSAIDPLGGNIYYADSVKGRFTISRDNSKNTLYLQMNSLRAEDTAVYYCARMALDFDYWGQGTLVTVSS

SEQ ID NO: 40 - DNA, 348 bp, Artificial Sequence
  N3 VH mutant 3
gaggtgcagctgttggagtctgggggaggcttggtacagcctggggggtccctgagactctcctgtgcagcctctggattcacctttagcagttatgatatgagctgggtccgccaggctccagggaaggggctggagtgggtctcagcgatcgatccgttggggggtaatatttattacgctgattctgtaaaaggtcggttcaccatctccagagacaattccaagaacacgctgtatctgcaaatgaacagcctgagagccgaggacacggccgtgtattactgtgcgagaatggcgcttgatttcgactactggggccagggtacactggtcaccgtgagctca

SEQ ID NO: 41 - protein, 116 aa, Artificial Sequence
  N3 VH mutant 4
EVQLLESGGGLVQPGGSLRLSCAASGFTFSSYDMSWVRQAPGKGLEWVSAISPYSGRIYYADSVKGRFTISRDNSKNTLYLQMNSLRAEDTAVYYSARMALDFDYWGQGTLVTVSS

SEQ ID NO: 42 - DNA, 348 bp, Artificial Sequence
  N3 VH mutant 4
gaggtgcagctgttggagtctgggggaggcttggtacagcctggggggtccctgagactctcctgtgcagcctctggattcacctttagcagttatgatatgagctgggtccgccaggctccagggaaggggctggagtgggtctcagcgatctctccgtattcgggtaggatttattacgctgattctgtaaaaggtcggttcaccatctccagagacaattccaagaacacgctgtatctgcaaatgaacagcctgagagccgaggacacggccgtgtattactctgcgagaatggcgcttgatttcgactactggggccagggtacactggtcaccgtgagctca

SEQ ID NO: 43 - protein, 116 aa, Artificial Sequence
  N3 VH mutant 5
EVQLLESGGGLVQPGGSLRLSCAASGFTFSSYDMSWVRQAPGKGLEWVSAIGADGGPSYYADSVKGRFTISRDNSKNTLYLQMNSLRAEDTAVYYCARMALDFDYWGQGTLVTVSS

SEQ ID NO: 44 - DNA, 348 bp, Artificial Sequence
  N3 VH mutant 5
gaggtgcagctgttggagtctgggggaggcttggtacagcctggggggtccctgagactctcctgtgcagcctctggattcacctttagcagttatgatatgagctgggtccgccaggctccagggaaggggctggagtgggtctcagcgatcggggctgatgggggtccgtcttattacgctgattctgtaaaaggtcggttcaccatctccagagacaattccaagaacacgctgtatctgcaaatgaacagcctgagagccgaggacacggccgtgtattactgtgcgagaatggcgcttgatttcgactactggggccagggtacactggtcaccgtgagctca

SEQ ID NO: 45 - protein, 116 aa, Artificial Sequence
  N3 VH mutant 6
EVQLLESGGGLVQPGGSLRLSCAASGFTFSSYDMSWVRQAPGKGLEWVSAISPYSGRIYYADSVKGRFTISRDNSKNTLYLQMNSLRAEDTAVYYCARMALDFDYWGQGTLVTVSS

SEQ ID NO: 46 - DNA, 348 bp, Artificial Sequence
  N3 VH mutant 6
gaggtgcagctgttggagtctgggggaggcttggtacagcctggggggtccctgagactctcctgtgcagcctctggattcacctttagcagttatgatatgagctgggtccgccaggctccagggaaggggctggagtgggtctcagcgatctctccgtattcgggtaggatttattacgctgattctgtaaaaggtcggttcaccatctccagagacaattccaagaacacgctgtatctgcaaatgaacagcctgagagccgaggacacggccgtgtattactgtgcgagaatggcgcttgatttcgactactggggccagggtacactggtcaccgtgagctca

SEQ ID NO: 47 - protein, 116 aa, Artificial Sequence
  N3 VH mutant 7
EVQLLESGGGLVQPGGSLRLSCAASGFTFSSYDMSWVRQAPGKGLEWVSAISPYSGRIYYADSVKGRFTISRDNSKNTLYLQMNSLRAEDTAVYYCARLALDFDYWGQGTLVTVSS

SEQ ID NO: 48 - DNA, 348 bp, Artificial Sequence
  N3 VH mutant 7
gaggtgcagctgttggagtctgggggaggcttggtacagcctggggggtccctgagactctcctgtgcagcctctggattcacctttagcagttatgatatgagctgggtccgccaggctccagggaaggggctggagtgggtctcagcgatctctccgtattcgggtaggatttattacgctgattctgtaaaaggtcggttcaccatctccagagacaattccaagaacacgctgtatctgcaaatgaacagcctgagagccgaggacacggccgtgtattactgtgcgagactggcgcttgatttcgactactggggccagggtacactggtcaccgtgagctca

SEQ ID NO: 49 - protein, 110 aa, Artificial Sequence
  N3 VL mutant 1
QSVLTQPPSASGTPGQRVTISCTGSSSNIGSNYVTWYQQLPGTAPKLLIYDNSNRPSGVPDRFSGSKSGTSASLAISGLQSEDEADYYCASFSDELGAYVFGGGTKLTVL

SEQ ID NO: 50 - DNA, 330 bp, Artificial Sequence
  N3 VL mutant 1
cagtctgtgctgactcagccaccctcagcgtctgggacccccgggcagagggtcaccatctcttgtactggctcttcatctaatattggcagtaattatgtcacctggtaccagcagctcccaggaacggcccccaaactcctcatctatgataatagtaatcggccaagcggggtccctgaccgattctctggctccaagtctggcacctcagcctccctggccatcagtgggctccagtccgaggatgaggctgattattactgtgcttcttttagtgatgagttgggggcttatgtcttcggcggaggcaccaagctgacggtccta

SEQ ID NO: 51 - protein, 110 aa, Artificial Sequence
  N3 VL mutant 2
QSVLTQPPSASGTPGQRVTISCTGSSSNIGSNYVTWYQQLPGTAPKLLIYDNSNRPSGVPDRFSGSKSGTSASLAISGLQSEDEADYYCSSFSDELGAYVFGGGTKLTVL

SEQ ID NO: 52 - DNA, 330 bp, Artificial Sequence
  N3 VL mutant 2
cagtctgtgctgactcagccaccctcagcgtctgggacccccgggcagagggtcaccatctcttgtactggctcttcatctaatattggcagtaattatgtcacctggtaccagcagctcccaggaacggcccccaaactcctcatctatgataatagtaatcggccaagcggggtccctgaccgattctctggctccaagtctggcacctcagcctccctggccatcagtgggctccagtccgaggatgaggctgattattactgttcttcttttagtgatgagttgggggcttatgtcttcggcggaggcaccaagctgacggtccta

SEQ ID NO: 53 - protein, 110 aa, Artificial Sequence
  N3 VL mutant 3
QSVLTQPPSASGTPGQRVTISCTGSSSNIGSNYVTWYQQLPGTAPKLLIYSNNQRPSGVPDRFSGSKSGTSASLAISGLQSEDEADYYCSSFSDELGAYVFGGGTKLTVL

SEQ ID NO: 54 - DNA, 330 bp, Artificial Sequence
  N3 VL mutant 3
cagtctgtgctgactcagccaccctcagcgtctgggacccccgggcagagggtcaccatctcttgtactggctcttcatctaatattggcagtaattatgtcacctggtaccagcagctcccaggaacggcccccaaactcctcatctatagtaataatcagcggccaagcggggtccctgaccgattctctggctccaagtctggcacctcagcctccctggccatcagtgggctccagtccgaggatgaggctgattattactgttcttcttttagtgatgagttgggggcttatgtcttcggcggaggcaccaagctgacggtccta

SEQ ID NO: 55 - protein, 110 aa, Artificial Sequence
  N3 VL mutant 4
QSVLTQPPSASGTPGQRVTISCTGSSSNIGSNYVTWYQQLPGTAPKLLIYRNNQRPSGVPDRFSGSKSGTSASLAISGLQSEDEADYYCSSFSDELGAYVFGGGTKLTVL

SEQ ID NO: 56 - DNA, 330 bp, Artificial Sequence
  N3 VL mutant 4
cagtctgtgctgactcagccaccctcagcgtctgggacccccgggcagagggtcaccatctcttgtactggctcttcatctaatattggcagtaattatgtcacctggtaccagcagctcccaggaacggcccccaaactcctcatctatcggaataatcagcggccaagcggggtccctgaccgattctctggctccaagtctggcacctcagcctccctggccatcagtgggctccagtccgaggatgaggctgattattactgttcttcttttagtgatgagttgggggcttatgtcttcggcggaggcaccaagctgacggtccta

SEQ ID NO: 57 - protein, 15 aa, Artificial Sequence
  Linker for scFv
GGGGSGGGGSGGGGS

SEQ ID NO: 58 - DNA, 45 bp, Artificial Sequence
  Linker for scFv
ggtggaggcggttcaggcggaggtggatccggcggtggcggatcg

SEQ ID NO: 59 - protein, 241 aa, Artificial Sequence
  N3 scFv (VH+linker+VL)
EVQLLESGGGLVQPGGSLRLSCAASGFTFSSYDMSWVRQAPGKGLEWVSAISYDNGNTYYADSVKGRFTISRDNSKNTLYLQMNSLRAEDTAVYYSARMALDFDYWGQGTLVTVSSGGGGSGGGGSGGGGSQSVLTQPPSASGTPGQRVTISCTGSSSNIGSNYVTWYQQLPGTAPKLLIYDNSNRPSGVPDRFSGSKSGTSASLAISGLRSEDEADYYCASWDDSLSAYVFGGGTKLTVL

SEQ ID NO: 60 - DNA, 723 bp, Artificial Sequence
  N3 scFv (VH+linker+VL)
gaggtgcagctgttggagtctgggggaggcttggtacagcctggggggtccctgagactctcctgtgcagcctctggattcacctttagcagttatgatatgagctgggtccgccaggctccagggaaggggctggagtgggtctcagcgatctcttatgataatggtaatacatattacgctgattctgtaaaaggtcggttcaccatctccagagacaattccaagaacacgctgtatctgcaaatgaacagcctgagagccgaggacacggccgtgtattactctgcgagaatggcgcttgatttcgactactggggccagggtacactggtcaccgtgagctcaggtggaggcggttcaggcggaggtggatccggcggtggcggatcgcagtctgtgctgactcagccaccctcagcgtctgggacccccgggcagagggtcaccatctcttgtactggctcttcatctaatattggcagtaattatgtcacctggtaccagcagctcccaggaacggcccccaaactcctcatctatgataatagtaatcggccaagcggggtccctgaccgattctctggctccaagtctggcacctcagcctccctggccatcagtgggctccggtccgaggatgaggctgattattactgtgcttcttgggatgatagcctgagtgcttatgtcttcggcggaggcaccaagctgacggtccta

SEQ ID NO: 61 - protein, 241 aa, Artificial Sequence
  N3-1 scFv (VH+linker+VL)
EVQLLESGGGLVQPGGSLRLSCAASGFTFSSYDMSWVRQAPGKGLEWVSAISYDNGNTYYADSVKGRFTISRDNSKNTLYLQMNSLRAEDTAVYYSARMALDFDYWGQGTLVTVSSGGGGSGGGGSGGGGSQSVLTQPPSASGTPGQRVTISCTGSSSNIGSNYVTWYQQLPGTAPKLLIYDNSNRPSGVPDRFSGSKSGTSASLAISGLQSEDEADYYCASFSDELGAYVFGGGTKLTVL

SEQ ID NO: 62 - DNA, 723 bp, Artificial Sequence
  N3-1 scFv (VH+linker+VL)
gaggtgcagctgttggagtctgggggaggcttggtacagcctggggggtccctgagactctcctgtgcagcctctggattcacctttagcagttatgatatgagctgggtccgccaggctccagggaaggggctggagtgggtctcagcgatctcttatgataatggtaatacatattacgctgattctgtaaaaggtcggttcaccatctccagagacaattccaagaacacgctgtatctgcaaatgaacagcctgagagccgaggacacggccgtgtattactctgcgagaatggcgcttgatttcgactactggggccagggtacactggtcaccgtgagctcaggtggaggcggttcaggcggaggtggatccggcggtggcggatcgcagtctgtgctgactcagccaccctcagcgtctgggacccccgggcagagggtcaccatctcttgtactggctcttcatctaatattggcagtaattatgtcacctggtaccagcagctcccaggaacggcccccaaactcctcatctatgataatagtaatcggccaagcggggtccctgaccgattctctggctccaagtctggcacctcagcctccctggccatcagtgggctccagtccgaggatgaggctgattattactgtgcttcttttagtgatgagttgggggcttatgtcttcggcggaggcaccaagctgacggtccta

SEQ ID NO: 63 - protein, 241 aa, Artificial Sequence
  N3-3 scFv (VH+linker+VL)
EVQLLESGGGLVQPGGSLRLSCAASGFTFSSYDMSWVRQAPGKGLEWVSAISYDNGNTYYADSVKGRFTISRDNSKNTLYLQMNSLRAEDTAVYYSARMALDFDYWGQGTLVTVSSGGGGSGGGGSGGGGSQSVLTQPPSASGTPGQRVTISCTGSSSNIGSNYVTWYQQLPGTAPKLLIYDNSNRPSGVPDRFSGSKSGTSASLAISGLQSEDEADYYCSSFSDELGAYVFGGGTKLTVL

SEQ ID NO: 64 - DNA, 723 bp, Artificial Sequence
  N3-3 scFv (VH+linker+VL)
gaggtgcagctgttggagtctgggggaggcttggtacagcctggggggtccctgagactctcctgtgcagcctctggattcacctttagcagttatgatatgagctgggtccgccaggctccagggaaggggctggagtgggtctcagcgatctcttatgataatggtaatacatattacgctgattctgtaaaaggtcggttcaccatctccagagacaattccaagaacacgctgtatctgcaaatgaacagcctgagagccgaggacacggccgtgtattactctgcgagaatggcgcttgatttcgactactggggccagggtacactggtcaccgtgagctcaggtggaggcggttcaggcggaggtggatccggcggtggcggatcgcagtctgtgctgactcagccaccctcagcgtctgggacccccgggcagagggtcaccatctcttgtactggctcttcatctaatattggcagtaattatgtcacctggtaccagcagctcccaggaacggcccccaaactcctcatctatgataatagtaatcggccaagcggggtccctgaccgattctctggctccaagtctggcacctcagcctccctggccatcagtgggctccagtccgaggatgaggctgattattactgttcttcttttagtgatgagttgggggcttatgtcttcggcggaggcaccaagctgacggtccta

SEQ ID NO: 65 - protein, 241 aa, Artificial Sequence
  N3-4 scFv (VH+linker+VL)
EVQLLESGGGLVQPGGSLRLSCAASGFTFSSYDMSWVRQAPGKGLEWVSVISSDGGNTYYADSVKGRFTISRDNSKNTLYLQMNSLRAEDTAVYYSARMALDFDYWGQGTLVTVSSGGGGSGGGGSGGGGSQSVLTQPPSASGTPGQRVTISCTGSSSNIGSNYVTWYQQLPGTAPKLLIYDNSNRPSGVPDRFSGSKSGTSASLAISGLQSEDEADYYCASFSDELGAYVFGGGTKLTVL

SEQ ID NO: 66 - DNA, 723 bp, Artificial Sequence
  N3-4 scFv (VH+linker+VL)
gaggtgcagctgttggagtctgggggaggcttggtacagcctggggggtccctgagactctcctgtgcagcctctggattcacctttagcagttatgatatgagctgggtccgccaggctccagggaaggggctggagtgggtctcagtgatctcttctgatggtggtaatacatattacgctgattctgtaaaaggtcggttcaccatctccagagacaattccaagaacacgctgtatctgcaaatgaacagcctgagagccgaggacacggccgtgtattactctgcgagaatggcgcttgatttcgactactggggccagggtacactggtcaccgtgagctcaggtggaggcggttcaggcggaggtggatccggcggtggcggatcgcagtctgtgctgactcagccaccctcagcgtctgggacccccgggcagagggtcaccatctcttgtactggctcttcatctaatattggcagtaattatgtcacctggtaccagcagctcccaggaacggcccccaaactcctcatctatgataatagtaatcggccaagcggggtccctgaccgattctctggctccaagtctggcacctcagcctccctggccatcagtgggctccagtccgaggatgaggctgattattactgtgcttcttttagtgatgagttgggggcttatgtcttcggcggaggcaccaagctgacggtccta

SEQ ID NO: 67 - protein, 241 aa, Artificial Sequence
  N3-5 scFv (VH+linker+VL)
EVQLLESGGGLVQPGGSLRLSCAASGFTFSSYDMSWVRQAPGKGLEWVSVISSDGGNTYYADSVKGRFTISRDNSKNTLYLQMNSLRAEDTAVYYSARMALDFDYWGQGTLVTVSSGGGGSGGGGSGGGGSQSVLTQPPSASGTPGQRVTISCTGSSSNIGSNYVTWYQQLPGTAPKLLIYDNSNRPSGVPDRFSGSKSGTSASLAISGLQSEDEADYYCSSFSDELGAYVFGGGTKLTVL

SEQ ID NO: 68 - DNA, 723 bp, Artificial Sequence
  N3-5 scFv (VH+linker+VL)
gaggtgcagctgttggagtctgggggaggcttggtacagcctggggggtccctgagactctcctgtgcagcctctggattcacctttagcagttatgatatgagctgggtccgccaggctccagggaaggggctggagtgggtctcagtgatctcttctgatggtggtaatacatattacgctgattctgtaaaaggtcggttcaccatctccagagacaattccaagaacacgctgtatctgcaaatgaacagcctgagagccgaggacacggccgtgtattactctgcgagaatggcgcttgatttcgactactggggccagggtacactggtcaccgtgagctcaggtggaggcggttcaggcggaggtggatccggcggtggcggatcgcagtctgtgctgactcagccaccctcagcgtctgggacccccgggcagagggtcaccatctcttgtactggctcttcatctaatattggcagtaattatgtcacctggtaccagcagctcccaggaacggcccccaaactcctcatctatgataatagtaatcggccaagcggggtccctgaccgattctctggctccaagtctggcacctcagcctccctggccatcagtgggctccagtccgaggatgaggctgattattactgttcttcttttagtgatgagttgggggcttatgtcttcggcggaggcaccaagctgacggtccta

SEQ ID NO: 69 - protein, 241 aa, Artificial Sequence
  N3-6 scFv (VH+linker+VL)
EVQLLESGGGLVQPGGSLRLSCAASGFTFSSYDMSWVRQAPGKGLEWVSAISPQMGRVYYADSVKGRFTISRDNSKNTLYLQMNSLRAEDTAVYYCARMALDFDYWGQGTLVTVSSGGGGSGGGGSGGGGSQSVLTQPPSASGTPGQRVTISCTGSSSNIGSNYVTWYQQLPGTAPKLLIYDNSNRPSGVPDRFSGSKSGTSASLAISGLQSEDEADYYCSSFSDELGAYVFGGGTKLTVL

SEQ ID NO: 70 - DNA, 723 bp, Artificial Sequence
  N3-6 scFv (VH+linker+VL)
gaggtgcagctgttggagtctgggggaggcttggtacagcctggggggtccctgagactctcctgtgcagcctctggattcacctttagcagttatgatatgagctgggtccgccaggctccagggaaggggctggagtgggtctcagcgatctcgccgcagatgggtcgggtgtattacgctgattctgtaaaaggtcggttcaccatctccagagacaattccaagaacacgctgtatctgcaaatgaacagcctgagagccgaggacacggccgtgtattactgtgcgagaatggcgcttgatttcgactactggggccagggtacactggtcaccgtgagctcaggtggaggcggttcaggcggaggtggatccggcggtggcggatcgcagtctgtgctgactcagccaccctcagcgtctgggacccccgggcagagggtcaccatctcttgtactggctcttcatctaatattggcagtaattatgtcacctggtaccagcagctcccaggaacggcccccaaactcctcatctatgataatagtaatcggccaagcggggtccctgaccgattctctggctccaagtctggcacctcagcctccctggccatcagtgggctccagtccgaggatgaggctgattattactgttcttcttttagtgatgagttgggggcttatgtcttcggcggaggcaccaagctgacggtccta

SEQ ID NO: 71 - protein, 241 aa, Artificial Sequence
  N3-7 scFv (VH+linker+VL)
EVQLLESGGGLVQPGGSLRLSCAASGFTFSSYDMSWVRQAPGKGLEWVSAIDPLGGNIYYADSVKGRFTISRDNSKNTLYLQMNSLRAEDTAVYYCARMALDFDYWGQGTLVTVSSGGGGSGGGGSGGGGSQSVLTQPPSASGTPGQRVTISCTGSSSNIGSNYVTWYQQLPGTAPKLLIYDNSNRPSGVPDRFSGSKSGTSASLAISGLQSEDEADYYCSSFSDELGAYVFGGGTKLTVL

SEQ ID NO: 72 - DNA, 723 bp, Artificial Sequence
  N3-7 scFv (VH+linker+VL)
gaggtgcagctgttggagtctgggggaggcttggtacagcctggggggtccctgagactctcctgtgcagcctctggattcacctttagcagttatgatatgagctgggtccgccaggctccagggaaggggctggagtgggtctcagcgatcgatccgttggggggtaatatttattacgctgattctgtaaaaggtcggttcaccatctccagagacaattccaagaacacgctgtatctgcaaatgaacagcctgagagccgaggacacggccgtgtattactgtgcgagaatggcgcttgatttcgactactggggccagggtacactggtcaccgtgagctcaggtggaggcggttcaggcggaggtggatccggcggtggcggatcgcagtctgtgctgactcagccaccctcagcgtctgggacccccgggcagagggtcaccatctcttgtactggctcttcatctaatattggcagtaattatgtcacctggtaccagcagctcccaggaacggcccccaaactcctcatctatgataatagtaatcggccaagcggggtccctgaccgattctctggctccaagtctggcacctcagcctccctggccatcagtgggctccagtccgaggatgaggctgattattactgttcttcttttagtgatgagttgggggcttatgtcttcggcggaggcaccaagctgacggtccta

SEQ ID NO: 73 - protein, 241 aa, Artificial Sequence
  N3-8-7 scFv (VH+linker+VL)
EVQLLESGGGLVQPGGSLRLSCAASGFTFSSYDMSWVRQAPGKGLEWVSAISPYSGRIYYADSVKGRFTISRDNSKNTLYLQMNSLRAEDTAVYYSARMALDFDYWGQGTLVTVSSGGGGSGGGGSGGGGSQSVLTQPPSASGTPGQRVTISCTGSSSNIGSNYVTWYQQLPGTAPKLLIYDNSNRPSGVPDRFSGSKSGTSASLAISGLQSEDEADYYCSSFSDELGAYVFGGGTKLTVL

SEQ ID NO: 74 - DNA, 723 bp, Artificial Sequence
  N3-8-7 scFv (VH+linker+VL)
gaggtgcagctgttggagtctgggggaggcttggtacagcctggggggtccctgagactctcctgtgcagcctctggattcacctttagcagttatgatatgagctgggtccgccaggctccagggaaggggctggagtgggtctcagcgatctctccgtattcgggtaggatttattacgctgattctgtaaaaggtcggttcaccatctccagagacaattccaagaacacgctgtatctgcaaatgaacagcctgagagccgaggacacggccgtgtattactctgcgagaatggcgcttgatttcgactactggggccagggtacactggtcaccgtgagctcaggtggaggcggttcaggcggaggtggatccggcggtggcggatcgcagtctgtgctgactcagccaccctcagcgtctgggacccccgggcagagggtcaccatctcttgtactggctcttcatctaatattggcagtaattatgtcacctggtaccagcagctcccaggaacggcccccaaactcctcatctatgataatagtaatcggccaagcggggtccctgaccgattctctggctccaagtctggcacctcagcctccctggccatcagtgggctccagtccgaggatgaggctgattattactgttcttcttttagtgatgagttgggggcttatgtcttcggcggaggcaccaagctgacggtccta

SEQ ID NO: 75 - protein, 241 aa, Artificial Sequence
  N3-9 scFv (VH+linker+VL)
EVQLLESGGGLVQPGGSLRLSCAASGFTFSSYDMSWVRQAPGKGLEWVSAIGADGGPSYYADSVKGRFTISRDNSKNTLYLQMNSLRAEDTAVYYCARMALDFDYWGQGTLVTVSSGGGGSGGGGSGGGGSQSVLTQPPSASGTPGQRVTISCTGSSSNIGSNYVTWYQQLPGTAPKLLIYDNSNRPSGVPDRFSGSKSGTSASLAISGLQSEDEADYYCSSFSDELGAYVFGGGTKLTVL

SEQ ID NO: 76 - DNA, 723 bp, Artificial Sequence
  N3-9 scFv (VH+linker+VL)
gaggtgcagctgttggagtctgggggaggcttggtacagcctggggggtccctgagactctcctgtgcagcctctggattcacctttagcagttatgatatgagctgggtccgccaggctccagggaaggggctggagtgggtctcagcgatcggggctgatgggggtccgtcttattacgctgattctgtaaaaggtcggttcaccatctccagagacaattccaagaacacgctgtatctgcaaatgaacagcctgagagccgaggacacggccgtgtattactgtgcgagaatggcgcttgatttcgactactggggccagggtacactggtcaccgtgagctcaggtggaggcggttcaggcggaggtggatccggcggtggcggatcgcagtctgtgctgactcagccaccctcagcgtctgggacccccgggcagagggtcaccatctcttgtactggctcttcatctaatattggcagtaattatgtcacctggtaccagcagctcccaggaacggcccccaaactcctcatctatgataatagtaatcggccaagcggggtccctgaccgattctctggctccaagtctggcacctcagcctccctggccatcagtgggctccagtccgaggatgaggctgattattactgttcttcttttagtgatgagttgggggcttatgtcttcggcggaggcaccaagctgacggtccta

SEQ ID NO: 77 - protein, 241 aa, Artificial Sequence
  N3-8 scFv, N3-8-1 scFv (VH+linker+VL)
EVQLLESGGGLVQPGGSLRLSCAASGFTFSSYDMSWVRQAPGKGLEWVSAISPYSGRIYYADSVKGRFTISRDNSKNTLYLQMNSLRAEDTAVYYCARMALDFDYWGQGTLVTVSSGGGGSGGGGSGGGGSQSVLTQPPSASGTPGQRVTISCTGSSSNIGSNYVTWYQQLPGTAPKLLIYDNSNRPSGVPDRFSGSKSGTSASLAISGLQSEDEADYYCSSFSDELGAYVFGGGTKLTVL

SEQ ID NO: 78 - DNA, 723 bp, Artificial Sequence
  N3-8 scFv, N3-8-1 scFv (VH+linker+VL)
gaggtgcagctgttggagtctgggggaggcttggtacagcctggggggtccctgagactctcctgtgcagcctctggattcacctttagcagttatgatatgagctgggtccgccaggctccagggaaggggctggagtgggtctcagcgatctctccgtattcgggtaggatttattacgctgattctgtaaaaggtcggttcaccatctccagagacaattccaagaacacgctgtatctgcaaatgaacagcctgagagccgaggacacggccgtgtattactgtgcgagaatggcgcttgatttcgactactggggccagggtacactggtcaccgtgagctcaggtggaggcggttcaggcggaggtggatccggcggtggcggatcgcagtctgtgctgactcagccaccctcagcgtctgggacccccgggcagagggtcaccatctcttgtactggctcttcatctaatattggcagtaattatgtcacctggtaccagcagctcccaggaacggcccccaaactcctcatctatgataatagtaatcggccaagcggggtccctgaccgattctctggctccaagtctggcacctcagcctccctggccatcagtgggctccagtccgaggatgaggctgattattactgttcttcttttagtgatgagttgggggcttatgtcttcggcggaggcaccaagctgacggtccta

SEQ ID NO: 79 - protein, 241 aa, Artificial Sequence
  N3-8-2 scFv (VH+linker+VL)
EVQLLESGGGLVQPGGSLRLSCAASGFTFSSYDMSWVRQAPGKGLEWVSAISPYSGRIYYADSVKGRFTISRDNSKNTLYLQMNSLRAEDTAVYYCARMALDFDYWGQGTLVTVSSGGGGSGGGGSGGGGSQSVLTQPPSASGTPGQRVTISCTGSSSNIGSNYVTWYQQLPGTAPKLLIYSNNQRPSGVPDRFSGSKSGTSASLAISGLQSEDEADYYCSSFSDELGAYVFGGGTKLTVL

SEQ ID NO: 80 - DNA, 723 bp, Artificial Sequence
  N3-8-2 scFv (VH+linker+VL)
gaggtgcagctgttggagtctgggggaggcttggtacagcctggggggtccctgagactctcctgtgcagcctctggattcacctttagcagttatgatatgagctgggtccgccaggctccagggaaggggctggagtgggtctcagcgatctctccgtattcgggtaggatttattacgctgattctgtaaaaggtcggttcaccatctccagagacaattccaagaacacgctgtatctgcaaatgaacagcctgagagccgaggacacggccgtgtattactgtgcgagaatggcgcttgatttcgactactggggccagggtacactggtcaccgtgagctcaggtggaggcggttcaggcggaggtggatccggcggtggcggatcgcagtctgtgctgactcagccaccctcagcgtctgggacccccgggcagagggtcaccatctcttgtactggctcttcatctaatattggcagtaattatgtcacctggtaccagcagctcccaggaacggcccccaaactcctcatctatagtaataatcagcggccaagcggggtccctgaccgattctctggctccaagtctggcacctcagcctccctggccatcagtgggctccagtccgaggatgaggctgattattactgttcttcttttagtgatgagttgggggcttatgtcttcggcggaggcaccaagctgacggtccta

SEQ ID NO: 81 - protein, 241 aa, Artificial Sequence
  N3-8-3 scFv (VH+linker+VL)
EVQLLESGGGLVQPGGSLRLSCAASGFTFSSYDMSWVRQAPGKGLEWVSAISPYSGRIYYADSVKGRFTISRDNSKNTLYLQMNSLRAEDTAVYYCARMALDFDYWGQGTLVTVSSGGGGSGGGGSGGGGSQSVLTQPPSASGTPGQRVTISCTGSSSNIGSNYVTWYQQLPGTAPKLLIYRNNQRPSGVPDRFSGSKSGTSASLAISGLQSEDEADYYCSSFSDELGAYVFGGGTKLTVL

SEQ ID NO: 82 - DNA, 723 bp, Artificial Sequence
  N3-8-3 scFv (VH+linker+VL)
gaggtgcagctgttggagtctgggggaggcttggtacagcctggggggtccctgagactctcctgtgcagcctctggattcacctttagcagttatgatatgagctgggtccgccaggctccagggaaggggctggagtgggtctcagcgatctctccgtattcgggtaggatttattacgctgattctgtaaaaggtcggttcaccatctccagagacaattccaagaacacgctgtatctgcaaatgaacagcctgagagccgaggacacggccgtgtattactgtgcgagaatggcgcttgatttcgactactggggccagggtacactggtcaccgtgagctcaggtggaggcggttcaggcggaggtggatccggcggtggcggatcgcagtctgtgctgactcagccaccctcagcgtctgggacccccgggcagagggtcaccatctcttgtactggctcttcatctaatattggcagtaattatgtcacctggtaccagcagctcccaggaacggcccccaaactcctcatctatcggaataatcagcggccaagcggggtccctgaccgattctctggctccaagtctggcacctcagcctccctggccatcagtgggctccagtccgaggatgaggctgattattactgttcttcttttagtgatgagttgggggcttatgtcttcggcggaggcaccaagctgacggtccta

SEQ ID NO: 83 - protein, 241 aa, Artificial Sequence
  N3-8-4 scFv (VH+linker+VL)
EVQLLESGGGLVQPGGSLRLSCAASGFTFSSYDMSWVRQAPGKGLEWVSAISPYSGRIYYADSVKGRFTISRDNSKNTLYLQMNSLRAEDTAVYYCARLALDFDYWGQGTLVTVSSGGGGSGGGGSGGGGSQSVLTQPPSASGTPGQRVTISCTGSSSNIGSNYVTWYQQLPGTAPKLLIYDNSNRPSGVPDRFSGSKSGTSASLAISGLQSEDEADYYCSSFSDELGAYVFGGGTKLTVL

SEQ ID NO: 84 - DNA, 723 bp, Artificial Sequence
  N3-8-4 scFv (VH+linker+VL)
gaggtgcagctgttggagtctgggggaggcttggtacagcctggggggtccctgagactctcctgtgcagcctctggattcacctttagcagttatgatatgagctgggtccgccaggctccagggaaggggctggagtgggtctcagcgatctctccgtattcgggtaggatttattacgctgattctgtaaaaggtcggttcaccatctccagagacaattccaagaacacgctgtatctgcaaatgaacagcctgagagccgaggacacggccgtgtattactgtgcgagactggcgcttgatttcgactactggggccagggtacactggtcaccgtgagctcaggtggaggcggttcaggcggaggtggatccggcggtggcggatcgcagtctgtgctgactcagccaccctcagcgtctgggacccccgggcagagggtcaccatctcttgtactggctcttcatctaatattggcagtaattatgtcacctggtaccagcagctcccaggaacggcccccaaactcctcatctatgataatagtaatcggccaagcggggtccctgaccgattctctggctccaagtctggcacctcagcctccctggccatcagtgggctccagtccgaggatgaggctgattattactgttcttcttttagtgatgagttgggggcttatgtcttcggcggaggcaccaagctgacggtccta

SEQ ID NO: 85 - protein, 241 aa, Artificial Sequence
  N3-8-5 scFv (VH+linker+VL)
EVQLLESGGGLVQPGGSLRLSCAASGFTFSSYDMSWVRQAPGKGLEWVSAISPYSGRIYYADSVKGRFTISRDNSKNTLYLQMNSLRAEDTAVYYCARLALDFDYWGQGTLVTVSSGGGGSGGGGSGGGGSQSVLTQPPSASGTPGQRVTISCTGSSSNIGSNYVTWYQQLPGTAPKLLIYSNNQRPSGVPDRFSGSKSGTSASLAISGLQSEDEADYYCSSFSDELGAYVFGGGTKLTVL

SEQ ID NO: 86 - DNA, 723 bp, Artificial Sequence
  N3-8-5 scFv (VH+linker+VL)
gaggtgcagctgttggagtctgggggaggcttggtacagcctggggggtccctgagactctcctgtgcagcctctggattcacctttagcagttatgatatgagctgggtccgccaggctccagggaaggggctggagtgggtctcagcgatctctccgtattcgggtaggatttattacgctgattctgtaaaaggtcggttcaccatctccagagacaattccaagaacacgctgtatctgcaaatgaacagcctgagagccgaggacacggccgtgtattactgtgcgagactggcgcttgatttcgactactggggccagggtacactggtcaccgtgagctcaggtggaggcggttcaggcggaggtggatccggcggtggcggatcgcagtctgtgctgactcagccaccctcagcgtctgggacccccgggcagagggtcaccatctcttgtactggctcttcatctaatattggcagtaattatgtcacctggtaccagcagctcccaggaacggcccccaaactcctcatctatagtaataatcagcggccaagcggggtccctgaccgattctctggctccaagtctggcacctcagcctccctggccatcagtgggctccagtccgaggatgaggctgattattactgttcttcttttagtgatgagttgggggcttatgtcttcggcggaggcaccaagctgacggtccta

SEQ ID NO: 87 - protein, 241 aa, Artificial Sequence
  N3-8-6 scFv (VH+linker+VL)
EVQLLESGGGLVQPGGSLRLSCAASGFTFSSYDMSWVRQAPGKGLEWVSAISPYSGRIYYADSVKGRFTISRDNSKNTLYLQMNSLRAEDTAVYYCARLALDFDYWGQGTLVTVSSGGGGSGGGGSGGGGSQSVLTQPPSASGTPGQRVTISCTGSSSNIGSNYVTWYQQLPGTAPKLLIYRNNQRPSGVPDRFSGSKSGTSASLAISGLQSEDEADYYCSSFSDELGAYVFGGGTKLTVL

SEQ ID NO: 88 - DNA, 723 bp, Artificial Sequence
  N3-8-6 scFv (VH+linker+VL)
gaggtgcagctgttggagtctgggggaggcttggtacagcctggggggtccctgagactctcctgtgcagcctctggattcacctttagcagttatgatatgagctgggtccgccaggctccagggaaggggctggagtgggtctcagcgatctctccgtattcgggtaggatttattacgctgattctgtaaaaggtcggttcaccatctccagagacaattccaagaacacgctgtatctgcaaatgaacagcctgagagccgaggacacggccgtgtattactgtgcgagactggcgcttgatttcgactactggggccagggtacactggtcaccgtgagctcaggtggaggcggttcaggcggaggtggatccggcggtggcggatcgcagtctgtgctgactcagccaccctcagcgtctgggacccccgggcagagggtcaccatctcttgtactggctcttcatctaatattggcagtaattatgtcacctggtaccagcagctcccaggaacggcccccaaactcctcatctatcggaataatcagcggccaagcggggtccctgaccgattctctggctccaagtctggcacctcagcctccctggccatcagtgggctccagtccgaggatgaggctgattattactgttcttcttttagtgatgagttgggggcttatgtcttcggcggaggcaccaagctgacggtccta

SEQ ID NO: 89 - protein, 446 aa, Artificial Sequence
  N3 IgG heavy chain
EVQLLESGGGLVQPGGSLRLSCAASGFTFSSYDMSWVRQAPGKGLEWVSAISYDNGNTYYADSVKGRFTISRDNSKNTLYLQMNSLRAEDTAVYYSARMALDFDYWGQGTLVTVSSASTKGPSVFPLAPSSKSTSGGTAALGCLVKDYFPEPVTVSWNSGALTSGVHTFPAVLQSSGLYSLSSVVTVPSSSLGTQTYICNVNHKPSNTKVDKKVEPKSCDKTHTCPPCPAPELLGGPSVFLFPPKPKDTLMISRTPEVTCVVVDVSHEDPEVKFNWYVDGVEVHNAKTKPREEQYNSTYRVVSVLTVLHQDWLNGKEYKCKVSNKALPAPIEKTISKAKGQPREPQVYTLPPSRDELTKNQVSLTCLVKGFYPSDIAVEWESNGQPENNYKTTPPVLDSDGSFFLYSKLTVDKSRWQQGNVFSCSVMHEALHNHYTQKSLSLSPGK

SEQ ID NO: 90 - DNA, 1338 bp, Artificial Sequence
  N3 IgG heavy chain
gaggtgcagctgttggagtctgggggaggcttggtacagcctggggggtccctgagactctcctgtgcagcctctggattcacctttagcagttatgatatgagctgggtccgccaggctccagggaaggggctggagtgggtctcagcgatctcttatgataatggtaatacatattacgctgattctgtaaaaggtcggttcaccatctccagagacaattccaagaacacgctgtatctgcaaatgaacagcctgagagccgaggacacggccgtgtattactctgcgagaatggcgcttgatttcgactactggggccagggtacactggtcaccgtgagctcagcctccaccaagggcccatcggtcttccccctggcaccctcctccaagagcacctctgggggcacagcggccctgggctgcctggtcaaggactacttccccgaaccggtgacggtgtcgtggaactcaggcgccctgaccagcggcgtgcacaccttcccggctgtcctacagtcctcaggactctactccctcagcagcgtggtgaccgtgccctccagcagcttgggcacccagacctacatctgcaacgtgaatcacaagcccagcaacaccaaggtggacaagaaagttgagcccaaatcttgtgacaaaactcacacatgcccaccgtgcccagcacctgaactcctggggggaccgtcagtcttcctcttccccccaaaacccaaggacaccctcatgatctcccggacccctgaggtcacatgcgtggtggtggacgtgagccacgaagaccctgaggtcaagttcaactggtacgtggacggcgtggaggtgcataatgccaagacaaagccgcgggaggagcagtacaacagcacgtaccgtgtggtcagcgtcctcaccgtcctgcaccaggactggctgaatggcaaggagtacaagtgcaaggtctccaacaaagccctcccagcccccatcgagaaaaccatctccaaagccaaagggcagccccgagaaccacaggtgtataccctgcccccatcccgggatgagctgaccaagaaccaggtcagcctgacctgcctggtcaaaggcttctatcccagcgacatcgccgtggagtgggagagcaatgggcagccggagaacaactacaagaccacgcctcccgtgctggactccgacggctccttcttcctctacagcaagctcaccgtggacaagagcaggtggcagcaggggaacgtcttctcatgctccgtgatgcatgaggctctgcacaaccactacacgcagaagagcctctccctgtccccgggtaaa

SEQ ID NO: 91 - protein, 217 aa, Artificial Sequence
  N3 IgG light chain
QSVLTQPPSASGTPGQRVTISCTGSSSNIGSNYVTWYQQLPGTAPKLLIYDNSNRPSGVPDRFSGSKSGTSASLAISGLRSEDEADYYCASWDDSLSAYVFGGGTKLTVLRTVAAPSVFIFPPSDEQLKSGTASVVCLLNNFYPREAKVQWKVDNALQSGNSQESVTEQDSKDSTYSLSSTLTLSKADYEKHKVYACEVTHQGLSSPVTKSFNRGEC

SEQ ID NO: 92 - DNA, 651 bp, Artificial Sequence
  N3 IgG light chain
cagtctgtgctgactcagccaccctcagcgtctgggacccccgggcagagggtcaccatctcttgtactggctcttcatctaatattggcagtaattatgtcacctggtaccagcagctcccaggaacggcccccaaactcctcatctatgataatagtaatcggccaagcggggtccctgaccgattctctggctccaagtctggcacctcagcctccctggccatcagtgggctccggtccgaggatgaggctgattattactgtgcttcttgggatgatagcctgagtgcttatgtcttcggcggaggcaccaagctgacggtcctacgtacggtggctgcaccatctgtcttcatcttcccgccatctgatgagcagttgaaatctggaactgcctctgttgtgtgcctgctgaataacttctatcccagagaggccaaagtacagtggaaggtggataacgccctccaatcgggtaactcccaggagagtgtcacagagcaggacagcaaggacagcacctacagcctcagcagcaccctgacgctgagcaaagcagactacgagaaacacaaagtctacgcctgcgaagtcacccatcagggcctgagctcgcccgtcacaaagagcttcaacaggggagagtgt

SEQ ID NO: 93 - protein, 446 aa, Artificial Sequence
  IgG heavy chain 1
EVQLLESGGGLVQPGGSLRLSCAASGFTFSSYDMSWVRQAPGKGLEWVSVISSDGGNTYYADSVKGRFTISRDNSKNTLYLQMNSLRAEDTAVYYSARMALDFDYWGQGTLVTVSSASTKGPSVFPLAPSSKSTSGGTAALGCLVKDYFPEPVTVSWNSGALTSGVHTFPAVLQSSGLYSLSSVVTVPSSSLGTQTYICNVNHKPSNTKVDKKVEPKSCDKTHTCPPCPAPELLGGPSVFLFPPKPKDTLMISRTPEVTCVVVDVSHEDPEVKFNWYVDGVEVHNAKTKPREEQYNSTYRVVSVLTVLHQDWLNGKEYKCKVSNKALPAPIEKTISKAKGQPREPQVYTLPPSRDELTKNQVSLTCLVKGFYPSDIAVEWESNGQPENNYKTTPPVLDSDGSFFLYSKLTVDKSRWQQGNVFSCSVMHEALHNHYTQKSLSLSPGK

SEQ ID NO: 94 - DNA, 1338 bp, Artificial Sequence
  IgG heavy chain 1
gaggtgcagctgttggagtctgggggaggcttggtacagcctggggggtccctgagactctcctgtgcagcctctggattcacctttagcagttatgatatgagctgggtccgccaggctccagggaaggggctggagtgggtctcagtgatctcttctgatggtggtaatacatattacgctgattctgtaaaaggtcggttcaccatctccagagacaattccaagaacacgctgtatctgcaaatgaacagcctgagagccgaggacacggccgtgtattactctgcgagaatggcgcttgatttcgactactggggccagggtacactggtcaccgtgagctcagcctccaccaagggcccatcggtcttccccctggcaccctcctccaagagcacctctgggggcacagcggccctgggctgcctggtcaaggactacttccccgaaccggtgacggtgtcgtggaactcaggcgccctgaccagcggcgtgcacaccttcccggctgtcctacagtcctcaggactctactccctcagcagcgtggtgaccgtgccctccagcagcttgggcacccagacctacatctgcaacgtgaatcacaagcccagcaacaccaaggtggacaagaaagttgagcccaaatcttgtgacaaaactcacacatgcccaccgtgcccagcacctgaactcctggggggaccgtcagtcttcctcttccccccaaaacccaaggacaccctcatgatctcccggacccctgaggtcacatgcgtggtggtggacgtgagccacgaagaccctgaggtcaagttcaactggtacgtggacggcgtggaggtgcataatgccaagacaaagccgcgggaggagcagtacaacagcacgtaccgtgtggtcagcgtcctcaccgtcctgcaccaggactggctgaatggcaaggagtacaagtgcaaggtctccaacaaagccctcccagcccccatcgagaaaaccatctccaaagccaaagggcagccccgagaaccacaggtgtataccctgcccccatcccgggatgagctgaccaagaaccaggtcagcctgacctgcctggtcaaaggcttctatcccagcgacatcgccgtggagtgggagagcaatgggcagccggagaacaactacaagaccacgcctcccgtgctggactccgacggctccttcttcctctacagcaagctcaccgtggacaagagcaggtggcagcaggggaacgtcttctcatgctccgtgatgcatgaggctctgcacaaccactacacgcagaagagcctctccctgtccccgggtaaa

SEQ ID NO: 95 - protein, 446 aa, Artificial Sequence
  IgG heavy chain 2
EVQLLESGGGLVQPGGSLRLSCAASGFTFSSYDMSWVRQAPGKGLEWVSAISPQMGRVYYADSVKGRFTISRDNSKNTLYLQMNSLRAEDTAVYYCARMALDFDYWGQGTLVTVSSASTKGPSVFPLAPSSKSTSGGTAALGCLVKDYFPEPVTVSWNSGALTSGVHTFPAVLQSSGLYSLSSVVTVPSSSLGTQTYICNVNHKPSNTKVDKKVEPKSCDKTHTCPPCPAPELLGGPSVFLFPPKPKDTLMISRTPEVTCVVVDVSHEDPEVKFNWYVDGVEVHNAKTKPREEQYNSTYRVVSVLTVLHQDWLNGKEYKCKVSNKALPAPIEKTISKAKGQPREPQVYTLPPSRDELTKNQVSLTCLVKGFYPSDIAVEWESNGQPENNYKTTPPVLDSDGSFFLYSKLTVDKSRWQQGNVFSCSVMHEALHNHYTQKSLSLSPGK

SEQ ID NO: 96 - DNA, 1338 bp, Artificial Sequence
  IgG heavy chain 2
gaggtgcagctgttggagtctgggggaggcttggtacagcctggggggtccctgagactctcctgtgcagcctctggattcacctttagcagttatgatatgagctgggtccgccaggctccagggaaggggctggagtgggtctcagcgatctcgccgcagatgggtcgggtgtattacgctgattctgtaaaaggtcggttcaccatctccagagacaattccaagaacacgctgtatctgcaaatgaacagcctgagagccgaggacacggccgtgtattactgtgcgagaatggcgcttgatttcgactactggggccagggtacactggtcaccgtgagctcagcctccaccaagggcccatcggtcttccccctggcaccctcctccaagagcacctctgggggcacagcggccctgggctgcctggtcaaggactacttccccgaaccggtgacggtgtcgtggaactcaggcgccctgaccagcggcgtgcacaccttcccggctgtcctacagtcctcaggactctactccctcagcagcgtggtgaccgtgccctccagcagcttgggcacccagacctacatctgcaacgtgaatcacaagcccagcaacaccaaggtggacaagaaagttgagcccaaatcttgtgacaaaactcacacatgcccaccgtgcccagcacctgaactcctggggggaccgtcagtcttcctcttccccccaaaacccaaggacaccctcatgatctcccggacccctgaggtcacatgcgtggtggtggacgtgagccacgaagaccctgaggtcaagttcaactggtacgtggacggcgtggaggtgcataatgccaagacaaagccgcgggaggagcagtacaacagcacgtaccgtgtggtcagcgtcctcaccgtcctgcaccaggactggctgaatggcaaggagtacaagtgcaaggtctccaacaaagccctcccagcccccatcgagaaaaccatctccaaagccaaagggcagccccgagaaccacaggtgtataccctgcccccatcccgggatgagctgaccaagaaccaggtcagcctgacctgcctggtcaaaggcttctatcccagcgacatcgccgtggagtgggagagcaatgggcagccggagaacaactacaagaccacgcctcccgtgctggactccgacggctccttcttcctctacagcaagctcaccgtggacaagagcaggtggcagcaggggaacgtcttctcatgctccgtgatgcatgaggctctgcacaaccactacacgcagaagagcctctccctgtccccgggtaaa

SEQ ID NO: 97 - protein, 446 aa, Artificial Sequence
  IgG heavy chain 3
EVQLLESGGGLVQPGGSLRLSCAASGFTFSSYDMSWVRQAPGKGLEWVSAIDPLGGNIYYADSVKGRFTISRDNSKNTLYLQMNSLRAEDTAVYYCARMALDFDYWGQGTLVTVSSASTKGPSVFPLAPSSKSTSGGTAALGCLVKDYFPEPVTVSWNSGALTSGVHTFPAVLQSSGLYSLSSVVTVPSSSLGTQTYICNVNHKPSNTKVDKKVEPKSCDKTHTCPPCPAPELLGGPSVFLFPPKPKDTLMISRTPEVTCVVVDVSHEDPEVKFNWYVDGVEVHNAKTKPREEQYNSTYRVVSVLTVLHQDWLNGKEYKCKVSNKALPAPIEKTISKAKGQPREPQVYTLPPSRDELTKNQVSLTCLVKGFYPSDIAVEWESNGQPENNYKTTPPVLDSDGSFFLYSKLTVDKSRWQQGNVFSCSVMHEALHNHYTQKSLSLSPGK

SEQ ID NO: 98 - DNA, 1338 bp, Artificial Sequence
  IgG heavy chain 3
gaggtgcagctgttggagtctgggggaggcttggtacagcctggggggtccctgagactctcctgtgcagcctctggattcacctttagcagttatgatatgagctgggtccgccaggctccagggaaggggctggagtgggtctcagcgatcgatccgttggggggtaatatttattacgctgattctgtaaaaggtcggttcaccatctccagagacaattccaagaacacgctgtatctgcaaatgaacagcctgagagccgaggacacggccgtgtattactgtgcgagaatggcgcttgatttcgactactggggccagggtacactggtcaccgtgagctcagcctccaccaagggcccatcggtcttccccctggcaccctcctccaagagcacctctgggggcacagcggccctgggctgcctggtcaaggactacttccccgaaccggtgacggtgtcgtggaactcaggcgccctgaccagcggcgtgcacaccttcccggctgtcctacagtcctcaggactctactccctcagcagcgtggtgaccgtgccctccagcagcttgggcacccagacctacatctgcaacgtgaatcacaagcccagcaacaccaaggtggacaagaaagttgagcccaaatcttgtgacaaaactcacacatgcccaccgtgcccagcacctgaactcctggggggaccgtcagtcttcctcttccccccaaaacccaaggacaccctcatgatctcccggacccctgaggtcacatgcgtggtggtggacgtgagccacgaagaccctgaggtcaagttcaactggtacgtggacggcgtggaggtgcataatgccaagacaaagccgcgggaggagcagtacaacagcacgtaccgtgtggtcagcgtcctcaccgtcctgcaccaggactggctgaatggcaaggagtacaagtgcaaggtctccaacaaagccctcccagcccccatcgagaaaaccatctccaaagccaaagggcagccccgagaaccacaggtgtataccctgcccccatcccgggatgagctgaccaagaaccaggtcagcctgacctgcctggtcaaaggcttctatcccagcgacatcgccgtggagtgggagagcaatgggcagccggagaacaactacaagaccacgcctcccgtgctggactccgacggctccttcttcctctacagcaagctcaccgtggacaagagcaggtggcagcaggggaacgtcttctcatgctccgtgatgcatgaggctctgcacaaccactacacgcagaagagcctctccctgtccccgggtaaa

SEQ ID NO: 99 - protein, 446 aa, Artificial Sequence
  IgG heavy chain 4
EVQLLESGGGLVQPGGSLRLSCAASGFTFSSYDMSWVRQAPGKGLEWVSAISPYSGRIYYADSVKGRFTISRDNSKNTLYLQMNSLRAEDTAVYYSARMALDFDYWGQGTLVTVSSASTKGPSVFPLAPSSKSTSGGTAALGCLVKDYFPEPVTVSWNSGALTSGVHTFPAVLQSSGLYSLSSVVTVPSSSLGTQTYICNVNHKPSNTKVDKKVEPKSCDKTHTCPPCPAPELLGGPSVFLFPPKPKDTLMISRTPEVTCVVVDVSHEDPEVKFNWYVDGVEVHNAKTKPREEQYNSTYRVVSVLTVLHQDWLNGKEYKCKVSNKALPAPIEKTISKAKGQPREPQVYTLPPSRDELTKNQVSLTCLVKGFYPSDIAVEWESNGQPENNYKTTPPVLDSDGSFFLYSKLTVDKSRWQQGNVFSCSVMHEALHNHYTQKSLSLSPGK

SEQ ID NO: 100 - DNA, 1338 bp, Artificial Sequence
  IgG heavy chain 4
gaggtgcagctgttggagtctgggggaggcttggtacagcctggggggtccctgagactctcctgtgcagcctctggattcacctttagcagttatgatatgagctgggtccgccaggctccagggaaggggctggagtgggtctcagcgatctctccgtattcgggtaggatttattacgctgattctgtaaaaggtcggttcaccatctccagagacaattccaagaacacgctgtatctgcaaatgaacagcctgagagccgaggacacggccgtgtattactctgcgagaatggcgcttgatttcgactactggggccagggtacactggtcaccgtgagctcagcctccaccaagggcccatcggtcttccccctggcaccctcctccaagagcacctctgggggcacagcggccctgggctgcctggtcaaggactacttccccgaaccggtgacggtgtcgtggaactcaggcgccctgaccagcggcgtgcacaccttcccggctgtcctacagtcctcaggactctactccctcagcagcgtggtgaccgtgccctccagcagcttgggcacccagacctacatctgcaacgtgaatcacaagcccagcaacaccaaggtggacaagaaagttgagcccaaatcttgtgacaaaactcacacatgcccaccgtgcccagcacctgaactcctggggggaccgtcagtcttcctcttccccccaaaacccaaggacaccctcatgatctcccggacccctgaggtcacatgcgtggtggtggacgtgagccacgaagaccctgaggtcaagttcaactggtacgtggacggcgtggaggtgcataatgccaagacaaagccgcgggaggagcagtacaacagcacgtaccgtgtggtcagcgtcctcaccgtcctgcaccaggactggctgaatggcaaggagtacaagtgcaaggtctccaacaaagccctcccagcccccatcgagaaaaccatctccaaagccaaagggcagccccgagaaccacaggtgtataccctgcccccatcccgggatgagctgaccaagaaccaggtcagcctgacctgcctggtcaaaggcttctatcccagcgacatcgccgtggagtgggagagcaatgggcagccggagaacaactacaagaccacgcctcccgtgctggactccgacggctccttcttcctctacagcaagctcaccgtggacaagagcaggtggcagcaggggaacgtcttctcatgctccgtgatgcatgaggctctgcacaaccactacacgcagaagagcctctccctgtccccgggtaaa

SEQ ID NO: 101 - protein, 446 aa, Artificial Sequence
  IgG heavy chain 5
EVQLLESGGGLVQPGGSLRLSCAASGFTFSSYDMSWVRQAPGKGLEWVSAIGADGGPSYYADSVKGRFTISRDNSKNTLYLQMNSLRAEDTAVYYCARMALDFDYWGQGTLVTVSSASTKGPSVFPLAPSSKSTSGGTAALGCLVKDYFPEPVTVSWNSGALTSGVHTFPAVLQSSGLYSLSSVVTVPSSSLGTQTYICNVNHKPSNTKVDKKVEPKSCDKTHTCPPCPAPELLGGPSVFLFPPKPKDTLMISRTPEVTCVVVDVSHEDPEVKFNWYVDGVEVHNAKTKPREEQYNSTYRVVSVLTVLHQDWLNGKEYKCKVSNKALPAPIEKTISKAKGQPREPQVYTLPPSRDELTKNQVSLTCLVKGFYPSDIAVEWESNGQPENNYKTTPPVLDSDGSFFLYSKLTVDKSRWQQGNVFSCSVMHEALHNHYTQKSLSLSPGK

SEQ ID NO: 102 - DNA, 1338 bp, Artificial Sequence
  IgG heavy chain 5
gaggtgcagctgttggagtctgggggaggcttggtacagcctggggggtccctgagactctcctgtgcagcctctggattcacctttagcagttatgatatgagctgggtccgccaggctccagggaaggggctggagtgggtctcagcgatcggggctgatgggggtccgtcttattacgctgattctgtaaaaggtcggttcaccatctccagagacaattccaagaacacgctgtatctgcaaatgaacagcctgagagccgaggacacggccgtgtattactgtgcgagaatggcgcttgatttcgactactggggccagggtacactggtcaccgtgagctcagcctccaccaagggcccatcggtcttccccctggcaccctcctccaagagcacctctgggggcacagcggccctgggctgcctggtcaaggactacttccccgaaccggtgacggtgtcgtggaactcaggcgccctgaccagcggcgtgcacaccttcccggctgtcctacagtcctcaggactctactccctcagcagcgtggtgaccgtgccctccagcagcttgggcacccagacctacatctgcaacgtgaatcacaagcccagcaacaccaaggtggacaagaaagttgagcccaaatcttgtgacaaaactcacacatgcccaccgtgcccagcacctgaactcctggggggaccgtcagtcttcctcttccccccaaaacccaaggacaccctcatgatctcccggacccctgaggtcacatgcgtggtggtggacgtgagccacgaagaccctgaggtcaagttcaactggtacgtggacggcgtggaggtgcataatgccaagacaaagccgcgggaggagcagtacaacagcacgtaccgtgtggtcagcgtcctcaccgtcctgcaccaggactggctgaatggcaaggagtacaagtgcaaggtctccaacaaagccctcccagcccccatcgagaaaaccatctccaaagccaaagggcagccccgagaaccacaggtgtataccctgcccccatcccgggatgagctgaccaagaaccaggtcagcctgacctgcctggtcaaaggcttctatcccagcgacatcgccgtggagtgggagagcaatgggcagccggagaacaactacaagaccacgcctcccgtgctggactccgacggctccttcttcctctacagcaagctcaccgtggacaagagcaggtggcagcaggggaacgtcttctcatgctccgtgatgcatgaggctctgcacaaccactacacgcagaagagcctctccctgtccccgggtaaa

SEQ ID NO: 103 - protein, 446 aa, Artificial Sequence
  IgG heavy chain 6
EVQLLESGGGLVQPGGSLRLSCAASGFTFSSYDMSWVRQAPGKGLEWVSAISPYSGRIYYADSVKGRFTISRDNSKNTLYLQMNSLRAEDTAVYYCARMALDFDYWGQGTLVTVSSASTKGPSVFPLAPSSKSTSGGTAALGCLVKDYFPEPVTVSWNSGALTSGVHTFPAVLQSSGLYSLSSVVTVPSSSLGTQTYICNVNHKPSNTKVDKKVEPKSCDKTHTCPPCPAPELLGGPSVFLFPPKPKDTLMISRTPEVTCVVVDVSHEDPEVKFNWYVDGVEVHNAKTKPREEQYNSTYRVVSVLTVLHQDWLNGKEYKCKVSNKALPAPIEKTISKAKGQPREPQVYTLPPSRDELTKNQVSLTCLVKGFYPSDIAVEWESNGQPENNYKTTPPVLDSDGSFFLYSKLTVDKSRWQQGNVFSCSVMHEALHNHYTQKSLSLSPGK

SEQ ID NO: 104 - DNA, 1338 bp, Artificial Sequence
  IgG heavy chain 6
gaggtgcagctgttggagtctgggggaggcttggtacagcctggggggtccctgagactctcctgtgcagcctctggattcacctttagcagttatgatatgagctgggtccgccaggctccagggaaggggctggagtgggtctcagcgatctctccgtattcgggtaggatttattacgctgattctgtaaaaggtcggttcaccatctccagagacaattccaagaacacgctgtatctgcaaatgaacagcctgagagccgaggacacggccgtgtattactgtgcgagaatggcgcttgatttcgactactggggccagggtacactggtcaccgtgagctcagcctccaccaagggcccatcggtcttccccctggcaccctcctccaagagcacctctgggggcacagcggccctgggctgcctggtcaaggactacttccccgaaccggtgacggtgtcgtggaactcaggcgccctgaccagcggcgtgcacaccttcccggctgtcctacagtcctcaggactctactccctcagcagcgtggtgaccgtgccctccagcagcttgggcacccagacctacatctgcaacgtgaatcacaagcccagcaacaccaaggtggacaagaaagttgagcccaaatcttgtgacaaaactcacacatgcccaccgtgcccagcacctgaactcctggggggaccgtcagtcttcctcttccccccaaaacccaaggacaccctcatgatctcccggacccctgaggtcacatgcgtggtggtggacgtgagccacgaagaccctgaggtcaagttcaactggtacgtggacggcgtggaggtgcataatgccaagacaaagccgcgggaggagcagtacaacagcacgtaccgtgtggtcagcgtcctcaccgtcctgcaccaggactggctgaatggcaaggagtacaagtgcaaggtctccaacaaagccctcccagcccccatcgagaaaaccatctccaaagccaaagggcagccccgagaaccacaggtgtataccctgcccccatcccgggatgagctgaccaagaaccaggtcagcctgacctgcctggtcaaaggcttctatcccagcgacatcgccgtggagtgggagagcaatgggcagccggagaacaactacaagaccacgcctcccgtgctggactccgacggctccttcttcctctacagcaagctcaccgtggacaagagcaggtggcagcaggggaacgtcttctcatgctccgtgatgcatgaggctctgcacaaccactacacgcagaagagcctctccctgtccccgggtaaa

SEQ ID NO: 105 - protein, 446 aa, Artificial Sequence
  IgG heavy chain 7
EVQLLESGGGLVQPGGSLRLSCAASGFTFSSYDMSWVRQAPGKGLEWVSAISPYSGRIYYADSVKGRFTISRDNSKNTLYLQMNSLRAEDTAVYYCARLALDFDYWGQGTLVTVSSASTKGPSVFPLAPSSKSTSGGTAALGCLVKDYFPEPVTVSWNSGALTSGVHTFPAVLQSSGLYSLSSVVTVPSSSLGTQTYICNVNHKPSNTKVDKKVEPKSCDKTHTCPPCPAPELLGGPSVFLFPPKPKDTLMISRTPEVTCVVVDVSHEDPEVKFNWYVDGVEVHNAKTKPREEQYNSTYRVVSVLTVLHQDWLNGKEYKCKVSNKALPAPIEKTISKAKGQPREPQVYTLPPSRDELTKNQVSLTCLVKGFYPSDIAVEWESNGQPENNYKTTPPVLDSDGSFFLYSKLTVDKSRWQQGNVFSCSVMHEALHNHYTQKSLSLSPGK

SEQ ID NO: 106 - DNA, 1338 bp, Artificial Sequence
  IgG heavy chain 7
gaggtgcagctgttggagtctgggggaggcttggtacagcctggggggtccctgagactctcctgtgcagcctctggattcacctttagcagttatgatatgagctgggtccgccaggctccagggaaggggctggagtgggtctcagcgatctctccgtattcgggtaggatttattacgctgattctgtaaaaggtcggttcaccatctccagagacaattccaagaacacgctgtatctgcaaatgaacagcctgagagccgaggacacggccgtgtattactgtgcgagactggcgcttgatttcgactactggggccagggtacactggtcaccgtgagctcagcctccaccaagggcccatcggtcttccccctggcaccctcctccaagagcacctctgggggcacagcggccctgggctgcctggtcaaggactacttccccgaaccggtgacggtgtcgtggaactcaggcgccctgaccagcggcgtgcacaccttcccggctgtcctacagtcctcaggactctactccctcagcagcgtggtgaccgtgccctccagcagcttgggcacccagacctacatctgcaacgtgaatcacaagcccagcaacaccaaggtggacaagaaagttgagcccaaatcttgtgacaaaactcacacatgcccaccgtgcccagcacctgaactcctggggggaccgtcagtcttcctcttccccccaaaacccaaggacaccctcatgatctcccggacccctgaggtcacatgcgtggtggtggacgtgagccacgaagaccctgaggtcaagttcaactggtacgtggacggcgtggaggtgcataatgccaagacaaagccgcgggaggagcagtacaacagcacgtaccgtgtggtcagcgtcctcaccgtcctgcaccaggactggctgaatggcaaggagtacaagtgcaaggtctccaacaaagccctcccagcccccatcgagaaaaccatctccaaagccaaagggcagccccgagaaccacaggtgtataccctgcccccatcccgggatgagctgaccaagaaccaggtcagcctgacctgcctggtcaaaggcttctatcccagcgacatcgccgtggagtgggagagcaatgggcagccggagaacaactacaagaccacgcctcccgtgctggactccgacggctccttcttcctctacagcaagctcaccgtggacaagagcaggtggcagcaggggaacgtcttctcatgctccgtgatgcatgaggctctgcacaaccactacacgcagaagagcctctccctgtccccgggtaaa

SEQ ID NO: 107 - protein, 217 aa, Artificial Sequence
  IgG light chain 1
QSVLTQPPSASGTPGQRVTISCTGSSSNIGSNYVTWYQQLPGTAPKLLIYDNSNRPSGVPDRFSGSKSGTSASLAISGLQSEDEADYYCASFSDELGAYVFGGGTKLTVLRTVAAPSVFIFPPSDEQLKSGTASVVCLLNNFYPREAKVQWKVDNALQSGNSQESVTEQDSKDSTYSLSSTLTLSKADYEKHKVYACEVTHQGLSSPVTKSFNRGEC

SEQ ID NO: 108 - DNA, 651 bp, Artificial Sequence
  IgG light chain 1
cagtctgtgctgactcagccaccctcagcgtctgggacccccgggcagagggtcaccatctcttgtactggctcttcatctaatattggcagtaattatgtcacctggtaccagcagctcccaggaacggcccccaaactcctcatctatgataatagtaatcggccaagcggggtccctgaccgattctctggctccaagtctggcacctcagcctccctggccatcagtgggctccagtccgaggatgaggctgattattactgtgcttcttttagtgatgagttgggggcttatgtcttcggcggaggcaccaagctgacggtcctacgtacggtggctgcaccatctgtcttcatcttcccgccatctgatgagcagttgaaatctggaactgcctctgttgtgtgcctgctgaataacttctatcccagagaggccaaagtacagtggaaggtggataacgccctccaatcgggtaactcccaggagagtgtcacagagcaggacagcaaggacagcacctacagcctcagcagcaccctgacgctgagcaaagcagactacgagaaacacaaagtctacgcctgcgaagtcacccatcagggcctgagctcgcccgtcacaaagagcttcaacaggggagagtgt

SEQ ID NO: 109 - protein, 217 aa, Artificial Sequence
  IgG light chain 2
QSVLTQPPSASGTPGQRVTISCTGSSSNIGSNYVTWYQQLPGTAPKLLIYDNSNRPSGVPDRFSGSKSGTSASLAISGLQSEDEADYYCSSFSDELGAYVFGGGTKLTVLRTVAAPSVFIFPPSDEQLKSGTASVVCLLNNFYPREAKVQWKVDNALQSGNSQESVTEQDSKDSTYSLSSTLTLSKADYEKHKVYACEVTHQGLSSPVTKSFNRGEC

SEQ ID NO: 110 - DNA, 651 bp, Artificial Sequence
  IgG light chain 2
cagtctgtgctgactcagccaccctcagcgtctgggacccccgggcagagggtcaccatctcttgtactggctcttcatctaatattggcagtaattatgtcacctggtaccagcagctcccaggaacggcccccaaactcctcatctatgataatagtaatcggccaagcggggtccctgaccgattctctggctccaagtctggcacctcagcctccctggccatcagtgggctccagtccgaggatgaggctgattattactgttcttcttttagtgatgagttgggggcttatgtcttcggcggaggcaccaagctgacggtcctacgtacggtggctgcaccatctgtcttcatcttcccgccatctgatgagcagttgaaatctggaactgcctctgttgtgtgcctgctgaataacttctatcccagagaggccaaagtacagtggaaggtggataacgccctccaatcgggtaactcccaggagagtgtcacagagcaggacagcaaggacagcacctacagcctcagcagcaccctgacgctgagcaaagcagactacgagaaacacaaagtctacgcctgcgaagtcacccatcagggcctgagctcgcccgtcacaaagagcttcaacaggggagagtgt

SEQ ID NO: 111 - protein, 216 aa, Artificial Sequence
  IgG light chain 3
QSVLTQPPSASGTPGQRVTISCTGSSSNIGSNYVTWYQQLPGTAPKLLIYDNSNRPSGVPDRFSGSKSGTSASLAISGLQSEDEADYYCSSFSDELGAYVFGGGTKLTVLGQPKAAPSVTLFPPSSEELQANKATLVCLISDFYPGAVTVAWKADSSPVKAGVETTTPSKQSNNKYAASSYLSLTPEQWKSHRSYSCQVTHEGSTVEKTVAPTECS

SEQ ID NO: 112 - DNA, 648 bp, Artificial Sequence
  IgG light chain 3
cagtctgtgctgactcagccaccctcagcgtctgggacccccgggcagagggtcaccatctcttgtactggctcttcatctaatattggcagtaattatgtcacctggtaccagcagctcccaggaacggcccccaaactcctcatctatgataatagtaatcggccaagcggggtccctgaccgattctctggctccaagtctggcacctcagcctccctggccatcagtgggctccagtccgaggatgaggctgattattactgttcttcttttagtgatgagttgggggcttatgtcttcggcggaggcaccaagctgacggtcctaggtcagcccaaggctgccccctcggtcacgctcttcccaccctcctctgaggagcttcaagccaacaaggccacactggtgtgtctcataagtgacttctacccgggagccgtgacagtggcctggaaggcagatagcagccccgtcaaggcgggagtggagaccaccacaccctccaaacaaagcaacaacaagtacgcggccagcagctacctgagcctgacgcctgagcagtggaagtcccacagaagctacagctgccaggtcacgcatgaagggagcaccgtggagaagacagtggcccctacagaatgctct

SEQ ID NO: 113 - protein, 216 aa, Artificial Sequence
  IgG light chain 4
QSVLTQPPSASGTPGQRVTISCTGSSSNIGSNYVTWYQQLPGTAPKLLIYSNNQRPSGVPDRFSGSKSGTSASLAISGLQSEDEADYYCSSFSDELGAYVFGGGTKLTVLGQPKAAPSVTLFPPSSEELQANKATLVCLISDFYPGAVTVAWKADSSPVKAGVETTTPSKQSNNKYAASSYLSLTPEQWKSHRSYSCQVTHEGSTVEKTVAPTECS

SEQ ID NO: 114 - DNA, 648 bp, Artificial Sequence
  IgG light chain 4
cagtctgtgctgactcagccaccctcagcgtctgggacccccgggcagagggtcaccatctcttgtactggctcttcatctaatattggcagtaattatgtcacctggtaccagcagctcccaggaacggcccccaaactcctcatctatagtaataatcagcggccaagcggggtccctgaccgattctctggctccaagtctggcacctcagcctccctggccatcagtgggctccagtccgaggatgaggctgattattactgttcttcttttagtgatgagttgggggcttatgtcttcggcggaggcaccaagctgacggtcctaagtcagcccaaggctgccccctcggtcacgctcttcccaccctcctctgaggagcttcaagccaacaaggccacactggtgtgtctcataagtgacttctacccgggagccgtgacagtggcctggaaggcagatagcagccccgtcaaggcgggagtggagaccaccacaccctccaaacaaagcaacaacaagtacgcggccagcagctacctgagcctgacgcctgagcagtggaagtcccacagaagctacagctgccaggtcacgcatgaagggagcaccgtggagaagacagtggcccctacagaatgctct

SEQ ID NO: 115 - protein, 216 aa, Artificial Sequence
  IgG light chain 5
QSVLTQPPSASGTPGQRVTISCTGSSSNIGSNYVTWYQQLPGTAPKLLIYRNNQRPSGVPDRFSGSKSGTSASLAISGLQSEDEADYYCSSFSDELGAYVFGGGTKLTVLGQPKAAPSVTLFPPSSEELQANKATLVCLISDFYPGAVTVAWKADSSPVKAGVETTTPSKQSNNKYAASSYLSLTPEQWKSHRSYSCQVTHEGSTVEKTVAPTECS

SEQ ID NO: 116 - DNA, 648 bp, Artificial Sequence
  IgG light chain 5
cagtctgtgctgactcagccaccctcagcgtctgggacccccgggcagagggtcaccatctcttgtactggctcttcatctaatattggcagtaattatgtcacctggtaccagcagctcccaggaacggcccccaaactcctcatctatcggaataatcagcggccaagcggggtccctgaccgattctctggctccaagtctggcacctcagcctccctggccatcagtgggctccagtccgaggatgaggctgattattactgttcttcttttagtgatgagttgggggcttatgtcttcggcggaggcaccaagctgacggtcctaggtcagcccaaggctgccccctcggtcacgctcttcccaccctcctctgaggagcttcaagccaacaaggccacactggtgtgtctcataagtgacttctacccgggagccgtgacagtggcctggaaggcagatagcagccccgtcaaggcgggagtggagaccaccacaccctccaaacaaagcaacaacaagtacgcggccagcagctacctgagcctgacgcctgagcagtggaagtcccacagaagctacagctgccaggtcacgcatgaagggagcaccgtggagaagacagtggcccctacagaatgctct

SEQ ID NO: 117 - protein, 28 aa, Artificial Sequence
  KRS epitope F4
EPKLSKNELKRRLKAEKKVAEKEAKQKE

SEQ ID NO: 118 - protein, 17 aa, Artificial Sequence
  CDR H2 mutant 5 amino acid
VISSDGGNTYYADSVKG

SEQ ID NO: 119 - DNA, 51 bp, Artificial Sequence
  CDR H2 mutant 5 DNA
gtgatctcttctgatggtggtaatacatattacgctgattctgtaaaaggt

SEQ ID NO: 120 - protein, 107 aa, Artificial Sequence [sequence omitted]

SEQ ID NO: 121 - DNA, 321 bp, Artificial Sequence
  light chain constant region ver.1_DNA
cgtacggtggctgcaccatctgtcttcatcttcccgccatctgatgagcagttgaaatctggaactgcctctgttgtgtgcctgctgaataacttctatcccagagaggccaaagtacagtggaaggtggataacgccctccaatcgggtaactcccaggagagtgtcacagagcaggacagcaaggacagcacctacagcctcagcagcaccctgacgctgagcaaagcagactacgagaaacacaaagtctacgcctgcgaagtcacccatcagggcctgagctcgcccgtcacaaagagcttcaacaggggagagtgt

SEQ ID NO: 122 - protein, 106 aa, Artificial Sequence
  light chain constant region ver.2_amino acid
GQPKAAPSVTLFPPSSEELQANKATLVCLISDFYPGAVTVAWKADSSPVKAGVETTTPSKQSNNKYAASSYLSLTPEQWKSHRSYSCQVTHEGSTVEKTVAPTECS

SEQ ID NO: 123 - DNA, 318 bp, Artificial Sequence
  light chain constant region ver.2_DNA
ggtcagcccaaggctgccccctcggtcacgctcttcccaccctcctctgaggagcttcaagccaacaaggccacactggtgtgtctcataagtgacttctacccgggagccgtgacagtggcctggaaggcagatagcagccccgtcaaggcgggagtggagaccaccacaccctccaaacaaagcaacaacaagtacgcggccagcagctacctgagcctgacgcctgagcagtggaagtcccacagaagctacagctgccaggtcacgcatgaagggagcaccgtggagaagacagtggcccctacagaatgctct

SEQ ID NO: 124 - protein, 330 aa, Artificial Sequence [sequence omitted]

SEQ ID NO: 125 - DNA, 990 bp, Artificial Sequence
  heavy chain constant region(CH1, CH2, CH3)_IgG1 wild type_DNA
gcctccaccaagggcccatcggtcttccccctggcaccctcctccaagagcacctctgggggcacagcggccctgggctgcctggtcaaggactacttccccgaaccggtgacggtgtcgtggaactcaggcgccctgaccagcggcgtgcacaccttcccggctgtcctacagtcctcaggactctactccctcagcagcgtggtgaccgtgccctccagcagcttgggcacccagacctacatctgcaacgtgaatcacaagcccagcaacaccaaggtggacaagaaagttgagcccaaatcttgtgacaaaactcacacatgcccaccgtgcccagcacctgaactcctggggggaccgtcagtcttcctcttccccccaaaacccaaggacaccctcatgatctcccggacccctgaggtcacatgcgtggtggtggacgtgagccacgaagaccctgaggtcaagttcaactggtacgtggacggcgtggaggtgcataatgccaagacaaagccgcgggaggagcagtacaacagcacgtaccgtgtggtcagcgtcctcaccgtcctgcaccaggactggctgaatggcaaggagtacaagtgcaaggtctccaacaaagccctcccagcccccatcgagaaaaccatctccaaagccaaagggcagccccgagaaccacaggtgtataccctgcccccatcccgggatgagctgaccaagaaccaggtcagcctgacctgcctggtcaaaggcttctatcccagcgacatcgccgtggagtgggagagcaatgggcagccggagaacaactacaagaccacgcctcccgtgctggactccgacggctccttcttcctctacagcaagctcaccgtggacaagagcaggtggcagcaggggaacgtcttctcatgctccgtgatgcatgaggctctgcacaaccactacacgcagaagagcctctccctgtccccgggtaaa

SEQ ID NO: 126 - protein, 330 aa, Artificial Sequence
  heavy chain constant region(CH1, CH2, CH3)_IgG1 mutant TA_amino acid
ASTKGPSVFPLAPSSKSTSGGTAALGCLVKDYFPEPVTVSWNSGALTSGVHTFPAVLQSSGLYSLSSVVTVPSSSLGTQTYICNVNHKPSNTKVDKKVEPKSCDKTHTCPPCPAPELLGGPSVFLFPPKPKDTLMISRTPEVTCVVVDVSHEDPEVKFNWYVDGVEVHNAKTKPREEQYNSAYRVVSVLTVLHQDWLNGKEYKCKVSNKALPAPIEKTISKAKGQPREPQVYTLPPSRDELTKNQVSLTCLVKGFYPSDIAVEWESNGQPENNYKTTPPVLDSDGSFFLYSKLTVDKSRWQQGNVFSCSVMHEALHNHYTQKSLSLSPGK

SEQ ID NO: 127 - DNA, 990 bp, Artificial Sequence
  heavy chain constant region(CH1, CH2, CH3)_IgG1 mutant TA_DNA
gcctccaccaagggcccatcggtcttccccctggcaccctcctccaagagcacctctgggggcacagcggccctgggctgcctggtcaaggactacttccccgaaccggtgacggtgtcgtggaactcaggcgccctgaccagcggcgtgcacaccttcccggctgtcctacagtcctcaggactctactccctcagcagcgtggtgaccgtgccctccagcagcttgggcacccagacctacatctgcaacgtgaatcacaagcccagcaacaccaaggtggacaagaaagttgagcccaaatcttgtgacaaaactcacacatgcccaccgtgcccagcacctgaactcctggggggaccgtcagtcttcctcttccccccaaaacccaaggacaccctcatgatctcccggacccctgaggtcacatgcgtggtggtggacgtgagccacgaagaccctgaggtcaagttcaactggtacgtggacggcgtggaggtgcataatgccaagacaaagccgcgggaggagcagtacaacagcgcctaccgtgtggtcagcgtcctcaccgtcctgcaccaggactggctgaatggcaaggagtacaagtgcaaggtctccaacaaagccctcccagcccccatcgagaaaaccatctccaaagccaaagggcagccccgagaaccacaggtgtataccctgcccccatcccgggatgagctgaccaagaaccaggtcagcctgacctgcctggtcaaaggcttctatcccagcgacatcgccgtggagtgggagagcaatgggcagccggagaacaactacaagaccacgcctcccgtgctggactccgacggctccttcttcctctacagcaagctcaccgtggacaagagcaggtggcagcaggggaacgtcttctcatgctccgtgatgcatgaggctctgcacaaccactacacgcagaagagcctctccctgtccccgggtaaa

SEQ ID NO: 128 - protein, 330 aa, Artificial Sequence
  heavy chain constant region(CH1, CH2, CH3)_IgG1 mutant LALA_amino acid
ASTKGPSVFPLAPSSKSTSGGTAALGCLVKDYFPEPVTVSWNSGALTSGVHTFPAVLQSSGLYSLSSVVTVPSSSLGTQTYICNVNHKPSNTKVDKKVEPKSCDKTHTCPPCPAPEAAGGPSVFLFPPKPKDTLMISRTPEVTCVVVDVSHEDPEVKFNWYVDGVEVHNAKTKPREEQYNSTYRVVSVLTVLHQDWLNGKEYKCKVSNKALPAPIEKTISKAKGQPREPQVYTLPPSRDELTKNQVSLTCLVKGFYPSDIAVEWESNGQPENNYKTTPPVLDSDGSFFLYSKLTVDKSRWQQGNVFSCSVMHEALHNHYTQKSLSLSPGK

SEQ ID NO: 129 - DNA, 990 bp, Artificial Sequence
  heavy chain constant region(CH1, CH2, CH3)_IgG1 mutant LALA_DNA
gcctccaccaagggcccatcggtcttccccctggcaccctcctccaagagcacctctgggggcacagcggccctgggctgcctggtcaaggactacttccccgaaccggtgacggtgtcgtggaactcaggcgccctgaccagcggcgtgcacaccttcccggctgtcctacagtcctcaggactctactccctcagcagcgtggtgaccgtgccctccagcagcttgggcacccagacctacatctgcaacgtgaatcacaagcccagcaacaccaaggtggacaagaaagttgagcccaaatcttgtgacaaaactcacacatgcccaccgtgcccagcacctgaagccgccgggggaccgtcagtcttcctcttccccccaaaacccaaggacaccctcatgatctcccggacccctgaggtcacatgcgtggtggtggacgtgagccacgaagaccctgaggtcaagttcaactggtacgtggacggcgtggaggtgcataatgccaagacaaagccgcgggaggagcagtacaacagcacgtaccgtgtggtcagcgtcctcaccgtcctgcaccaggactggctgaatggcaaggagtacaagtgcaaggtctccaacaaagccctcccagcccccatcgagaaaaccatctccaaagccaaagggcagccccgagaaccacaggtgtataccctgcccccatcccgggatgagctgaccaagaaccaggtcagcctgacctgcctggtcaaaggcttctatcccagcgacatcgccgtggagtgggagagcaatgggcagccggagaacaactacaagaccacgcctcccgtgctggactccgacggctccttcttcctctacagcaagctcaccgtggacaagagcaggtggcagcaggggaacgtcttctcatgctccgtgatgcatgaggctctgcacaaccactacacgcagaagagcctctccctgtccccgggtaaa

SEQ ID NO: 130 - protein, 330 aa, Artificial Sequence
  heavy chain constant region(CH1, CH2, CH3)_IgG1 mutant LALATA_amino acid
ASTKGPSVFPLAPSSKSTSGGTAALGCLVKDYFPEPVTVSWNSGALTSGVHTFPAVLQSSGLYSLSSVVTVPSSSLGTQTYICNVNHKPSNTKVDKKVEPKSCDKTHTCPPCPAPEAAGGPSVFLFPPKPKDTLMISRTPEVTCVVVDVSHEDPEVKFNWYVDGVEVHNAKTKPREEQYNSAYRVVSVLTVLHQDWLNGKEYKCKVSNKALPAPIEKTISKAKGQPREPQVYTLPPSRDELTKNQVSLTCLVKGFYPSDIAVEWESNGQPENNYKTTPPVLDSDGSFFLYSKLTVDKSRWQQGNVFSCSVMHEALHNHYTQKSLSLSPGK

SEQ ID NO: 131 - DNA, 990 bp, Artificial Sequence
  heavy chain constant region(CH1, CH2, CH3)_IgG1 mutant LALATA_DNA
gcctccaccaagggcccatcggtcttccccctggcaccctcctccaagagcacctctgggggcacagcggccctgggctgcctggtcaaggactacttccccgaaccggtgacggtgtcgtggaactcaggcgccctgaccagcggcgtgcacaccttcccggctgtcctacagtcctcaggactctactccctcagcagcgtggtgaccgtgccctccagcagcttgggcacccagacctacatctgcaacgtgaatcacaagcccagcaacaccaaggtggacaagaaagttgagcccaaatcttgtgacaaaactcacacatgcccaccgtgcccagcacctgaagccgccgggggaccgtcagtcttcctcttccccccaaaacccaaggacaccctcatgatctcccggacccctgaggtcacatgcgtggtggtggacgtgagccacgaagaccctgaggtcaagttcaactggtacgtggacggcgtggaggtgcataatgccaagacaaagccgcgggaggagcagtacaacagcgcctaccgtgtggtcagcgtcctcaccgtcctgcaccaggactggctgaatggcaaggagtacaagtgcaaggtctccaacaaagccctcccagcccccatcgagaaaaccatctccaaagccaaagggcagccccgagaaccacaggtgtataccctgcccccatcccgggatgagctgaccaagaaccaggtcagcctgacctgcctggtcaaaggcttctatcccagcgacatcgccgtggagtgggagagcaatgggcagccggagaacaactacaagaccacgcctcccgtgctggactccgacggctccttcttcctctacagcaagctcaccgtggacaagagcaggtggcagcaggggaacgtcttctcatgctccgtgatgcatgaggctctgcacaaccactacacgcagaagagcctctccctgtccccgggtaaa

SEQ ID NO: 132 - protein, 330 aa, Artificial Sequence
  heavy chain constant region(CH1, CH2, CH3)_IgG1 mutant LALAPG_amino acid
ASTKGPSVFPLAPSSKSTSGGTAALGCLVKDYFPEPVTVSWNSGALTSGVHTFPAVLQSSGLYSLSSVVTVPSSSLGTQTYICNVNHKPSNTKVDKKVEPKSCDKTHTCPPCPAPEAAGGPSVFLFPPKPKDTLMISRTPEVTCVVVDVSHEDPEVKFNWYVDGVEVHNAKTKPREEQYNSTYRVVSVLTVLHQDWLNGKEYKCKVSNKALGAPIEKTISKAKGQPREPQVYTLPPSRDELTKNQVSLTCLVKGFYPSDIAVEWESNGQPENNYKTTPPVLDSDGSFFLYSKLTVDKSRWQQGNVFSCSVMHEALHNHYTQKSLSLSPGK

SEQ ID NO: 133 - DNA, 990 bp, Artificial Sequence
  heavy chain constant region(CH1, CH2, CH3)_IgG1 mutant LALAPG_DNA
gcctccaccaagggcccatcggtcttccccctggcaccctcctccaagagcacctctgggggcacagcggccctgggctgcctggtcaaggactacttccccgaaccggtgacggtgtcgtggaactcaggcgccctgaccagcggcgtgcacaccttcccggctgtcctacagtcctcaggactctactccctcagcagcgtggtgaccgtgccctccagcagcttgggcacccagacctacatctgcaacgtgaatcacaagcccagcaacaccaaggtggacaagaaagttgagcccaaatcttgtgacaaaactcacacatgcccaccgtgcccagcacctgaagccgccgggggaccgtcagtcttcctcttccccccaaaacccaaggacaccctcatgatctcccggacccctgaggtcacatgcgtggtggtggacgtgagccacgaagaccctgaggtcaagttcaactggtacgtggacggcgtggaggtgcataatgccaagacaaagccgcgggaggagcagtacaacagcacgtaccgtgtggtcagcgtcctcaccgtcctgcaccaggactggctgaatggcaaggagtacaagtgcaaggtctccaacaaagccctcggcgcccccatcgagaaaaccatctccaaagccaaagggcagccccgagaaccacaggtgtataccctgcccccatcccgggatgagctgaccaagaaccaggtcagcctgacctgcctggtcaaaggcttctatcccagcgacatcgccgtggagtgggagagcaatgggcagccggagaacaactacaagaccacgcctcccgtgctggactccgacggctccttcttcctctacagcaagctcaccgtggacaagagcaggtggcagcaggggaacgtcttctcatgctccgtgatgcatgaggctctgcacaaccactacacgcagaagagcctctccctgtccccgggtaaa

SEQ ID NO: 134 - protein, 330 aa, Artificial Sequence
  heavy chain constant region(CH1, CH2, CH3)_IgG1 mutant LALAPGTA_amino acid
ASTKGPSVFPLAPSSKSTSGGTAALGCLVKDYFPEPVTVSWNSGALTSGVHTFPAVLQSSGLYSLSSVVTVPSSSLGTQTYICNVNHKPSNTKVDKKVEPKSCDKTHTCPPCPAPEAAGGPSVFLFPPKPKDTLMISRTPEVTCVVVDVSHEDPEVKFNWYVDGVEVHNAKTKPREEQYNSAYRVVSVLTVLHQDWLNGKEYKCKVSNKALGAPIEKTISKAKGQPREPQVYTLPPSRDELTKNQVSLTCLVKGFYPSDIAVEWESNGQPENNYKTTPPVLDSDGSFFLYSKLTVDKSRWQQGNVFSCSVMHEALHNHYTQKSLSLSPGK

SEQ ID NO: 135 - DNA, 990 bp, Artificial Sequence
  heavy chain constant region(CH1, CH2, CH3)_IgG1 mutant LALAPGTA_DNA
gcctccaccaagggcccatcggtcttccccctggcaccctcctccaagagcacctctgggggcacagcggccctgggctgcctggtcaaggactacttccccgaaccggtgacggtgtcgtggaactcaggcgccctgaccagcggcgtgcacaccttcccggctgtcctacagtcctcaggactctactccctcagcagcgtggtgaccgtgccctccagcagcttgggcacccagacctacatctgcaacgtgaatcacaagcccagcaacaccaaggtggacaagaaagttgagcccaaatcttgtgacaaaactcacacatgcccaccgtgcccagcacctgaagccgccgggggaccgtcagtcttcctcttccccccaaaacccaaggacaccctcatgatctcccggacccctgaggtcacatgcgtggtggtggacgtgagccacgaagaccctgaggtcaagttcaactggtacgtggacggcgtggaggtgcataatgccaagacaaagccgcgggaggagcagtacaacagcgcctaccgtgtggtcagcgtcctcaccgtcctgcaccaggactggctgaatggcaaggagtacaagtgcaaggtctccaacaaagccctcggcgcccccatcgagaaaaccatctccaaagccaaagggcagccccgagaaccacaggtgtataccctgcccccatcccgggatgagctgaccaagaaccaggtcagcctgacctgcctggtcaaaggcttctatcccagcgacatcgccgtggagtgggagagcaatgggcagccggagaacaactacaagaccacgcctcccgtgctggactccgacggctccttcttcctctacagcaagctcaccgtggacaagagcaggtggcagcaggggaacgtcttctcatgctccgtgatgcatgaggctctgcacaaccactacacgcagaagagcctctccctgtccccgggtaaa

SEQ ID NO: 136 - protein, 327 aa, Artificial Sequence
  heavy chain constant region(CH1, CH2, CH3)_IgG4 wild type_amino acid
ASTKGPSVFPLAPCSRSTSESTAALGCLVKDYFPEPVTVSWNSGALTSGVHTFPAVLQSSGLYSLSSVVTVPSSSLGTKTYTCNVDHKPSNTKVDKRVESKYGPPCPSCPAPEFLGGPSVFLFPPKPKDTLMISRTPEVTCVVVDVSQEDPEVQFNWYVDGVEVHNAKTKPREEQFNSTYRVVSVLTVLHQDWLNGKEYKCKVSNKGLPSSIEKTISKAKGQPREPQVYTLPPSQEEMTKNQVSLTCLVKGFYPSDIAVEWESNGQPENNYKTTPPVLDSDGSFFLYSRLTVDKSRWQEGNVFSCSVMHEALHNHYTQKSLSLSLGK

SEQ ID NO: 137 - DNA, 981 bp, Artificial Sequence
  heavy chain constant region(CH1, CH2, CH3)_IgG4 wild type_DNA
gccagcaccaagggcccttccgtgtttcccctggccccttgctcccggtccacatctgagagcaccgccgccctgggctgtctggtgaaggactacttcccagagcccgtgaccgtgagctggaacagcggcgccctgacaagcggcgtgcacacatttcccgccgtgctgcagagctccggcctgtactccctgtctagcgtggtgacagtgccttcctctagcctgggcaccaagacatatacctgtaacgtggaccacaagccaagcaataccaaggtggataagcgggtggagtctaagtacggccctccttgccctagctgtcctgctccagagtttctgggcggcccttccgtgttcctgtttccacccaaaccaaaggacacactgatgatctctagaacaccagaggtgacctgcgtggtggtggacgtgagccaggaggatcccgaggtgcagttcaactggtacgtggatggcgtggaggtgcacaatgccaagaccaagccaagagaggagcagtttaactctacatacagggtggtgagcgtgctgaccgtgctgcaccaggattggctcaacggcaaggagtataagtgcaaggtgtccaataagggcctgccctcctctatcgagaagacaatctctaaggctaagggccagccaagagagcctcaggtgtacaccctgcctccaagccaggaggagatgacaaagaaccaggtgtccctgacatgtctggtgaagggcttctatccctccgacatcgccgtggagtgggagtctaatggccagcctgagaacaattacaagaccacaccccctgtgctggactctgatggcagcttctttctgtattccaggctgaccgtggataagtctcggtggcaggagggcaacgtgttcagctgctctgtgatgcacgaagccctgcataatcactatactcagaaaagtctgtcactgtcactgggaaag

SEQ ID NO: 138 - protein, 327 aa, Artificial Sequence
  heavy chain constant region(CH1, CH2, CH3)_IgG4 mutant TA_amino acid
ASTKGPSVFPLAPCSRSTSESTAALGCLVKDYFPEPVTVSWNSGALTSGVHTFPAVLQSSGLYSLSSVVTVPSSSLGTKTYTCNVDHKPSNTKVDKRVESKYGPPCPSCPAPEFLGGPSVFLFPPKPKDTLMISRTPEVTCVVVDVSQEDPEVQFNWYVDGVEVHNAKTKPREEQFNSAYRVVSVLTVLHQDWLNGKEYKCKVSNKGLPSSIEKTISKAKGQPREPQVYTLPPSQEEMTKNQVSLTCLVKGFYPSDIAVEWESNGQPENNYKTTPPVLDSDGSFFLYSRLTVDKSRWQEGNVFSCSVMHEALHNHYTQKSLSLSLGK

SEQ ID NO: 139 - DNA, 981 bp, Artificial Sequence
  heavy chain constant region(CH1, CH2, CH3)_IgG4 mutant TA_DNA
gccagcaccaagggcccttccgtgtttcccctggccccttgctcccggtccacatctgagagcaccgccgccctgggctgtctggtgaaggactacttcccagagcccgtgaccgtgagctggaacagcggcgccctgacaagcggcgtgcacacatttcccgccgtgctgcagagctccggcctgtactccctgtctagcgtggtgacagtgccttcctctagcctgggcaccaagacatatacctgtaacgtggaccacaagccaagcaataccaaggtggataagcgggtggagtctaagtacggccctccttgccctagctgtcctgctccagagtttctgggcggcccttccgtgttcctgtttccacccaaaccaaaggacacactgatgatctctagaacaccagaggtgacctgcgtggtggtggacgtgagccaggaggatcccgaggtgcagttcaactggtacgtggatggcgtggaggtgcacaatgccaagaccaagccaagagaggagcagtttaactctgcctacagggtggtgagcgtgctgaccgtgctgcaccaggattggctcaacggcaaggagtataagtgcaaggtgtccaataagggcctgccctcctctatcgagaagacaatctctaaggctaagggccagccaagagagcctcaggtgtacaccctgcctccaagccaggaggagatgacaaagaaccaggtgtccctgacatgtctggtgaagggcttctatccctccgacatcgccgtggagtgggagtctaatggccagcctgagaacaattacaagaccacaccccctgtgctggactctgatggcagcttctttctgtattccaggctgaccgtggataagtctcggtggcaggagggcaacgtgttcagctgctctgtgatgcacgaagccctgcataatcactatactcagaaaagtctgtcactgtcactgggaaag

SEQ ID NO: 140 - protein, 446 aa, Artificial Sequence
  IgG heavy chain_IgG1 mutant TA_amino acid
EVQLLESGGGLVQPGGSLRLSCAASGFTFSSYDMSWVRQAPGKGLEWVSAISYDNGNTYYADSVKGRFTISRDNSKNTLYLQMNSLRAEDTAVYYSARMALDFDYWGQGTLVTVSSASTKGPSVFPLAPSSKSTSGGTAALGCLVKDYFPEPVTVSWNSGALTSGVHTFPAVLQSSGLYSLSSVVTVPSSSLGTQTYICNVNHKPSNTKVDKKVEPKSCDKTHTCPPCPAPELLGGPSVFLFPPKPKDTLMISRTPEVTCVVVDVSHEDPEVKFNWYVDGVEVHNAKTKPREEQYNSAYRVVSVLTVLHQDWLNGKEYKCKVSNKALPAPIEKTISKAKGQPREPQVYTLPPSRDELTKNQVSLTCLVKGFYPSDIAVEWESNGQPENNYKTTPPVLDSDGSFFLYSKLTVDKSRWQQGNVFSCSVMHEALHNHYTQKSLSLSPGK

SEQ ID NO: 141 - DNA, 1338 bp, Artificial Sequence
  IgG heavy chain_IgG1 mutant TA_DNA
gaggtgcagctgttggagtctgggggaggcttggtacagcctggggggtccctgagactctcctgtgcagcctctggattcacctttagcagttatgatatgagctgggtccgccaggctccagggaaggggctggagtgggtctcagcgatctcttatgataatggtaatacatattacgctgattctgtaaaaggtcggttcaccatctccagagacaattccaagaacacgctgtatctgcaaatgaacagcctgagagccgaggacacggccgtgtattactctgcgagaatggcgcttgatttcgactactggggccagggtacactggtcaccgtgagctcagcctccaccaagggcccatcggtcttccccctggcaccctcctccaagagcacctctgggggcacagcggccctgggctgcctggtcaaggactacttccccgaaccggtgacggtgtcgtggaactcaggcgccctgaccagcggcgtgcacaccttcccggctgtcctacagtcctcaggactctactccctcagcagcgtggtgaccgtgccctccagcagcttgggcacccagacctacatctgcaacgtgaatcacaagcccagcaacaccaaggtggacaagaaagttgagcccaaatcttgtgacaaaactcacacatgcccaccgtgcccagcacctgaactcctggggggaccgtcagtcttcctcttccccccaaaacccaaggacaccctcatgatctcccggacccctgaggtcacatgcgtggtggtggacgtgagccacgaagaccctgaggtcaagttcaactggtacgtggacggcgtggaggtgcataatgccaagacaaagccgcgggaggagcagtacaacagcgcctaccgtgtggtcagcgtcctcaccgtcctgcaccaggactggctgaatggcaaggagtacaagtgcaaggtctccaacaaagccctcccagcccccatcgagaaaaccatctccaaagccaaagggcagccccgagaaccacaggtgtataccctgcccccatcccgggatgagctgaccaagaaccaggtcagcctgacctgcctggtcaaaggcttctatcccagcgacatcgccgtggagtgggagagcaatgggcagccggagaacaactacaagaccacgcctcccgtgctggactccgacggctccttcttcctctacagcaagctcaccgtggacaagagcaggtggcagcaggggaacgtcttctcatgctccgtgatgcatgaggctctgcacaaccactacacgcagaagagcctctccctgtccccgggtaaa

SEQ ID NO: 142 - protein, 446 aa, Artificial Sequence
  IgG heavy chain_IgG1 mutant LALA_amino acid
EVQLLESGGGLVQPGGSLRLSCAASGFTFSSYDMSWVRQAPGKGLEWVSAISYDNGNTYYADSVKGRFTISRDNSKNTLYLQMNSLRAEDTAVYYSARMALDFDYWGQGTLVTVSSASTKGPSVFPLAPSSKSTSGGTAALGCLVKDYFPEPVTVSWNSGALTSGVHTFPAVLQSSGLYSLSSVVTVPSSSLGTQTYICNVNHKPSNTKVDKKVEPKSCDKTHTCPPCPAPEAAGGPSVFLFPPKPKDTLMISRTPEVTCVVVDVSHEDPEVKFNWYVDGVEVHNAKTKPREEQYNSTYRVVSVLTVLHQDWLNGKEYKCKVSNKALPAPIEKTISKAKGQPREPQVYTLPPSRDELTKNQVSLTCLVKGFYPSDIAVEWESNGQPENNYKTTPPVLDSDGSFFLYSKLTVDKSRWQQGNVFSCSVMHEALHNHYTQKSLSLSPGK

SEQ ID NO: 143 - DNA, 1338 bp, Artificial Sequence
  IgG heavy chain_IgG1 mutant LALA_DNA
gaggtgcagctgttggagtctgggggaggcttggtacagcctggggggtccctgagactctcctgtgcagcctctggattcacctttagcagttatgatatgagctgggtccgccaggctccagggaaggggctggagtgggtctcagcgatctcttatgataatggtaatacatattacgctgattctgtaaaaggtcggttcaccatctccagagacaattccaagaacacgctgtatctgcaaatgaacagcctgagagccgaggacacggccgtgtattactctgcgagaatggcgcttgatttcgactactggggccagggtacactggtcaccgtgagctcagcctccaccaagggcccatcggtcttccccctggcaccctcctccaagagcacctctgggggcacagcggccctgggctgcctggtcaaggactacttccccgaaccggtgacggtgtcgtggaactcaggcgccctgaccagcggcgtgcacaccttcccggctgtcctacagtcctcaggactctactccctcagcagcgtggtgaccgtgccctccagcagcttgggcacccagacctacatctgcaacgtgaatcacaagcccagcaacaccaaggtggacaagaaagttgagcccaaatcttgtgacaaaactcacacatgcccaccgtgcccagcacctgaagccgccgggggaccgtcagtcttcctcttccccccaaaacccaaggacaccctcatgatctcccggacccctgaggtcacatgcgtggtggtggacgtgagccacgaagaccctgaggtcaagttcaactggtacgtggacggcgtggaggtgcataatgccaagacaaagccgcgggaggagcagtacaacagcacgtaccgtgtggtcagcgtcctcaccgtcctgcaccaggactggctgaatggcaaggagtacaagtgcaaggtctccaacaaagccctcccagcccccatcgagaaaaccatctccaaagccaaagggcagccccgagaaccacaggtgtataccctgcccccatcccgggatgagctgaccaagaaccaggtcagcctgacctgcctggtcaaaggcttctatcccagcgacatcgccgtggagtgggagagcaatgggcagccggagaacaactacaagaccacgcctcccgtgctggactccgacggctccttcttcctctacagcaagctcaccgtggacaagagcaggtggcagcaggggaacgtcttctcatgctccgtgatgcatgaggctctgcacaaccactacacgcagaagagcctctccctgtccccgggtaaa

SEQ ID NO: 144 - protein, 446 aa, Artificial Sequence
  IgG heavy chain_IgG1 mutant LALATA_amino acid
EVQLLESGGGLVQPGGSLRLSCAASGFTFSSYDMSWVRQAPGKGLEWVSAISYDNGNTYYADSVKGRFTISRDNSKNTLYLQMNSLRAEDTAVYYSARMALDFDYWGQGTLVTVSSASTKGPSVFPLAPSSKSTSGGTAALGCLVKDYFPEPVTVSWNSGALTSGVHTFPAVLQSSGLYSLSSVVTVPSSSLGTQTYICNVNHKPSNTKVDKKVEPKSCDKTHTCPPCPAPEAAGGPSVFLFPPKPKDTLMISRTPEVTCVVVDVSHEDPEVKFNWYVDGVEVHNAKTKPREEQYNSAYRVVSVLTVLHQDWLNGKEYKCKVSNKALPAPIEKTISKAKGQPREPQVYTLPPSRDELTKNQVSLTCLVKGFYPSDIAVEWESNGQPENNYKTTPPVLDSDGSFFLYSKLTVDKSRWQQGNVFSCSVMHEALHNHYTQKSLSLSPGK

SEQ ID NO: 145 - DNA, 1338 bp, Artificial Sequence
  IgG heavy chain_IgG1 mutant LALATA_DNA
gaggtgcagctgttggagtctgggggaggcttggtacagcctggggggtccctgagactctcctgtgcagcctctggattcacctttagcagttatgatatgagctgggtccgccaggctccagggaaggggctggagtgggtctcagcgatctcttatgataatggtaatacatattacgctgattctgtaaaaggtcggttcaccatctccagagacaattccaagaacacgctgtatctgcaaatgaacagcctgagagccgaggacacggccgtgtattactctgcgagaatggcgcttgatttcgactactggggccagggtacactggtcaccgtgagctcagcctccaccaagggcccatcggtcttccccctggcaccctcctccaagagcacctctgggggcacagcggccctgggctgcctggtcaaggactacttccccgaaccggtgacggtgtcgtggaactcaggcgccctgaccagcggcgtgcacaccttcccggctgtcctacagtcctcaggactctactccctcagcagcgtggtgaccgtgccctccagcagcttgggcacccagacctacatctgcaacgtgaatcacaagcccagcaacaccaaggtggacaagaaagttgagcccaaatcttgtgacaaaactcacacatgcccaccgtgcccagcacctgaagccgccgggggaccgtcagtcttcctcttccccccaaaacccaaggacaccctcatgatctcccggacccctgaggtcacatgcgtggtggtggacgtgagccacgaagaccctgaggtcaagttcaactggtacgtggacggcgtggaggtgcataatgccaagacaaagccgcgggaggagcagtacaacagcgcctaccgtgtggtcagcgtcctcaccgtcctgcaccaggactggctgaatggcaaggagtacaagtgcaaggtctccaacaaagccctcccagcccccatcgagaaaaccatctccaaagccaaagggcagccccgagaaccacaggtgtataccctgcccccatcccgggatgagctgaccaagaaccaggtcagcctgacctgcctggtcaaaggcttctatcccagcgacatcgccgtggagtgggagagcaatgggcagccggagaacaactacaagaccacgcctcccgtgctggactccgacggctccttcttcctctacagcaagctcaccgtggacaagagcaggtggcagcaggggaacgtcttctcatgctccgtgatgcatgaggctctgcacaaccactacacgcagaagagcctctccctgtccccgggtaaa

SEQ ID NO: 146 - protein, 446 aa, Artificial Sequence
  IgG heavy chain_IgG1 mutant LALAPG_amino acid
EVQLLESGGGLVQPGGSLRLSCAASGFTFSSYDMSWVRQAPGKGLEWVSAISYDNGNTYYADSVKGRFTISRDNSKNTLYLQMNSLRAEDTAVYYSARMALDFDYWGQGTLVTVSSASTKGPSVFPLAPSSKSTSGGTAALGCLVKDYFPEPVTVSWNSGALTSGVHTFPAVLQSSGLYSLSSVVTVPSSSLGTQTYICNVNHKPSNTKVDKKVEPKSCDKTHTCPPCPAPEAAGGPSVFLFPPKPKDTLMISRTPEVTCVVVDVSHEDPEVKFNWYVDGVEVHNAKTKPREEQYNSTYRVVSVLTVLHQDWLNGKEYKCKVSNKALGAPIEKTISKAKGQPREPQVYTLPPSRDELTKNQVSLTCLVKGFYPSDIAVEWESNGQPENNYKTTPPVLDSDGSFFLYSKLTVDKSRWQQGNVFSCSVMHEALHNHYTQKSLSLSPGK

SEQ ID NO: 147 - DNA, 1338 bp, Artificial Sequence
  IgG heavy chain_IgG1 mutant LALAPG_DNA
gaggtgcagctgttggagtctgggggaggcttggtacagcctggggggtccctgagactctcctgtgcagcctctggattcacctttagcagttatgatatgagctgggtccgccaggctccagggaaggggctggagtgggtctcagcgatctcttatgataatggtaatacatattacgctgattctgtaaaaggtcggttcaccatctccagagacaattccaagaacacgctgtatctgcaaatgaacagcctgagagccgaggacacggccgtgtattactctgcgagaatggcgcttgatttcgactactggggccagggtacactggtcaccgtgagctcagcctccaccaagggcccatcggtcttccccctggcaccctcctccaagagcacctctgggggcacagcggccctgggctgcctggtcaaggactacttccccgaaccggtgacggtgtcgtggaactcaggcgccctgaccagcggcgtgcacaccttcccggctgtcctacagtcctcaggactctactccctcagcagcgtggtgaccgtgccctccagcagcttgggcacccagacctacatctgcaacgtgaatcacaagcccagcaacaccaaggtggacaagaaagttgagcccaaatcttgtgacaaaactcacacatgcccaccgtgcccagcacctgaagccgccgggggaccgtcagtcttcctcttccccccaaaacccaaggacaccctcatgatctcccggacccctgaggtcacatgcgtggtggtggacgtgagccacgaagaccctgaggtcaagttcaactggtacgtggacggcgtggaggtgcataatgccaagacaaagccgcgggaggagcagtacaacagcacgtaccgtgtggtcagcgtcctcaccgtcctgcaccaggactggctgaatggcaaggagtacaagtgcaaggtctccaacaaagccctcggcgcccccatcgagaaaaccatctccaaagccaaagggcagccccgagaaccacaggtgtataccctgcccccatcccgggatgagctgaccaagaaccaggtcagcctgacctgcctggtcaaaggcttctatcccagcgacatcgccgtggagtgggagagcaatgggcagccggagaacaactacaagaccacgcctcccgtgctggactccgacggctccttcttcctctacagcaagctcaccgtggacaagagcaggtggcagcaggggaacgtcttctcatgctccgtgatgcatgaggctctgcacaaccactacacgcagaagagcctctccctgtccccgggtaaa

SEQ ID NO: 148 - protein, 446 aa, Artificial Sequence
  IgG heavy chain_IgG1 mutant LALAPGTA_amino acid
EVQLLESGGGLVQPGGSLRLSCAASGFTFSSYDMSWVRQAPGKGLEWVSAISYDNGNTYYADSVKGRFTISRDNSKNTLYLQMNSLRAEDTAVYYSARMALDFDYWGQGTLVTVSSASTKGPSVFPLAPSSKSTSGGTAALGCLVKDYFPEPVTVSWNSGALTSGVHTFPAVLQSSGLYSLSSVVTVPSSSLGTQTYICNVNHKPSNTKVDKKVEPKSCDKTHTCPPCPAPEAAGGPSVFLFPPKPKDTLMISRTPEVTCVVVDVSHEDPEVKFNWYVDGVEVHNAKTKPREEQYNSAYRVVSVLTVLHQDWLNGKEYKCKVSNKALGAPIEKTISKAKGQPREPQVYTLPPSRDELTKNQVSLTCLVKGFYPSDIAVEWESNGQPENNYKTTPPVLDSDGSFFLYSKLTVDKSRWQQGNVFSCSVMHEALHNHYTQKSLSLSPGK

SEQ ID NO: 149 - DNA, 1338 bp, Artificial Sequence
  IgG heavy chain_IgG1 mutant LALAPGTA_DNA
gaggtgcagctgttggagtctgggggaggcttggtacagcctggggggtccctgagactctcctgtgcagcctctggattcacctttagcagttatgatatgagctgggtccgccaggctccagggaaggggctggagtgggtctcagcgatctcttatgataatggtaatacatattacgctgattctgtaaaaggtcggttcaccatctccagagacaattccaagaacacgctgtatctgcaaatgaacagcctgagagccgaggacacggccgtgtattactctgcgagaatggcgcttgatttcgactactggggccagggtacactggtcaccgtgagctcagcctccaccaagggcccatcggtcttccccctggcaccctcctccaagagcacctctgggggcacagcggccctgggctgcctggtcaaggactacttccccgaaccggtgacggtgtcgtggaactcaggcgccctgaccagcggcgtgcacaccttcccggctgtcctacagtcctcaggactctactccctcagcagcgtggtgaccgtgccctccagcagcttgggcacccagacctacatctgcaacgtgaatcacaagcccagcaacaccaaggtggacaagaaagttgagcccaaatcttgtgacaaaactcacacatgcccaccgtgcccagcacctgaagccgccgggggaccgtcagtcttcctcttccccccaaaacccaaggacaccctcatgatctcccggacccctgaggtcacatgcgtggtggtggacgtgagccacgaagaccctgaggtcaagttcaactggtacgtggacggcgtggaggtgcataatgccaagacaaagccgcgggaggagcagtacaacagcgcctaccgtgtggtcagcgtcctcaccgtcctgcaccaggactggctgaatggcaaggagtacaagtgcaaggtctccaacaaagccctcggcgcccccatcgagaaaaccatctccaaagccaaagggcagccccgagaaccacaggtgtataccctgcccccatcccgggatgagctgaccaagaaccaggtcagcctgacctgcctggtcaaaggcttctatcccagcgacatcgccgtggagtgggagagcaatgggcagccggagaacaactacaagaccacgcctcccgtgctggactccgacggctccttcttcctctacagcaagctcaccgtggacaagagcaggtggcagcaggggaacgtcttctcatgctccgtgatgcatgaggctctgcacaaccactacacgcagaagagcctctccctgtccccgggtaaa

SEQ ID NO: 150 - protein, 443 aa, Artificial Sequence
  IgG heavy chain_IgG4 wild type_amino acid
EVQLLESGGGLVQPGGSLRLSCAASGFTFSSYDMSWVRQAPGKGLEWVSAISYDNGNTYYADSVKGRFTISRDNSKNTLYLQMNSLRAEDTAVYYSARMALDFDYWGQGTLVTVSSASTKGPSVFPLAPCSRSTSESTAALGCLVKDYFPEPVTVSWNSGALTSGVHTFPAVLQSSGLYSLSSVVTVPSSSLGTKTYTCNVDHKPSNTKVDKRVESKYGPPCPSCPAPEFLGGPSVFLFPPKPKDTLMISRTPEVTCVVVDVSQEDPEVQFNWYVDGVEVHNAKTKPREEQFNSTYRVVSVLTVLHQDWLNGKEYKCKVSNKGLPSSIEKTISKAKGQPREPQVYTLPPSQEEMTKNQVSLTCLVKGFYPSDIAVEWESNGQPENNYKTTPPVLDSDGSFFLYSRLTVDKSRWQEGNVFSCSVMHEALHNHYTQKSLSLSLGK

SEQ ID NO: 151 - DNA, 1329 bp, Artificial Sequence
  IgG heavy chain_IgG4 wild type_DNA
gaggtgcagctgttggagtctgggggaggcttggtacagcctggggggtccctgagactctcctgtgcagcctctggattcacctttagcagttatgatatgagctgggtccgccaggctccagggaaggggctggagtgggtctcagcgatctcttatgataatggtaatacatattacgctgattctgtaaaaggtcggttcaccatctccagagacaattccaagaacacgctgtatctgcaaatgaacagcctgagagccgaggacacggccgtgtattactctgcgagaatggcgcttgatttcgactactggggccagggtacactggtcaccgtgagctcagccagcaccaagggcccttccgtgtttcccctggccccttgctcccggtccacatctgagagcaccgccgccctgggctgtctggtgaaggactacttcccagagcccgtgaccgtgagctggaacagcggcgccctgacaagcggcgtgcacacatttcccgccgtgctgcagagctccggcctgtactccctgtctagcgtggtgacagtgccttcctctagcctgggcaccaagacatatacctgtaacgtggaccacaagccaagcaataccaaggtggataagcgggtggagtctaagtacggccctccttgccctagctgtcctgctccagagtttctgggcggcccttccgtgttcctgtttccacccaaaccaaaggacacactgatgatctctagaacaccagaggtgacctgcgtggtggtggacgtgagccaggaggatcccgaggtgcagttcaactggtacgtggatggcgtggaggtgcacaatgccaagaccaagccaagagaggagcagtttaactctacatacagggtggtgagcgtgctgaccgtgctgcaccaggattggctcaacggcaaggagtataagtgcaaggtgtccaataagggcctgccctcctctatcgagaagacaatctctaaggctaagggccagccaagagagcctcaggtgtacaccctgcctccaagccaggaggagatgacaaagaaccaggtgtccctgacatgtctggtgaagggcttctatccctccgacatcgccgtggagtgggagtctaatggccagcctgagaacaattacaagaccacaccccctgtgctggactctgatggcagcttctttctgtattccaggctgaccgtggataagtctcggtggcaggagggcaacgtgttcagctgctctgtgatgcacgaagccctgcataatcactatactcagaaaagtctgtcactgtcactgggaaag

SEQ ID NO: 152 - protein, 443 aa, Artificial Sequence
  IgG heavy chain_IgG4 mutant TA_amino acid
EVQLLESGGGLVQPGGSLRLSCAASGFTFSSYDMSWVRQAPGKGLEWVSAISYDNGNTYYADSVKGRFTISRDNSKNTLYLQMNSLRAEDTAVYYSARMALDFDYWGQGTLVTVSSASTKGPSVFPLAPCSRSTSESTAALGCLVKDYFPEPVTVSWNSGALTSGVHTFPAVLQSSGLYSLSSVVTVPSSSLGTKTYTCNVDHKPSNTKVDKRVESKYGPPCPSCPAPEFLGGPSVFLFPPKPKDTLMISRTPEVTCVVVDVSQEDPEVQFNWYVDGVEVHNAKTKPREEQFNSAYRVVSVLTVLHQDWLNGKEYKCKVSNKGLPSSIEKTISKAKGQPREPQVYTLPPSQEEMTKNQVSLTCLVKGFYPSDIAVEWESNGQPENNYKTTPPVLDSDGSFFLYSRLTVDKSRWQEGNVFSCSVMHEALHNHYTQKSLSLSLGK

SEQ ID NO: 153 - DNA, 1329 bp, Artificial Sequence
  IgG heavy chain_IgG4 mutant TA_DNA
gaggtgcagctgttggagtctgggggaggcttggtacagcctggggggtccctgagactctcctgtgcagcctctggattcacctttagcagttatgatatgagctgggtccgccaggctccagggaaggggctggagtgggtctcagcgatctcttatgataatggtaatacatattacgctgattctgtaaaaggtcggttcaccatctccagagacaattccaagaacacgctgtatctgcaaatgaacagcctgagagccgaggacacggccgtgtattactctgcgagaatggcgcttgatttcgactactggggccagggtacactggtcaccgtgagctcagccagcaccaagggcccttccgtgtttcccctggccccttgctcccggtccacatctgagagcaccgccgccctgggctgtctggtgaaggactacttcccagagcccgtgaccgtgagctggaacagcggcgccctgacaagcggcgtgcacacatttcccgccgtgctgcagagctccggcctgtactccctgtctagcgtggtgacagtgccttcctctagcctgggcaccaagacatatacctgtaacgtggaccacaagccaagcaataccaaggtggataagcgggtggagtctaagtacggccctccttgccctagctgtcctgctccagagtttctgggcggcccttccgtgttcctgtttccacccaaaccaaaggacacactgatgatctctagaacaccagaggtgacctgcgtggtggtggacgtgagccaggaggatcccgaggtgcagttcaactggtacgtggatggcgtggaggtgcacaatgccaagaccaagccaagagaggagcagtttaactctgcctacagggtggtgagcgtgctgaccgtgctgcaccaggattggctcaacggcaaggagtataagtgcaaggtgtccaataagggcctgccctcctctatcgagaagacaatctctaaggctaagggccagccaagagagcctcaggtgtacaccctgcctccaagccaggaggagatgacaaagaaccaggtgtccctgacatgtctggtgaagggcttctatccctccgacatcgccgtggagtgggagtctaatggccagcctgagaacaattacaagaccacaccccctgtgctggactctgatggcagcttctttctgtattccaggctgaccgtggataagtctcggtggcaggagggcaacgtgttcagctgctctgtgatgcacgaagccctgcataatcactatactcagaaaagtctgtcactgtcactgggaaag

SEQ ID NO: 154 - protein, 446 aa, Artificial Sequence
  IgG heavy chain 1_IgG1 mutant TA_amino acid
EVQLLESGGGLVQPGGSLRLSCAASGFTFSSYDMSWVRQAPGKGLEWVSVISSDGGNTYYADSVKGRFTISRDNSKNTLYLQMNSLRAEDTAVYYSARMALDFDYWGQGTLVTVSSASTKGPSVFPLAPSSKSTSGGTAALGCLVKDYFPEPVTVSWNSGALTSGVHTFPAVLQSSGLYSLSSVVTVPSSSLGTQTYICNVNHKPSNTKVDKKVEPKSCDKTHTCPPCPAPELLGGPSVFLFPPKPKDTLMISRTPEVTCVVVDVSHEDPEVKFNWYVDGVEVHNAKTKPREEQYNSAYRVVSVLTVLHQDWLNGKEYKCKVSNKALPAPIEKTISKAKGQPREPQVYTLPPSRDELTKNQVSLTCLVKGFYPSDIAVEWESNGQPENNYKTTPPVLDSDGSFFLYSKLTVDKSRWQQGNVFSCSVMHEALHNHYTQKSLSLSPGK

SEQ ID NO: 155 - DNA, 1338 bp, Artificial Sequence
  IgG heavy chain 1_IgG1 mutant TA_DNA
gaggtgcagctgttggagtctgggggaggcttggtacagcctggggggtccctgagactctcctgtgcagcctctggattcacctttagcagttatgatatgagctgggtccgccaggctccagggaaggggctggagtgggtctcagtgatctcttctgatggtggtaatacatattacgctgattctgtaaaaggtcggttcaccatctccagagacaattccaagaacacgctgtatctgcaaatgaacagcctgagagccgaggacacggccgtgtattactctgcgagaatggcgcttgatttcgactactggggccagggtacactggtcaccgtgagctcagcctccaccaagggcccatcggtcttccccctggcaccctcctccaagagcacctctgggggcacagcggccctgggctgcctggtcaaggactacttccccgaaccggtgacggtgtcgtggaactcaggcgccctgaccagcggcgtgcacaccttcccggctgtcctacagtcctcaggactctactccctcagcagcgtggtgaccgtgccctccagcagcttgggcacccagacctacatctgcaacgtgaatcacaagcccagcaacaccaaggtggacaagaaagttgagcccaaatcttgtgacaaaactcacacatgcccaccgtgcccagcacctgaactcctggggggaccgtcagtcttcctcttccccccaaaacccaaggacaccctcatgatctcccggacccctgaggtcacatgcgtggtggtggacgtgagccacgaagaccctgaggtcaagttcaactggtacgtggacggcgtggaggtgcataatgccaagacaaagccgcgggaggagcagtacaacagcgcctaccgtgtggtcagcgtcctcaccgtcctgcaccaggactggctgaatggcaaggagtacaagtgcaaggtctccaacaaagccctcccagcccccatcgagaaaaccatctccaaagccaaagggcagccccgagaaccacaggtgtataccctgcccccatcccgggatgagctgaccaagaaccaggtcagcctgacctgcctggtcaaaggcttctatcccagcgacatcgccgtggagtgggagagcaatgggcagccggagaacaactacaagaccacgcctcccgtgctggactccgacggctccttcttcctctacagcaagctcaccgtggacaagagcaggtggcagcaggggaacgtcttctcatgctccgtgatgcatgaggctctgcacaaccactacacgcagaagagcctctccctgtccccgggtaaa

SEQ ID NO: 156 - protein, 446 aa, Artificial Sequence
  IgG heavy chain 1_IgG1 mutant LALA_amino acid
EVQLLESGGGLVQPGGSLRLSCAASGFTFSSYDMSWVRQAPGKGLEWVSVISSDGGNTYYADSVKGRFTISRDNSKNTLYLQMNSLRAEDTAVYYSARMALDFDYWGQGTLVTVSSASTKGPSVFPLAPSSKSTSGGTAALGCLVKDYFPEPVTVSWNSGALTSGVHTFPAVLQSSGLYSLSSVVTVPSSSLGTQTYICNVNHKPSNTKVDKKVEPKSCDKTHTCPPCPAPEAAGGPSVFLFPPKPKDTLMISRTPEVTCVVVDVSHEDPEVKFNWYVDGVEVHNAKTKPREEQYNSTYRVVSVLTVLHQDWLNGKEYKCKVSNKALPAPIEKTISKAKGQPREPQVYTLPPSRDELTKNQVSLTCLVKGFYPSDIAVEWESNGQPENNYKTTPPVLDSDGSFFLYSKLTVDKSRWQQGNVFSCSVMHEALHNHYTQKSLSLSPGK

SEQ ID NO: 157 - DNA, 1338 bp, Artificial Sequence
  IgG heavy chain 1_IgG1 mutant LALA_DNA
gaggtgcagctgttggagtctgggggaggcttggtacagcctggggggtccctgagactctcctgtgcagcctctggattcacctttagcagttatgatatgagctgggtccgccaggctccagggaaggggctggagtgggtctcagtgatctcttctgatggtggtaatacatattacgctgattctgtaaaaggtcggttcaccatctccagagacaattccaagaacacgctgtatctgcaaatgaacagcctgagagccgaggacacggccgtgtattactctgcgagaatggcgcttgatttcgactactggggccagggtacactggtcaccgtgagctcagcctccaccaagggcccatcggtcttccccctggcaccctcctccaagagcacctctgggggcacagcggccctgggctgcctggtcaaggactacttccccgaaccggtgacggtgtcgtggaactcaggcgccctgaccagcggcgtgcacaccttcccggctgtcctacagtcctcaggactctactccctcagcagcgtggtgaccgtgccctccagcagcttgggcacccagacctacatctgcaacgtgaatcacaagcccagcaacaccaaggtggacaagaaagttgagcccaaatcttgtgacaaaactcacacatgcccaccgtgcccagcacctgaagccgccgggggaccgtcagtcttcctcttccccccaaaacccaaggacaccctcatgatctcccggacccctgaggtcacatgcgtggtggtggacgtgagccacgaagaccctgaggtcaagttcaactggtacgtggacggcgtggaggtgcataatgccaagacaaagccgcgggaggagcagtacaacagcacgtaccgtgtggtcagcgtcctcaccgtcctgcaccaggactggctgaatggcaaggagtacaagtgcaaggtctccaacaaagccctcccagcccccatcgagaaaaccatctccaaagccaaagggcagccccgagaaccacaggtgtataccctgcccccatcccgggatgagctgaccaagaaccaggtcagcctgacctgcctggtcaaaggcttctatcccagcgacatcgccgtggagtgggagagcaatgggcagccggagaacaactacaagaccacgcctcccgtgctggactccgacggctccttcttcctctacagcaagctcaccgtggacaagagcaggtggcagcaggggaacgtcttctcatgctccgtgatgcatgaggctctgcacaaccactacacgcagaagagcctctccctgtccccgggtaaa

SEQ ID NO: 158 - protein, 446 aa, Artificial Sequence
  IgG heavy chain 1_IgG1 mutant LALATA_amino acid
EVQLLESGGGLVQPGGSLRLSCAASGFTFSSYDMSWVRQAPGKGLEWVSVISSDGGNTYYADSVKGRFTISRDNSKNTLYLQMNSLRAEDTAVYYSARMALDFDYWGQGTLVTVSSASTKGPSVFPLAPSSKSTSGGTAALGCLVKDYFPEPVTVSWNSGALTSGVHTFPAVLQSSGLYSLSSVVTVPSSSLGTQTYICNVNHKPSNTKVDKKVEPKSCDKTHTCPPCPAPEAAGGPSVFLFPPKPKDTLMISRTPEVTCVVVDVSHEDPEVKFNWYVDGVEVHNAKTKPREEQYNSAYRVVSVLTVLHQDWLNGKEYKCKVSNKALPAPIEKTISKAKGQPREPQVYTLPPSRDELTKNQVSLTCLVKGFYPSDIAVEWESNGQPENNYKTTPPVLDSDGSFFLYSKLTVDKSRWQQGNVFSCSVMHEALHNHYTQKSLSLSPGK

SEQ ID NO: 159 - DNA, 1338 bp, Artificial Sequence
  IgG heavy chain 1_IgG1 mutant LALATA_DNA
gaggtgcagctgttggagtctgggggaggcttggtacagcctggggggtccctgagactctcctgtgcagcctctggattcacctttagcagttatgatatgagctgggtccgccaggctccagggaaggggctggagtgggtctcagtgatctcttctgatggtggtaatacatattacgctgattctgtaaaaggtcggttcaccatctccagagacaattccaagaacacgctgtatctgcaaatgaacagcctgagagccgaggacacggccgtgtattactctgcgagaatggcgcttgatttcgactactggggccagggtacactggtcaccgtgagctcagcctccaccaagggcccatcggtcttccccctggcaccctcctccaagagcacctctgggggcacagcggccctgggctgcctggtcaaggactacttccccgaaccggtgacggtgtcgtggaactcaggcgccctgaccagcggcgtgcacaccttcccggctgtcctacagtcctcaggactctactccctcagcagcgtggtgaccgtgccctccagcagcttgggcacccagacctacatctgcaacgtgaatcacaagcccagcaacaccaaggtggacaagaaagttgagcccaaatcttgtgacaaaactcacacatgcccaccgtgcccagcacctgaagccgccgggggaccgtcagtcttcctcttccccccaaaacccaaggacaccctcatgatctcccggacccctgaggtcacatgcgtggtggtggacgtgagccacgaagaccctgaggtcaagttcaactggtacgtggacggcgtggaggtgcataatgccaagacaaagccgcgggaggagcagtacaacagcgcctaccgtgtggtcagcgtcctcaccgtcctgcaccaggactggctgaatggcaaggagtacaagtgcaaggtctccaacaaagccctcccagcccccatcgagaaaaccatctccaaagccaaagggcagccccgagaaccacaggtgtataccctgcccccatcccgggatgagctgaccaagaaccaggtcagcctgacctgcctggtcaaaggcttctatcccagcgacatcgccgtggagtgggagagcaatgggcagccggagaacaactacaagaccacgcctcccgtgctggactccgacggctccttcttcctctacagcaagctcaccgtggacaagagcaggtggcagcaggggaacgtcttctcatgctccgtgatgcatgaggctctgcacaaccactacacgcagaagagcctctccctgtccccgggtaaa

SEQ ID NO: 160 - protein, 446 aa, Artificial Sequence
  IgG heavy chain 1_IgG1 mutant LALAPG_amino acid
EVQLLESGGGLVQPGGSLRLSCAASGFTFSSYDMSWVRQAPGKGLEWVSVISSDGGNTYYADSVKGRFTISRDNSKNTLYLQMNSLRAEDTAVYYSARMALDFDYWGQGTLVTVSSASTKGPSVFPLAPSSKSTSGGTAALGCLVKDYFPEPVTVSWNSGALTSGVHTFPAVLQSSGLYSLSSVVTVPSSSLGTQTYICNVNHKPSNTKVDKKVEPKSCDKTHTCPPCPAPEAAGGPSVFLFPPKPKDTLMISRTPEVTCVVVDVSHEDPEVKFNWYVDGVEVHNAKTKPREEQYNSTYRVVSVLTVLHQDWLNGKEYKCKVSNKALGAPIEKTISKAKGQPREPQVYTLPPSRDELTKNQVSLTCLVKGFYPSDIAVEWESNGQPENNYKTTPPVLDSDGSFFLYSKLTVDKSRWQQGNVFSCSVMHEALHNHYTQKSLSLSPGK

SEQ ID NO: 161 - DNA, 1338 bp, Artificial Sequence
  IgG heavy chain 1_IgG1 mutant LALAPG_DNA
gaggtgcagctgttggagtctgggggaggcttggtacagcctggggggtccctgagactctcctgtgcagcctctggattcacctttagcagttatgatatgagctgggtccgccaggctccagggaaggggctggagtgggtctcagtgatctcttctgatggtggtaatacatattacgctgattctgtaaaaggtcggttcaccatctccagagacaattccaagaacacgctgtatctgcaaatgaacagcctgagagccgaggacacggccgtgtattactctgcgagaatggcgcttgatttcgactactggggccagggtacactggtcaccgtgagctcagcctccaccaagggcccatcggtcttccccctggcaccctcctccaagagcacctctgggggcacagcggccctgggctgcctggtcaaggactacttccccgaaccggtgacggtgtcgtggaactcaggcgccctgaccagcggcgtgcacaccttcccggctgtcctacagtcctcaggactctactccctcagcagcgtggtgaccgtgccctccagcagcttgggcacccagacctacatctgcaacgtgaatcacaagcccagcaacaccaaggtggacaagaaagttgagcccaaatcttgtgacaaaactcacacatgcccaccgtgcccagcacctgaagccgccgggggaccgtcagtcttcctcttccccccaaaacccaaggacaccctcatgatctcccggacccctgaggtcacatgcgtggtggtggacgtgagccacgaagaccctgaggtcaagttcaactggtacgtggacggcgtggaggtgcataatgccaagacaaagccgcgggaggagcagtacaacagcacgtaccgtgtggtcagcgtcctcaccgtcctgcaccaggactggctgaatggcaaggagtacaagtgcaaggtctccaacaaagccctcggcgcccccatcgagaaaaccatctccaaagccaaagggcagccccgagaaccacaggtgtataccctgcccccatcccgggatgagctgaccaagaaccaggtcagcctgacctgcctggtcaaaggcttctatcccagcgacatcgccgtggagtgggagagcaatgggcagccggagaacaactacaagaccacgcctcccgtgctggactccgacggctccttcttcctctacagcaagctcaccgtggacaagagcaggtggcagcaggggaacgtcttctcatgctccgtgatgcatgaggctctgcacaaccactacacgcagaagagcctctccctgtccccgggtaaa

SEQ ID NO: 162 - protein, 446 aa, Artificial Sequence
  IgG heavy chain 1_IgG1 mutant LALAPGTA_amino acid
EVQLLESGGGLVQPGGSLRLSCAASGFTFSSYDMSWVRQAPGKGLEWVSVISSDGGNTYYADSVKGRFTISRDNSKNTLYLQMNSLRAEDTAVYYSARMALDFDYWGQGTLVTVSSASTKGPSVFPLAPSSKSTSGGTAALGCLVKDYFPEPVTVSWNSGALTSGVHTFPAVLQSSGLYSLSSVVTVPSSSLGTQTYICNVNHKPSNTKVDKKVEPKSCDKTHTCPPCPAPEAAGGPSVFLFPPKPKDTLMISRTPEVTCVVVDVSHEDPEVKFNWYVDGVEVHNAKTKPREEQYNSAYRVVSVLTVLHQDWLNGKEYKCKVSNKALGAPIEKTISKAKGQPREPQVYTLPPSRDELTKNQVSLTCLVKGFYPSDIAVEWESNGQPENNYKTTPPVLDSDGSFFLYSKLTVDKSRWQQGNVFSCSVMHEALHNHYTQKSLSLSPGK

SEQ ID NO: 163 - DNA, 1338 bp, Artificial Sequence
  IgG heavy chain 1_IgG1 mutant LALAPGTA_DNA
gaggtgcagctgttggagtctgggggaggcttggtacagcctggggggtccctgagactctcctgtgcagcctctggattcacctttagcagttatgatatgagctgggtccgccaggctccagggaaggggctggagtgggtctcagtgatctcttctgatggtggtaatacatattacgctgattctgtaaaaggtcggttcaccatctccagagacaattccaagaacacgctgtatctgcaaatgaacagcctgagagccgaggacacggccgtgtattactctgcgagaatggcgcttgatttcgactactggggccagggtacactggtcaccgtgagctcagcctccaccaagggcccatcggtcttccccctggcaccctcctccaagagcacctctgggggcacagcggccctgggctgcctggtcaaggactacttccccgaaccggtgacggtgtcgtggaactcaggcgccctgaccagcggcgtgcacaccttcccggctgtcctacagtcctcaggactctactccctcagcagcgtggtgaccgtgccctccagcagcttgggcacccagacctacatctgcaacgtgaatcacaagcccagcaacaccaaggtggacaagaaagttgagcccaaatcttgtgacaaaactcacacatgcccaccgtgcccagcacctgaagccgccgggggaccgtcagtcttcctcttccccccaaaacccaaggacaccctcatgatctcccggacccctgaggtcacatgcgtggtggtggacgtgagccacgaagaccctgaggtcaagttcaactggtacgtggacggcgtggaggtgcataatgccaagacaaagccgcgggaggagcagtacaacagcgcctaccgtgtggtcagcgtcctcaccgtcctgcaccaggactggctgaatggcaaggagtacaagtgcaaggtctccaacaaagccctcggcgcccccatcgagaaaaccatctccaaagccaaagggcagccccgagaaccacaggtgtataccctgcccccatcccgggatgagctgaccaagaaccaggtcagcctgacctgcctggtcaaaggcttctatcccagcgacatcgccgtggagtgggagagcaatgggcagccggagaacaactacaagaccacgcctcccgtgctggactccgacggctccttcttcctctacagcaagctcaccgtggacaagagcaggtggcagcaggggaacgtcttctcatgctccgtgatgcatgaggctctgcacaaccactacacgcagaagagcctctccctgtccccgggtaaa

SEQ ID NO: 164 - protein, 443 aa, Artificial Sequence
  IgG heavy chain 1_IgG4 wild type_amino acid
EVQLLESGGGLVQPGGSLRLSCAASGFTFSSYDMSWVRQAPGKGLEWVSVISSDGGNTYYADSVKGRFTISRDNSKNTLYLQMNSLRAEDTAVYYSARMALDFDYWGQGTLVTVSSASTKGPSVFPLAPCSRSTSESTAALGCLVKDYFPEPVTVSWNSGALTSGVHTFPAVLQSSGLYSLSSVVTVPSSSLGTKTYTCNVDHKPSNTKVDKRVESKYGPPCPSCPAPEFLGGPSVFLFPPKPKDTLMISRTPEVTCVVVDVSQEDPEVQFNWYVDGVEVHNAKTKPREEQFNSTYRVVSVLTVLHQDWLNGKEYKCKVSNKGLPSSIEKTISKAKGQPREPQVYTLPPSQEEMTKNQVSLTCLVKGFYPSDIAVEWESNGQPENNYKTTPPVLDSDGSFFLYSRLTVDKSRWQEGNVFSCSVMHEALHNHYTQKSLSLSLGK

SEQ ID NO: 165 - DNA, 1329 bp, Artificial Sequence
  IgG heavy chain 1_IgG4 wild type_DNA
gaggtgcagctgttggagtctgggggaggcttggtacagcctggggggtccctgagactctcctgtgcagcctctggattcacctttagcagttatgatatgagctgggtccgccaggctccagggaaggggctggagtgggtctcagtgatctcttctgatggtggtaatacatattacgctgattctgtaaaaggtcggttcaccatctccagagacaattccaagaacacgctgtatctgcaaatgaacagcctgagagccgaggacacggccgtgtattactctgcgagaatggcgcttgatttcgactactggggccagggtacactggtcaccgtgagctcagccagcaccaagggcccttccgtgtttcccctggccccttgctcccggtccacatctgagagcaccgccgccctgggctgtctggtgaaggactacttcccagagcccgtgaccgtgagctggaacagcggcgccctgacaagcggcgtgcacacatttcccgccgtgctgcagagctccggcctgtactccctgtctagcgtggtgacagtgccttcctctagcctgggcaccaagacatatacctgtaacgtggaccacaagccaagcaataccaaggtggataagcgggtggagtctaagtacggccctccttgccctagctgtcctgctccagagtttctgggcggcccttccgtgttcctgtttccacccaaaccaaaggacacactgatgatctctagaacaccagaggtgacctgcgtggtggtggacgtgagccaggaggatcccgaggtgcagttcaactggtacgtggatggcgtggaggtgcacaatgccaagaccaagccaagagaggagcagtttaactctacatacagggtggtgagcgtgctgaccgtgctgcaccaggattggctcaacggcaaggagtataagtgcaaggtgtccaataagggcctgccctcctctatcgagaagacaatctctaaggctaagggccagccaagagagcctcaggtgtacaccctgcctccaagccaggaggagatgacaaagaaccaggtgtccctgacatgtctggtgaagggcttctatccctccgacatcgccgtggagtgggagtctaatggccagcctgagaacaattacaagaccacaccccctgtgctggactctgatggcagcttctttctgtattccaggctgaccgtggataagtctcggtggcaggagggcaacgtgttcagctgctctgtgatgcacgaagccctgcataatcactatactcagaaaagtctgtcactgtcactgggaaag

SEQ ID NO: 166 - protein, 443 aa, Artificial Sequence
  IgG heavy chain 1_IgG4 mutant TA_amino acid
EVQLLESGGGLVQPGGSLRLSCAASGFTFSSYDMSWVRQAPGKGLEWVSVISSDGGNTYYADSVKGRFTISRDNSKNTLYLQMNSLRAEDTAVYYSARMALDFDYWGQGTLVTVSSASTKGPSVFPLAPCSRSTSESTAALGCLVKDYFPEPVTVSWNSGALTSGVHTFPAVLQSSGLYSLSSVVTVPSSSLGTKTYTCNVDHKPSNTKVDKRVESKYGPPCPSCPAPEFLGGPSVFLFPPKPKDTLMISRTPEVTCVVVDVSQEDPEVQFNWYVDGVEVHNAKTKPREEQFNSAYRVVSVLTVLHQDWLNGKEYKCKVSNKGLPSSIEKTISKAKGQPREPQVYTLPPSQEEMTKNQVSLTCLVKGFYPSDIAVEWESNGQPENNYKTTPPVLDSDGSFFLYSRLTVDKSRWQEGNVFSCSVMHEALHNHYTQKSLSLSLGK

SEQ ID NO: 167 - DNA, 1329 bp, Artificial Sequence
  IgG heavy chain 1_IgG4 mutant TA_DNA
gaggtgcagctgttggagtctgggggaggcttggtacagcctggggggtccctgagactctcctgtgcagcctctggattcacctttagcagttatgatatgagctgggtccgccaggctccagggaaggggctggagtgggtctcagtgatctcttctgatggtggtaatacatattacgctgattctgtaaaaggtcggttcaccatctccagagacaattccaagaacacgctgtatctgcaaatgaacagcctgagagccgaggacacggccgtgtattactctgcgagaatggcgcttgatttcgactactggggccagggtacactggtcaccgtgagctcagccagcaccaagggcccttccgtgtttcccctggccccttgctcccggtccacatctgagagcaccgccgccctgggctgtctggtgaaggactacttcccagagcccgtgaccgtgagctggaacagcggcgccctgacaagcggcgtgcacacatttcccgccgtgctgcagagctccggcctgtactccctgtctagcgtggtgacagtgccttcctctagcctgggcaccaagacatatacctgtaacgtggaccacaagccaagcaataccaaggtggataagcgggtggagtctaagtacggccctccttgccctagctgtcctgctccagagtttctgggcggcccttccgtgttcctgtttccacccaaaccaaaggacacactgatgatctctagaacaccagaggtgacctgcgtggtggtggacgtgagccaggaggatcccgaggtgcagttcaactggtacgtggatggcgtggaggtgcacaatgccaagaccaagccaagagaggagcagtttaactctgcctacagggtggtgagcgtgctgaccgtgctgcaccaggattggctcaacggcaaggagtataagtgcaaggtgtccaataagggcctgccctcctctatcgagaagacaatctctaaggctaagggccagccaagagagcctcaggtgtacaccctgcctccaagccaggaggagatgacaaagaaccaggtgtccctgacatgtctggtgaagggcttctatccctccgacatcgccgtggagtgggagtctaatggccagcctgagaacaattacaagaccacaccccctgtgctggactctgatggcagcttctttctgtattccaggctgaccgtggataagtctcggtggcaggagggcaacgtgttcagctgctctgtgatgcacgaagccctgcataatcactatactcagaaaagtctgtcactgtcactgggaaag

SEQ ID NO: 168 - protein, 446 aa, Artificial Sequence
  IgG heavy chain 2_IgG1 mutant TA_amino acid
EVQLLESGGGLVQPGGSLRLSCAASGFTFSSYDMSWVRQAPGKGLEWVSAISPQMGRVYYADSVKGRFTISRDNSKNTLYLQMNSLRAEDTAVYYCARMALDFDYWGQGTLVTVSSASTKGPSVFPLAPSSKSTSGGTAALGCLVKDYFPEPVTVSWNSGALTSGVHTFPAVLQSSGLYSLSSVVTVPSSSLGTQTYICNVNHKPSNTKVDKKVEPKSCDKTHTCPPCPAPELLGGPSVFLFPPKPKDTLMISRTPEVTCVVVDVSHEDPEVKFNWYVDGVEVHNAKTKPREEQYNSAYRVVSVLTVLHQDWLNGKEYKCKVSNKALPAPIEKTISKAKGQPREPQVYTLPPSRDELTKNQVSLTCLVKGFYPSDIAVEWESNGQPENNYKTTPPVLDSDGSFFLYSKLTVDKSRWQQGNVFSCSVMHEALHNHYTQKSLSLSPGK

SEQ ID NO: 169 - DNA, 1338 bp, Artificial Sequence
  IgG heavy chain 2_IgG1 mutant TA_DNA
gaggtgcagctgttggagtctgggggaggcttggtacagcctggggggtccctgagactctcctgtgcagcctctggattcacctttagcagttatgatatgagctgggtccgccaggctccagggaaggggctggagtgggtctcagcgatctcgccgcagatgggtcgggtgtattacgctgattctgtaaaaggtcggttcaccatctccagagacaattccaagaacacgctgtatctgcaaatgaacagcctgagagccgaggacacggccgtgtattactgtgcgagaatggcgcttgatttcgactactggggccagggtacactggtcaccgtgagctcagcctccaccaagggcccatcggtcttccccctggcaccctcctccaagagcacctctgggggcacagcggccctgggctgcctggtcaaggactacttccccgaaccggtgacggtgtcgtggaactcaggcgccctgaccagcggcgtgcacaccttcccggctgtcctacagtcctcaggactctactccctcagcagcgtggtgaccgtgccctccagcagcttgggcacccagacctacatctgcaacgtgaatcacaagcccagcaacaccaaggtggacaagaaagttgagcccaaatcttgtgacaaaactcacacatgcccaccgtgcccagcacctgaactcctggggggaccgtcagtcttcctcttccccccaaaacccaaggacaccctcatgatctcccggacccctgaggtcacatgcgtggtggtggacgtgagccacgaagaccctgaggtcaagttcaactggtacgtggacggcgtggaggtgcataatgccaagacaaagccgcgggaggagcagtacaacagcgcctaccgtgtggtcagcgtcctcaccgtcctgcaccaggactggctgaatggcaaggagtacaagtgcaaggtctccaacaaagccctcccagcccccatcgagaaaaccatctccaaagccaaagggcagccccgagaaccacaggtgtataccctgcccccatcccgggatgagctgaccaagaaccaggtcagcctgacctgcctggtcaaaggcttctatcccagcgacatcgccgtggagtgggagagcaatgggcagccggagaacaactacaagaccacgcctcccgtgctggactccgacggctccttcttcctctacagcaagctcaccgtggacaagagcaggtggcagcaggggaacgtcttctcatgctccgtgatgcatgaggctctgcacaaccactacacgcagaagagcctctccctgtccccgggtaaa

SEQ ID NO: 170 - protein, 446 aa, Artificial Sequence
  IgG heavy chain 2_IgG1 mutant LALA_amino acid
EVQLLESGGGLVQPGGSLRLSCAASGFTFSSYDMSWVRQAPGKGLEWVSAISPQMGRVYYADSVKGRFTISRDNSKNTLYLQMNSLRAEDTAVYYCARMALDFDYWGQGTLVTVSSASTKGPSVFPLAPSSKSTSGGTAALGCLVKDYFPEPVTVSWNSGALTSGVHTFPAVLQSSGLYSLSSVVTVPSSSLGTQTYICNVNHKPSNTKVDKKVEPKSCDKTHTCPPCPAPEAAGGPSVFLFPPKPKDTLMISRTPEVTCVVVDVSHEDPEVKFNWYVDGVEVHNAKTKPREEQYNSTYRVVSVLTVLHQDWLNGKEYKCKVSNKALPAPIEKTISKAKGQPREPQVYTLPPSRDELTKNQVSLTCLVKGFYPSDIAVEWESNGQPENNYKTTPPVLDSDGSFFLYSKLTVDKSRWQQGNVFSCSVMHEALHNHYTQKSLSLSPGK

SEQ ID NO: 171 - DNA, 1338 bp, Artificial Sequence
  IgG heavy chain 2_IgG1 mutant LALA_DNA
gaggtgcagctgttggagtctgggggaggcttggtacagcctggggggtccctgagactctcctgtgcagcctctggattcacctttagcagttatgatatgagctgggtccgccaggctccagggaaggggctggagtgggtctcagcgatctcgccgcagatgggtcgggtgtattacgctgattctgtaaaaggtcggttcaccatctccagagacaattccaagaacacgctgtatctgcaaatgaacagcctgagagccgaggacacggccgtgtattactgtgcgagaatggcgcttgatttcgactactggggccagggtacactggtcaccgtgagctcagcctccaccaagggcccatcggtcttccccctggcaccctcctccaagagcacctctgggggcacagcggccctgggctgcctggtcaaggactacttccccgaaccggtgacggtgtcgtggaactcaggcgccctgaccagcggcgtgcacaccttcccggctgtcctacagtcctcaggactctactccctcagcagcgtggtgaccgtgccctccagcagcttgggcacccagacctacatctgcaacgtgaatcacaagcccagcaacaccaaggtggacaagaaagttgagcccaaatcttgtgacaaaactcacacatgcccaccgtgcccagcacctgaagccgccgggggaccgtcagtcttcctcttccccccaaaacccaaggacaccctcatgatctcccggacccctgaggtcacatgcgtggtggtggacgtgagccacgaagaccctgaggtcaagttcaactggtacgtggacggcgtggaggtgcataatgccaagacaaagccgcgggaggagcagtacaacagcacgtaccgtgtggtcagcgtcctcaccgtcctgcaccaggactggctgaatggcaaggagtacaagtgcaaggtctccaacaaagccctcccagcccccatcgagaaaaccatctccaaagccaaagggcagccccgagaaccacaggtgtataccctgcccccatcccgggatgagctgaccaagaaccaggtcagcctgacctgcctggtcaaaggcttctatcccagcgacatcgccgtggagtgggagagcaatgggcagccggagaacaactacaagaccacgcctcccgtgctggactccgacggctccttcttcctctacagcaagctcaccgtggacaagagcaggtggcagcaggggaacgtcttctcatgctccgtgatgcatgaggctctgcacaaccactacacgcagaagagcctctccctgtccccgggtaaa

SEQ ID NO: 172 - protein, 446 aa, Artificial Sequence
  IgG heavy chain 2_IgG1 mutant LALATA_amino acid
EVQLLESGGGLVQPGGSLRLSCAASGFTFSSYDMSWVRQAPGKGLEWVSAISPQMGRVYYADSVKGRFTISRDNSKNTLYLQMNSLRAEDTAVYYCARMALDFDYWGQGTLVTVSSASTKGPSVFPLAPSSKSTSGGTAALGCLVKDYFPEPVTVSWNSGALTSGVHTFPAVLQSSGLYSLSSVVTVPSSSLGTQTYICNVNHKPSNTKVDKKVEPKSCDKTHTCPPCPAPEAAGGPSVFLFPPKPKDTLMISRTPEVTCVVVDVSHEDPEVKFNWYVDGVEVHNAKTKPREEQYNSAYRVVSVLTVLHQDWLNGKEYKCKVSNKALPAPIEKTISKAKGQPREPQVYTLPPSRDELTKNQVSLTCLVKGFYPSDIAVEWESNGQPENNYKTTPPVLDSDGSFFLYSKLTVDKSRWQQGNVFSCSVMHEALHNHYTQKSLSLSPGK

SEQ ID NO: 173 - DNA, 1338 bp, Artificial Sequence
  IgG heavy chain 2_IgG1 mutant LALATA_DNA
gaggtgcagctgttggagtctgggggaggcttggtacagcctggggggtccctgagactctcctgtgcagcctctggattcacctttagcagttatgatatgagctgggtccgccaggctccagggaaggggctggagtgggtctcagcgatctcgccgcagatgggtcgggtgtattacgctgattctgtaaaaggtcggttcaccatctccagagacaattccaagaacacgctgtatctgcaaatgaacagcctgagagccgaggacacggccgtgtattactgtgcgagaatggcgcttgatttcgactactggggccagggtacactggtcaccgtgagctcagcctccaccaagggcccatcggtcttccccctggcaccctcctccaagagcacctctgggggcacagcggccctgggctgcctggtcaaggactacttccccgaaccggtgacggtgtcgtggaactcaggcgccctgaccagcggcgtgcacaccttcccggctgtcctacagtcctcaggactctactccctcagcagcgtggtgaccgtgccctccagcagcttgggcacccagacctacatctgcaacgtgaatcacaagcccagcaacaccaaggtggacaagaaagttgagcccaaatcttgtgacaaaactcacacatgcccaccgtgcccagcacctgaagccgccgggggaccgtcagtcttcctcttccccccaaaacccaaggacaccctcatgatctcccggacccctgaggtcacatgcgtggtggtggacgtgagccacgaagaccctgaggtcaagttcaactggtacgtggacggcgtggaggtgcataatgccaagacaaagccgcgggaggagcagtacaacagcgcctaccgtgtggtcagcgtcctcaccgtcctgcaccaggactggctgaatggcaaggagtacaagtgcaaggtctccaacaaagccctcccagcccccatcgagaaaaccatctccaaagccaaagggcagccccgagaaccacaggtgtataccctgcccccatcccgggatgagctgaccaagaaccaggtcagcctgacctgcctggtcaaaggcttctatcccagcgacatcgccgtggagtgggagagcaatgggcagccggagaacaactacaagaccacgcctcccgtgctggactccgacggctccttcttcctctacagcaagctcaccgtggacaagagcaggtggcagcaggggaacgtcttctcatgctccgtgatgcatgaggctctgcacaaccactacacgcagaagagcctctccctgtccccgggtaaa

SEQ ID NO: 174 - protein, 446 aa, Artificial Sequence
  IgG heavy chain 2_IgG1 mutant LALAPG_amino acid
EVQLLESGGGLVQPGGSLRLSCAASGFTFSSYDMSWVRQAPGKGLEWVSAISPQMGRVYYADSVKGRFTISRDNSKNTLYLQMNSLRAEDTAVYYCARMALDFDYWGQGTLVTVSSASTKGPSVFPLAPSSKSTSGGTAALGCLVKDYFPEPVTVSWNSGALTSGVHTFPAVLQSSGLYSLSSVVTVPSSSLGTQTYICNVNHKPSNTKVDKKVEPKSCDKTHTCPPCPAPEAAGGPSVFLFPPKPKDTLMISRTPEVTCVVVDVSHEDPEVKFNWYVDGVEVHNAKTKPREEQYNSTYRVVSVLTVLHQDWLNGKEYKCKVSNKALGAPIEKTISKAKGQPREPQVYTLPPSRDELTKNQVSLTCLVKGFYPSDIAVEWESNGQPENNYKTTPPVLDSDGSFFLYSKLTVDKSRWQQGNVFSCSVMHEALHNHYTQKSLSLSPGK

SEQ ID NO: 175 - DNA, 1338 bp, Artificial Sequence
  IgG heavy chain 2_IgG1 mutant LALAPG_DNA
gaggtgcagctgttggagtctgggggaggcttggtacagcctggggggtccctgagactctcctgtgcagcctctggattcacctttagcagttatgatatgagctgggtccgccaggctccagggaaggggctggagtgggtctcagcgatctcgccgcagatgggtcgggtgtattacgctgattctgtaaaaggtcggttcaccatctccagagacaattccaagaacacgctgtatctgcaaatgaacagcctgagagccgaggacacggccgtgtattactgtgcgagaatggcgcttgatttcgactactggggccagggtacactggtcaccgtgagctcagcctccaccaagggcccatcggtcttccccctggcaccctcctccaagagcacctctgggggcacagcggccctgggctgcctggtcaaggactacttccccgaaccggtgacggtgtcgtggaactcaggcgccctgaccagcggcgtgcacaccttcccggctgtcctacagtcctcaggactctactccctcagcagcgtggtgaccgtgccctccagcagcttgggcacccagacctacatctgcaacgtgaatcacaagcccagcaacaccaaggtggacaagaaagttgagcccaaatcttgtgacaaaactcacacatgcccaccgtgcccagcacctgaagccgccgggggaccgtcagtcttcctcttccccccaaaacccaaggacaccctcatgatctcccggacccctgaggtcacatgcgtggtggtggacgtgagccacgaagaccctgaggtcaagttcaactggtacgtggacggcgtggaggtgcataatgccaagacaaagccgcgggaggagcagtacaacagcacgtaccgtgtggtcagcgtcctcaccgtcctgcaccaggactggctgaatggcaaggagtacaagtgcaaggtctccaacaaagccctcggcgcccccatcgagaaaaccatctccaaagccaaagggcagccccgagaaccacaggtgtataccctgcccccatcccgggatgagctgaccaagaaccaggtcagcctgacctgcctggtcaaaggcttctatcccagcgacatcgccgtggagtgggagagcaatgggcagccggagaacaactacaagaccacgcctcccgtgctggactccgacggctccttcttcctctacagcaagctcaccgtggacaagagcaggtggcagcaggggaacgtcttctcatgctccgtgatgcatgaggctctgcacaaccactacacgcagaagagcctctccctgtccccgggtaaa

SEQ ID NO: 176 - protein, 446 aa, Artificial Sequence
  IgG heavy chain 2_IgG1 mutant LALAPGTA_amino acid
EVQLLESGGGLVQPGGSLRLSCAASGFTFSSYDMSWVRQAPGKGLEWVSAISPQMGRVYYADSVKGRFTISRDNSKNTLYLQMNSLRAEDTAVYYCARMALDFDYWGQGTLVTVSSASTKGPSVFPLAPSSKSTSGGTAALGCLVKDYFPEPVTVSWNSGALTSGVHTFPAVLQSSGLYSLSSVVTVPSSSLGTQTYICNVNHKPSNTKVDKKVEPKSCDKTHTCPPCPAPEAAGGPSVFLFPPKPKDTLMISRTPEVTCVVVDVSHEDPEVKFNWYVDGVEVHNAKTKPREEQYNSAYRVVSVLTVLHQDWLNGKEYKCKVSNKALGAPIEKTISKAKGQPREPQVYTLPPSRDELTKNQVSLTCLVKGFYPSDIAVEWESNGQPENNYKTTPPVLDSDGSFFLYSKLTVDKSRWQQGNVFSCSVMHEALHNHYTQKSLSLSPGK

SEQ ID NO: 177 - DNA, 1338 bp, Artificial Sequence
  IgG heavy chain 2_IgG1 mutant LALAPGTA_DNA
gaggtgcagctgttggagtctgggggaggcttggtacagcctggggggtccctgagactctcctgtgcagcctctggattcacctttagcagttatgatatgagctgggtccgccaggctccagggaaggggctggagtgggtctcagcgatctcgccgcagatgggtcgggtgtattacgctgattctgtaaaaggtcggttcaccatctccagagacaattccaagaacacgctgtatctgcaaatgaacagcctgagagccgaggacacggccgtgtattactgtgcgagaatggcgcttgatttcgactactggggccagggtacactggtcaccgtgagctcagcctccaccaagggcccatcggtcttccccctggcaccctcctccaagagcacctctgggggcacagcggccctgggctgcctggtcaaggactacttccccgaaccggtgacggtgtcgtggaactcaggcgccctgaccagcggcgtgcacaccttcccggctgtcctacagtcctcaggactctactccctcagcagcgtggtgaccgtgccctccagcagcttgggcacccagacctacatctgcaacgtgaatcacaagcccagcaacaccaaggtggacaagaaagttgagcccaaatcttgtgacaaaactcacacatgcccaccgtgcccagcacctgaagccgccgggggaccgtcagtcttcctcttccccccaaaacccaaggacaccctcatgatctcccggacccctgaggtcacatgcgtggtggtggacgtgagccacgaagaccctgaggtcaagttcaactggtacgtggacggcgtggaggtgcataatgccaagacaaagccgcgggaggagcagtacaacagcgcctaccgtgtggtcagcgtcctcaccgtcctgcaccaggactggctgaatggcaaggagtacaagtgcaaggtctccaacaaagccctcggcgcccccatcgagaaaaccatctccaaagccaaagggcagccccgagaaccacaggtgtataccctgcccccatcccgggatgagctgaccaagaaccaggtcagcctgacctgcctggtcaaaggcttctatcccagcgacatcgccgtggagtgggagagcaatgggcagccggagaacaactacaagaccacgcctcccgtgctggactccgacggctccttcttcctctacagcaagctcaccgtggacaagagcaggtggcagcaggggaacgtcttctcatgctccgtgatgcatgaggctctgcacaaccactacacgcagaagagcctctccctgtccccgggtaaa

SEQ ID NO: 178 - protein, 443 aa, Artificial Sequence
  IgG heavy chain 2_IgG4 wild type_amino acid
EVQLLESGGGLVQPGGSLRLSCAASGFTFSSYDMSWVRQAPGKGLEWVSAISPQMGRVYYADSVKGRFTISRDNSKNTLYLQMNSLRAEDTAVYYCARMALDFDYWGQGTLVTVSSASTKGPSVFPLAPCSRSTSESTAALGCLVKDYFPEPVTVSWNSGALTSGVHTFPAVLQSSGLYSLSSVVTVPSSSLGTKTYTCNVDHKPSNTKVDKRVESKYGPPCPSCPAPEFLGGPSVFLFPPKPKDTLMISRTPEVTCVVVDVSQEDPEVQFNWYVDGVEVHNAKTKPREEQFNSTYRVVSVLTVLHQDWLNGKEYKCKVSNKGLPSSIEKTISKAKGQPREPQVYTLPPSQEEMTKNQVSLTCLVKGFYPSDIAVEWESNGQPENNYKTTPPVLDSDGSFFLYSRLTVDKSRWQEGNVFSCSVMHEALHNHYTQKSLSLSLGK

SEQ ID NO: 179 - DNA, 1329 bp, Artificial Sequence
  IgG heavy chain 2_IgG4 wild type_DNA
gaggtgcagctgttggagtctgggggaggcttggtacagcctggggggtccctgagactctcctgtgcagcctctggattcacctttagcagttatgatatgagctgggtccgccaggctccagggaaggggctggagtgggtctcagcgatctcgccgcagatgggtcgggtgtattacgctgattctgtaaaaggtcggttcaccatctccagagacaattccaagaacacgctgtatctgcaaatgaacagcctgagagccgaggacacggccgtgtattactgtgcgagaatggcgcttgatttcgactactggggccagggtacactggtcaccgtgagctcagccagcaccaagggcccttccgtgtttcccctggccccttgctcccggtccacatctgagagcaccgccgccctgggctgtctggtgaaggactacttcccagagcccgtgaccgtgagctggaacagcggcgccctgacaagcggcgtgcacacatttcccgccgtgctgcagagctccggcctgtactccctgtctagcgtggtgacagtgccttcctctagcctgggcaccaagacatatacctgtaacgtggaccacaagccaagcaataccaaggtggataagcgggtggagtctaagtacggccctccttgccctagctgtcctgctccagagtttctgggcggcccttccgtgttcctgtttccacccaaaccaaaggacacactgatgatctctagaacaccagaggtgacctgcgtggtggtggacgtgagccaggaggatcccgaggtgcagttcaactggtacgtggatggcgtggaggtgcacaatgccaagaccaagccaagagaggagcagtttaactctacatacagggtggtgagcgtgctgaccgtgctgcaccaggattggctcaacggcaaggagtataagtgcaaggtgtccaataagggcctgccctcctctatcgagaagacaatctctaaggctaagggccagccaagagagcctcaggtgtacaccctgcctccaagccaggaggagatgacaaagaaccaggtgtccctgacatgtctggtgaagggcttctatccctccgacatcgccgtggagtgggagtctaatggccagcctgagaacaattacaagaccacaccccctgtgctggactctgatggcagcttctttctgtattccaggctgaccgtggataagtctcggtggcaggagggcaacgtgttcagctgctctgtgatgcacgaagccctgcataatcactatactcagaaaagtctgtcactgtcactgggaaag

SEQ ID NO: 180 - protein, 443 aa, Artificial Sequence
  IgG heavy chain 2_IgG4 mutant TA_amino acid
EVQLLESGGGLVQPGGSLRLSCAASGFTFSSYDMSWVRQAPGKGLEWVSAISPQMGRVYYADSVKGRFTISRDNSKNTLYLQMNSLRAEDTAVYYCARMALDFDYWGQGTLVTVSSASTKGPSVFPLAPCSRSTSESTAALGCLVKDYFPEPVTVSWNSGALTSGVHTFPAVLQSSGLYSLSSVVTVPSSSLGTKTYTCNVDHKPSNTKVDKRVESKYGPPCPSCPAPEFLGGPSVFLFPPKPKDTLMISRTPEVTCVVVDVSQEDPEVQFNWYVDGVEVHNAKTKPREEQFNSAYRVVSVLTVLHQDWLNGKEYKCKVSNKGLPSSIEKTISKAKGQPREPQVYTLPPSQEEMTKNQVSLTCLVKGFYPSDIAVEWESNGQPENNYKTTPPVLDSDGSFFLYSRLTVDKSRWQEGNVFSCSVMHEALHNHYTQKSLSLSLGK

SEQ ID NO: 181 - DNA, 1329 bp, Artificial Sequence
  IgG heavy chain 2_IgG4 mutant TA_DNA
gaggtgcagctgttggagtctgggggaggcttggtacagcctggggggtccctgagactctcctgtgcagcctctggattcacctttagcagttatgatatgagctgggtccgccaggctccagggaaggggctggagtgggtctcagcgatctcgccgcagatgggtcgggtgtattacgctgattctgtaaaaggtcggttcaccatctccagagacaattccaagaacacgctgtatctgcaaatgaacagcctgagagccgaggacacggccgtgtattactgtgcgagaatggcgcttgatttcgactactggggccagggtacactggtcaccgtgagctcagccagcaccaagggcccttccgtgtttcccctggccccttgctcccggtccacatctgagagcaccgccgccctgggctgtctggtgaaggactacttcccagagcccgtgaccgtgagctggaacagcggcgccctgacaagcggcgtgcacacatttcccgccgtgctgcagagctccggcctgtactccctgtctagcgtggtgacagtgccttcctctagcctgggcaccaagacatatacctgtaacgtggaccacaagccaagcaataccaaggtggataagcgggtggagtctaagtacggccctccttgccctagctgtcctgctccagagtttctgggcggcccttccgtgttcctgtttccacccaaaccaaaggacacactgatgatctctagaacaccagaggtgacctgcgtggtggtggacgtgagccaggaggatcccgaggtgcagttcaactggtacgtggatggcgtggaggtgcacaatgccaagaccaagccaagagaggagcagtttaactctgcctacagggtggtgagcgtgctgaccgtgctgcaccaggattggctcaacggcaaggagtataagtgcaaggtgtccaataagggcctgccctcctctatcgagaagacaatctctaaggctaagggccagccaagagagcctcaggtgtacaccctgcctccaagccaggaggagatgacaaagaaccaggtgtccctgacatgtctggtgaagggcttctatccctccgacatcgccgtggagtgggagtctaatggccagcctgagaacaattacaagaccacaccccctgtgctggactctgatggcagcttctttctgtattccaggctgaccgtggataagtctcggtggcaggagggcaacgtgttcagctgctctgtgatgcacgaagccctgcataatcactatactcagaaaagtctgtcactgtcactgggaaag

SEQ ID NO: 182 - protein, 446 aa, Artificial Sequence
  IgG heavy chain 3_IgG1 mutant TA_amino acid
EVQLLESGGGLVQPGGSLRLSCAASGFTFSSYDMSWVRQAPGKGLEWVSAIDPLGGNIYYADSVKGRFTISRDNSKNTLYLQMNSLRAEDTAVYYCARMALDFDYWGQGTLVTVSSASTKGPSVFPLAPSSKSTSGGTAALGCLVKDYFPEPVTVSWNSGALTSGVHTFPAVLQSSGLYSLSSVVTVPSSSLGTQTYICNVNHKPSNTKVDKKVEPKSCDKTHTCPPCPAPELLGGPSVFLFPPKPKDTLMISRTPEVTCVVVDVSHEDPEVKFNWYVDGVEVHNAKTKPREEQYNSAYRVVSVLTVLHQDWLNGKEYKCKVSNKALPAPIEKTISKAKGQPREPQVYTLPPSRDELTKNQVSLTCLVKGFYPSDIAVEWESNGQPENNYKTTPPVLDSDGSFFLYSKLTVDKSRWQQGNVFSCSVMHEALHNHYTQKSLSLSPGK

SEQ ID NO: 183 - DNA, 1338 bp, Artificial Sequence
  IgG heavy chain 3_IgG1 mutant TA_DNA
gaggtgcagctgttggagtctgggggaggcttggtacagcctggggggtccctgagactctcctgtgcagcctctggattcacctttagcagttatgatatgagctgggtccgccaggctccagggaaggggctggagtgggtctcagcgatcgatccgttggggggtaatatttattacgctgattctgtaaaaggtcggttcaccatctccagagacaattccaagaacacgctgtatctgcaaatgaacagcctgagagccgaggacacggccgtgtattactgtgcgagaatggcgcttgatttcgactactggggccagggtacactggtcaccgtgagctcagcctccaccaagggcccatcggtcttccccctggcaccctcctccaagagcacctctgggggcacagcggccctgggctgcctggtcaaggactacttccccgaaccggtgacggtgtcgtggaactcaggcgccctgaccagcggcgtgcacaccttcccggctgtcctacagtcctcaggactctactccctcagcagcgtggtgaccgtgccctccagcagcttgggcacccagacctacatctgcaacgtgaatcacaagcccagcaacaccaaggtggacaagaaagttgagcccaaatcttgtgacaaaactcacacatgcccaccgtgcccagcacctgaactcctggggggaccgtcagtcttcctcttccccccaaaacccaaggacaccctcatgatctcccggacccctgaggtcacatgcgtggtggtggacgtgagccacgaagaccctgaggtcaagttcaactggtacgtggacggcgtggaggtgcataatgccaagacaaagccgcgggaggagcagtacaacagcgcctaccgtgtggtcagcgtcctcaccgtcctgcaccaggactggctgaatggcaaggagtacaagtgcaaggtctccaacaaagccctcccagcccccatcgagaaaaccatctccaaagccaaagggcagccccgagaaccacaggtgtataccctgcccccatcccgggatgagctgaccaagaaccaggtcagcctgacctgcctggtcaaaggcttctatcccagcgacatcgccgtggagtgggagagcaatgggcagccggagaacaactacaagaccacgcctcccgtgctggactccgacggctccttcttcctctacagcaagctcaccgtggacaagagcaggtggcagcaggggaacgtcttctcatgctccgtgatgcatgaggctctgcacaaccactacacgcagaagagcctctccctgtccccgggtaaa

SEQ ID NO: 184 - protein, 446 aa, Artificial Sequence
  IgG heavy chain 3_IgG1 mutant LALA_amino acid
EVQLLESGGGLVQPGGSLRLSCAASGFTFSSYDMSWVRQAPGKGLEWVSAIDPLGGNIYYADSVKGRFTISRDNSKNTLYLQMNSLRAEDTAVYYCARMALDFDYWGQGTLVTVSSASTKGPSVFPLAPSSKSTSGGTAALGCLVKDYFPEPVTVSWNSGALTSGVHTFPAVLQSSGLYSLSSVVTVPSSSLGTQTYICNVNHKPSNTKVDKKVEPKSCDKTHTCPPCPAPEAAGGPSVFLFPPKPKDTLMISRTPEVTCVVVDVSHEDPEVKFNWYVDGVEVHNAKTKPREEQYNSTYRVVSVLTVLHQDWLNGKEYKCKVSNKALPAPIEKTISKAKGQPREPQVYTLPPSRDELTKNQVSLTCLVKGFYPSDIAVEWESNGQPENNYKTTPPVLDSDGSFFLYSKLTVDKSRWQQGNVFSCSVMHEALHNHYTQKSLSLSPGK

SEQ ID NO: 185 - DNA, 1338 bp, Artificial Sequence
  IgG heavy chain 3_IgG1 mutant LALA_DNA
gaggtgcagctgttggagtctgggggaggcttggtacagcctggggggtccctgagactctcctgtgcagcctctggattcacctttagcagttatgatatgagctgggtccgccaggctccagggaaggggctggagtgggtctcagcgatcgatccgttggggggtaatatttattacgctgattctgtaaaaggtcggttcaccatctccagagacaattccaagaacacgctgtatctgcaaatgaacagcctgagagccgaggacacggccgtgtattactgtgcgagaatggcgcttgatttcgactactggggccagggtacactggtcaccgtgagctcagcctccaccaagggcccatcggtcttccccctggcaccctcctccaagagcacctctgggggcacagcggccctgggctgcctggtcaaggactacttccccgaaccggtgacggtgtcgtggaactcaggcgccctgaccagcggcgtgcacaccttcccggctgtcctacagtcctcaggactctactccctcagcagcgtggtgaccgtgccctccagcagcttgggcacccagacctacatctgcaacgtgaatcacaagcccagcaacaccaaggtggacaagaaagttgagcccaaatcttgtgacaaaactcacacatgcccaccgtgcccagcacctgaagccgccgggggaccgtcagtcttcctcttccccccaaaacccaaggacaccctcatgatctcccggacccctgaggtcacatgcgtggtggtggacgtgagccacgaagaccctgaggtcaagttcaactggtacgtggacggcgtggaggtgcataatgccaagacaaagccgcgggaggagcagtacaacagcacgtaccgtgtggtcagcgtcctcaccgtcctgcaccaggactggctgaatggcaaggagtacaagtgcaaggtctccaacaaagccctcccagcccccatcgagaaaaccatctccaaagccaaagggcagccccgagaaccacaggtgtataccctgcccccatcccgggatgagctgaccaagaaccaggtcagcctgacctgcctggtcaaaggcttctatcccagcgacatcgccgtggagtgggagagcaatgggcagccggagaacaactacaagaccacgcctcccgtgctggactccgacggctccttcttcctctacagcaagctcaccgtggacaagagcaggtggcagcaggggaacgtcttctcatgctccgtgatgcatgaggctctgcacaaccactacacgcagaagagcctctccctgtccccgggtaaa

SEQ ID NO: 186 - protein, 446 aa, Artificial Sequence
  IgG heavy chain 3_IgG1 mutant LALATA_amino acid
EVQLLESGGGLVQPGGSLRLSCAASGFTFSSYDMSWVRQAPGKGLEWVSAIDPLGGNIYYADSVKGRFTISRDNSKNTLYLQMNSLRAEDTAVYYCARMALDFDYWGQGTLVTVSSASTKGPSVFPLAPSSKSTSGGTAALGCLVKDYFPEPVTVSWNSGALTSGVHTFPAVLQSSGLYSLSSVVTVPSSSLGTQTYICNVNHKPSNTKVDKKVEPKSCDKTHTCPPCPAPEAAGGPSVFLFPPKPKDTLMISRTPEVTCVVVDVSHEDPEVKFNWYVDGVEVHNAKTKPREEQYNSAYRVVSVLTVLHQDWLNGKEYKCKVSNKALPAPIEKTISKAKGQPREPQVYTLPPSRDELTKNQVSLTCLVKGFYPSDIAVEWESNGQPENNYKTTPPVLDSDGSFFLYSKLTVDKSRWQQGNVFSCSVMHEALHNHYTQKSLSLSPGK

SEQ ID NO: 187 - DNA, 1338 bp, Artificial Sequence
  IgG heavy chain 3_IgG1 mutant LALATA_DNA
gaggtgcagctgttggagtctgggggaggcttggtacagcctggggggtccctgagactctcctgtgcagcctctggattcacctttagcagttatgatatgagctgggtccgccaggctccagggaaggggctggagtgggtctcagcgatcgatccgttggggggtaatatttattacgctgattctgtaaaaggtcggttcaccatctccagagacaattccaagaacacgctgtatctgcaaatgaacagcctgagagccgaggacacggccgtgtattactgtgcgagaatggcgcttgatttcgactactggggccagggtacactggtcaccgtgagctcagcctccaccaagggcccatcggtcttccccctggcaccctcctccaagagcacctctgggggcacagcggccctgggctgcctggtcaaggactacttccccgaaccggtgacggtgtcgtggaactcaggcgccctgaccagcggcgtgcacaccttcccggctgtcctacagtcctcaggactctactccctcagcagcgtggtgaccgtgccctccagcagcttgggcacccagacctacatctgcaacgtgaatcacaagcccagcaacaccaaggtggacaagaaagttgagcccaaatcttgtgacaaaactcacacatgcccaccgtgcccagcacctgaagccgccgggggaccgtcagtcttcctcttccccccaaaacccaaggacaccctcatgatctcccggacccctgaggtcacatgcgtggtggtggacgtgagccacgaagaccctgaggtcaagttcaactggtacgtggacggcgtggaggtgcataatgccaagacaaagccgcgggaggagcagtacaacagcgcctaccgtgtggtcagcgtcctcaccgtcctgcaccaggactggctgaatggcaaggagtacaagtgcaaggtctccaacaaagccctcccagcccccatcgagaaaaccatctccaaagccaaagggcagccccgagaaccacaggtgtataccctgcccccatcccgggatgagctgaccaagaaccaggtcagcctgacctgcctggtcaaaggcttctatcccagcgacatcgccgtggagtgggagagcaatgggcagccggagaacaactacaagaccacgcctcccgtgctggactccgacggctccttcttcctctacagcaagctcaccgtggacaagagcaggtggcagcaggggaacgtcttctcatgctccgtgatgcatgaggctctgcacaaccactacacgcagaagagcctctccctgtccccgggtaaa

SEQ ID NO: 188 - protein, 446 aa, Artificial Sequence
  IgG heavy chain 3_IgG1 mutant LALAPG_amino acid
EVQLLESGGGLVQPGGSLRLSCAASGFTFSSYDMSWVRQAPGKGLEWVSAIDPLGGNIYYADSVKGRFTISRDNSKNTLYLQMNSLRAEDTAVYYCARMALDFDYWGQGTLVTVSSASTKGPSVFPLAPSSKSTSGGTAALGCLVKDYFPEPVTVSWNSGALTSGVHTFPAVLQSSGLYSLSSVVTVPSSSLGTQTYICNVNHKPSNTKVDKKVEPKSCDKTHTCPPCPAPEAAGGPSVFLFPPKPKDTLMISRTPEVTCVVVDVSHEDPEVKFNWYVDGVEVHNAKTKPREEQYNSTYRVVSVLTVLHQDWLNGKEYKCKVSNKALGAPIEKTISKAKGQPREPQVYTLPPSRDELTKNQVSLTCLVKGFYPSDIAVEWESNGQPENNYKTTPPVLDSDGSFFLYSKLTVDKSRWQQGNVFSCSVMHEALHNHYTQKSLSLSPGK

SEQ ID NO: 189 - DNA, 1338 bp, Artificial Sequence
  IgG heavy chain 3_IgG1 mutant LALAPG_DNA
gaggtgcagctgttggagtctgggggaggcttggtacagcctggggggtccctgagactctcctgtgcagcctctggattcacctttagcagttatgatatgagctgggtccgccaggctccagggaaggggctggagtgggtctcagcgatcgatccgttggggggtaatatttattacgctgattctgtaaaaggtcggttcaccatctccagagacaattccaagaacacgctgtatctgcaaatgaacagcctgagagccgaggacacggccgtgtattactgtgcgagaatggcgcttgatttcgactactggggccagggtacactggtcaccgtgagctcagcctccaccaagggcccatcggtcttccccctggcaccctcctccaagagcacctctgggggcacagcggccctgggctgcctggtcaaggactacttccccgaaccggtgacggtgtcgtggaactcaggcgccctgaccagcggcgtgcacaccttcccggctgtcctacagtcctcaggactctactccctcagcagcgtggtgaccgtgccctccagcagcttgggcacccagacctacatctgcaacgtgaatcacaagcccagcaacaccaaggtggacaagaaagttgagcccaaatcttgtgacaaaactcacacatgcccaccgtgcccagcacctgaagccgccgggggaccgtcagtcttcctcttccccccaaaacccaaggacaccctcatgatctcccggacccctgaggtcacatgcgtggtggtggacgtgagccacgaagaccctgaggtcaagttcaactggtacgtggacggcgtggaggtgcataatgccaagacaaagccgcgggaggagcagtacaacagcacgtaccgtgtggtcagcgtcctcaccgtcctgcaccaggactggctgaatggcaaggagtacaagtgcaaggtctccaacaaagccctcggcgcccccatcgagaaaaccatctccaaagccaaagggcagccccgagaaccacaggtgtataccctgcccccatcccgggatgagctgaccaagaaccaggtcagcctgacctgcctggtcaaaggcttctatcccagcgacatcgccgtggagtgggagagcaatgggcagccggagaacaactacaagaccacgcctcccgtgctggactccgacggctccttcttcctctacagcaagctcaccgtggacaagagcaggtggcagcaggggaacgtcttctcatgctccgtgatgcatgaggctctgcacaaccactacacgcagaagagcctctccctgtccccgggtaaa

SEQ ID NO: 190 - protein, 446 aa, Artificial Sequence
  IgG heavy chain 3_IgG1 mutant LALAPGTA_amino acid
EVQLLESGGGLVQPGGSLRLSCAASGFTFSSYDMSWVRQAPGKGLEWVSAIDPLGGNIYYADSVKGRFTISRDNSKNTLYLQMNSLRAEDTAVYYCARMALDFDYWGQGTLVTVSSASTKGPSVFPLAPSSKSTSGGTAALGCLVKDYFPEPVTVSWNSGALTSGVHTFPAVLQSSGLYSLSSVVTVPSSSLGTQTYICNVNHKPSNTKVDKKVEPKSCDKTHTCPPCPAPEAAGGPSVFLFPPKPKDTLMISRTPEVTCVVVDVSHEDPEVKFNWYVDGVEVHNAKTKPREEQYNSAYRVVSVLTVLHQDWLNGKEYKCKVSNKALGAPIEKTISKAKGQPREPQVYTLPPSRDELTKNQVSLTCLVKGFYPSDIAVEWESNGQPENNYKTTPPVLDSDGSFFLYSKLTVDKSRWQQGNVFSCSVMHEALHNHYTQKSLSLSPGK

SEQ ID NO: 191 - DNA, 1338 bp, Artificial Sequence
  IgG heavy chain 3_IgG1 mutant LALAPGTA_DNA
gaggtgcagctgttggagtctgggggaggcttggtacagcctggggggtccctgagactctcctgtgcagcctctggattcacctttagcagttatgatatgagctgggtccgccaggctccagggaaggggctggagtgggtctcagcgatcgatccgttggggggtaatatttattacgctgattctgtaaaaggtcggttcaccatctccagagacaattccaagaacacgctgtatctgcaaatgaacagcctgagagccgaggacacggccgtgtattactgtgcgagaatggcgcttgatttcgactactggggccagggtacactggtcaccgtgagctcagcctccaccaagggcccatcggtcttccccctggcaccctcctccaagagcacctctgggggcacagcggccctgggctgcctggtcaaggactacttccccgaaccggtgacggtgtcgtggaactcaggcgccctgaccagcggcgtgcacaccttcccggctgtcctacagtcctcaggactctactccctcagcagcgtggtgaccgtgccctccagcagcttgggcacccagacctacatctgcaacgtgaatcacaagcccagcaacaccaaggtggacaagaaagttgagcccaaatcttgtgacaaaactcacacatgcccaccgtgcccagcacctgaagccgccgggggaccgtcagtcttcctcttccccccaaaacccaaggacaccctcatgatctcccggacccctgaggtcacatgcgtggtggtggacgtgagccacgaagaccctgaggtcaagttcaactggtacgtggacggcgtggaggtgcataatgccaagacaaagccgcgggaggagcagtacaacagcgcctaccgtgtggtcagcgtcctcaccgtcctgcaccaggactggctgaatggcaaggagtacaagtgcaaggtctccaacaaagccctcggcgcccccatcgagaaaaccatctccaaagccaaagggcagccccgagaaccacaggtgtataccctgcccccatcccgggatgagctgaccaagaaccaggtcagcctgacctgcctggtcaaaggcttctatcccagcgacatcgccgtggagtgggagagcaatgggcagccggagaacaactacaagaccacgcctcccgtgctggactccgacggctccttcttcctctacagcaagctcaccgtggacaagagcaggtggcagcaggggaacgtcttctcatgctccgtgatgcatgaggctctgcacaaccactacacgcagaagagcctctccctgtccccgggtaaa

SEQ ID NO: 192 - protein, 443 aa, Artificial Sequence
  IgG heavy chain 3_IgG4 wild type_amino acid
EVQLLESGGGLVQPGGSLRLSCAASGFTFSSYDMSWVRQAPGKGLEWVSAIDPLGGNIYYADSVKGRFTISRDNSKNTLYLQMNSLRAEDTAVYYCARMALDFDYWGQGTLVTVSSASTKGPSVFPLAPCSRSTSESTAALGCLVKDYFPEPVTVSWNSGALTSGVHTFPAVLQSSGLYSLSSVVTVPSSSLGTKTYTCNVDHKPSNTKVDKRVESKYGPPCPSCPAPEFLGGPSVFLFPPKPKDTLMISRTPEVTCVVVDVSQEDPEVQFNWYVDGVEVHNAKTKPREEQFNSTYRVVSVLTVLHQDWLNGKEYKCKVSNKGLPSSIEKTISKAKGQPREPQVYTLPPSQEEMTKNQVSLTCLVKGFYPSDIAVEWESNGQPENNYKTTPPVLDSDGSFFLYSRLTVDKSRWQEGNVFSCSVMHEALHNHYTQKSLSLSLGK

SEQ ID NO: 193 - DNA, 1329 bp, Artificial Sequence
  IgG heavy chain 3_IgG4 wild type_DNA
gaggtgcagctgttggagtctgggggaggcttggtacagcctggggggtccctgagactctcctgtgcagcctctggattcacctttagcagttatgatatgagctgggtccgccaggctccagggaaggggctggagtgggtctcagcgatcgatccgttggggggtaatatttattacgctgattctgtaaaaggtcggttcaccatctccagagacaattccaagaacacgctgtatctgcaaatgaacagcctgagagccgaggacacggccgtgtattactgtgcgagaatggcgcttgatttcgactactggggccagggtacactggtcaccgtgagctcagccagcaccaagggcccttccgtgtttcccctggccccttgctcccggtccacatctgagagcaccgccgccctgggctgtctggtgaaggactacttcccagagcccgtgaccgtgagctggaacagcggcgccctgacaagcggcgtgcacacatttcccgccgtgctgcagagctccggcctgtactccctgtctagcgtggtgacagtgccttcctctagcctgggcaccaagacatatacctgtaacgtggaccacaagccaagcaataccaaggtggataagcgggtggagtctaagtacggccctccttgccctagctgtcctgctccagagtttctgggcggcccttccgtgttcctgtttccacccaaaccaaaggacacactgatgatctctagaacaccagaggtgacctgcgtggtggtggacgtgagccaggaggatcccgaggtgcagttcaactggtacgtggatggcgtggaggtgcacaatgccaagaccaagccaagagaggagcagtttaactctacatacagggtggtgagcgtgctgaccgtgctgcaccaggattggctcaacggcaaggagtataagtgcaaggtgtccaataagggcctgccctcctctatcgagaagacaatctctaaggctaagggccagccaagagagcctcaggtgtacaccctgcctccaagccaggaggagatgacaaagaaccaggtgtccctgacatgtctggtgaagggcttctatccctccgacatcgccgtggagtgggagtctaatggccagcctgagaacaattacaagaccacaccccctgtgctggactctgatggcagcttctttctgtattccaggctgaccgtggataagtctcggtggcaggagggcaacgtgttcagctgctctgtgatgcacgaagccctgcataatcactatactcagaaaagtctgtcactgtcactgggaaag

SEQ ID NO: 194 - protein, 443 aa, Artificial Sequence
  IgG heavy chain 3_IgG4 mutant TA_amino acid
EVQLLESGGGLVQPGGSLRLSCAASGFTFSSYDMSWVRQAPGKGLEWVSAIDPLGGNIYYADSVKGRFTISRDNSKNTLYLQMNSLRAEDTAVYYCARMALDFDYWGQGTLVTVSSASTKGPSVFPLAPCSRSTSESTAALGCLVKDYFPEPVTVSWNSGALTSGVHTFPAVLQSSGLYSLSSVVTVPSSSLGTKTYTCNVDHKPSNTKVDKRVESKYGPPCPSCPAPEFLGGPSVFLFPPKPKDTLMISRTPEVTCVVVDVSQEDPEVQFNWYVDGVEVHNAKTKPREEQFNSAYRVVSVLTVLHQDWLNGKEYKCKVSNKGLPSSIEKTISKAKGQPREPQVYTLPPSQEEMTKNQVSLTCLVKGFYPSDIAVEWESNGQPENNYKTTPPVLDSDGSFFLYSRLTVDKSRWQEGNVFSCSVMHEALHNHYTQKSLSLSLGK

SEQ ID NO: 195 - DNA, 1329 bp, Artificial Sequence
  IgG heavy chain 3_IgG4 mutant TA_DNA
gaggtgcagctgttggagtctgggggaggcttggtacagcctggggggtccctgagactctcctgtgcagcctctggattcacctttagcagttatgatatgagctgggtccgccaggctccagggaaggggctggagtgggtctcagcgatcgatccgttggggggtaatatttattacgctgattctgtaaaaggtcggttcaccatctccagagacaattccaagaacacgctgtatctgcaaatgaacagcctgagagccgaggacacggccgtgtattactgtgcgagaatggcgcttgatttcgactactggggccagggtacactggtcaccgtgagctcagccagcaccaagggcccttccgtgtttcccctggccccttgctcccggtccacatctgagagcaccgccgccctgggctgtctggtgaaggactacttcccagagcccgtgaccgtgagctggaacagcggcgccctgacaagcggcgtgcacacatttcccgccgtgctgcagagctccggcctgtactccctgtctagcgtggtgacagtgccttcctctagcctgggcaccaagacatatacctgtaacgtggaccacaagccaagcaataccaaggtggataagcgggtggagtctaagtacggccctccttgccctagctgtcctgctccagagtttctgggcggcccttccgtgttcctgtttccacccaaaccaaaggacacactgatgatctctagaacaccagaggtgacctgcgtggtggtggacgtgagccaggaggatcccgaggtgcagttcaactggtacgtggatggcgtggaggtgcacaatgccaagaccaagccaagagaggagcagtttaactctgcctacagggtggtgagcgtgctgaccgtgctgcaccaggattggctcaacggcaaggagtataagtgcaaggtgtccaataagggcctgccctcctctatcgagaagacaatctctaaggctaagggccagccaagagagcctcaggtgtacaccctgcctccaagccaggaggagatgacaaagaaccaggtgtccctgacatgtctggtgaagggcttctatccctccgacatcgccgtggagtgggagtctaatggccagcctgagaacaattacaagaccacaccccctgtgctggactctgatggcagcttctttctgtattccaggctgaccgtggataagtctcggtggcaggagggcaacgtgttcagctgctctgtgatgcacgaagccctgcataatcactatactcagaaaagtctgtcactgtcactgggaaag

SEQ ID NO: 196 - protein, 446 aa, Artificial Sequence
  IgG heavy chain 4_IgG1 mutant TA_amino acid
EVQLLESGGGLVQPGGSLRLSCAASGFTFSSYDMSWVRQAPGKGLEWVSAISPYSGRIYYADSVKGRFTISRDNSKNTLYLQMNSLRAEDTAVYYSARMALDFDYWGQGTLVTVSSASTKGPSVFPLAPSSKSTSGGTAALGCLVKDYFPEPVTVSWNSGALTSGVHTFPAVLQSSGLYSLSSVVTVPSSSLGTQTYICNVNHKPSNTKVDKKVEPKSCDKTHTCPPCPAPELLGGPSVFLFPPKPKDTLMISRTPEVTCVVVDVSHEDPEVKFNWYVDGVEVHNAKTKPREEQYNSAYRVVSVLTVLHQDWLNGKEYKCKVSNKALPAPIEKTISKAKGQPREPQVYTLPPSRDELTKNQVSLTCLVKGFYPSDIAVEWESNGQPENNYKTTPPVLDSDGSFFLYSKLTVDKSRWQQGNVFSCSVMHEALHNHYTQKSLSLSPGK

SEQ ID NO: 197 - DNA, 1338 bp, Artificial Sequence
  IgG heavy chain 4_IgG1 mutant TA_DNA
gaggtgcagctgttggagtctgggggaggcttggtacagcctggggggtccctgagactctcctgtgcagcctctggattcacctttagcagttatgatatgagctgggtccgccaggctccagggaaggggctggagtgggtctcagcgatctctccgtattcgggtaggatttattacgctgattctgtaaaaggtcggttcaccatctccagagacaattccaagaacacgctgtatctgcaaatgaacagcctgagagccgaggacacggccgtgtattactctgcgagaatggcgcttgatttcgactactggggccagggtacactggtcaccgtgagctcagcctccaccaagggcccatcggtcttccccctggcaccctcctccaagagcacctctgggggcacagcggccctgggctgcctggtcaaggactacttccccgaaccggtgacggtgtcgtggaactcaggcgccctgaccagcggcgtgcacaccttcccggctgtcctacagtcctcaggactctactccctcagcagcgtggtgaccgtgccctccagcagcttgggcacccagacctacatctgcaacgtgaatcacaagcccagcaacaccaaggtggacaagaaagttgagcccaaatcttgtgacaaaactcacacatgcccaccgtgcccagcacctgaactcctggggggaccgtcagtcttcctcttccccccaaaacccaaggacaccctcatgatctcccggacccctgaggtcacatgcgtggtggtggacgtgagccacgaagaccctgaggtcaagttcaactggtacgtggacggcgtggaggtgcataatgccaagacaaagccgcgggaggagcagtacaacagcgcctaccgtgtggtcagcgtcctcaccgtcctgcaccaggactggctgaatggcaaggagtacaagtgcaaggtctccaacaaagccctcccagcccccatcgagaaaaccatctccaaagccaaagggcagccccgagaaccacaggtgtataccctgcccccatcccgggatgagctgaccaagaaccaggtcagcctgacctgcctggtcaaaggcttctatcccagcgacatcgccgtggagtgggagagcaatgggcagccggagaacaactacaagaccacgcctcccgtgctggactccgacggctccttcttcctctacagcaagctcaccgtggacaagagcaggtggcagcaggggaacgtcttctcatgctccgtgatgcatgaggctctgcacaaccactacacgcagaagagcctctccctgtccccgggtaaa

SEQ ID NO: 198 - protein, 446 aa, Artificial Sequence
  IgG heavy chain 4_IgG1 mutant LALA_amino acid
EVQLLESGGGLVQPGGSLRLSCAASGFTFSSYDMSWVRQAPGKGLEWVSAISPYSGRIYYADSVKGRFTISRDNSKNTLYLQMNSLRAEDTAVYYSARMALDFDYWGQGTLVTVSSASTKGPSVFPLAPSSKSTSGGTAALGCLVKDYFPEPVTVSWNSGALTSGVHTFPAVLQSSGLYSLSSVVTVPSSSLGTQTYICNVNHKPSNTKVDKKVEPKSCDKTHTCPPCPAPEAAGGPSVFLFPPKPKDTLMISRTPEVTCVVVDVSHEDPEVKFNWYVDGVEVHNAKTKPREEQYNSTYRVVSVLTVLHQDWLNGKEYKCKVSNKALPAPIEKTISKAKGQPREPQVYTLPPSRDELTKNQVSLTCLVKGFYPSDIAVEWESNGQPENNYKTTPPVLDSDGSFFLYSKLTVDKSRWQQGNVFSCSVMHEALHNHYTQKSLSLSPGK

SEQ ID NO: 199 - DNA, 1338 bp, Artificial Sequence
  IgG heavy chain 4_IgG1 mutant LALA_DNA
gaggtgcagctgttggagtctgggggaggcttggtacagcctggggggtccctgagactctcctgtgcagcctctggattcacctttagcagttatgatatgagctgggtccgccaggctccagggaaggggctggagtgggtctcagcgatctctccgtattcgggtaggatttattacgctgattctgtaaaaggtcggttcaccatctccagagacaattccaagaacacgctgtatctgcaaatgaacagcctgagagccgaggacacggccgtgtattactctgcgagaatggcgcttgatttcgactactggggccagggtacactggtcaccgtgagctcagcctccaccaagggcccatcggtcttccccctggcaccctcctccaagagcacctctgggggcacagcggccctgggctgcctggtcaaggactacttccccgaaccggtgacggtgtcgtggaactcaggcgccctgaccagcggcgtgcacaccttcccggctgtcctacagtcctcaggactctactccctcagcagcgtggtgaccgtgccctccagcagcttgggcacccagacctacatctgcaacgtgaatcacaagcccagcaacaccaaggtggacaagaaagttgagcccaaatcttgtgacaaaactcacacatgcccaccgtgcccagcacctgaagccgccgggggaccgtcagtcttcctcttccccccaaaacccaaggacaccctcatgatctcccggacccctgaggtcacatgcgtggtggtggacgtgagccacgaagaccctgaggtcaagttcaactggtacgtggacggcgtggaggtgcataatgccaagacaaagccgcgggaggagcagtacaacagcacgtaccgtgtggtcagcgtcctcaccgtcctgcaccaggactggctgaatggcaaggagtacaagtgcaaggtctccaacaaagccctcccagcccccatcgagaaaaccatctccaaagccaaagggcagccccgagaaccacaggtgtataccctgcccccatcccgggatgagctgaccaagaaccaggtcagcctgacctgcctggtcaaaggcttctatcccagcgacatcgccgtggagtgggagagcaatgggcagccggagaacaactacaagaccacgcctcccgtgctggactccgacggctccttcttcctctacagcaagctcaccgtggacaagagcaggtggcagcaggggaacgtcttctcatgctccgtgatgcatgaggctctgcacaaccactacacgcagaagagcctctccctgtccccgggtaaa

SEQ ID NO: 200 - protein, 446 aa, Artificial Sequence
  IgG heavy chain 4_IgG1 mutant LALATA_amino acid
EVQLLESGGGLVQPGGSLRLSCAASGFTFSSYDMSWVRQAPGKGLEWVSAISPYSGRIYYADSVKGRFTISRDNSKNTLYLQMNSLRAEDTAVYYSARMALDFDYWGQGTLVTVSSASTKGPSVFPLAPSSKSTSGGTAALGCLVKDYFPEPVTVSWNSGALTSGVHTFPAVLQSSGLYSLSSVVTVPSSSLGTQTYICNVNHKPSNTKVDKKVEPKSCDKTHTCPPCPAPEAAGGPSVFLFPPKPKDTLMISRTPEVTCVVVDVSHEDPEVKFNWYVDGVEVHNAKTKPREEQYNSAYRVVSVLTVLHQDWLNGKEYKCKVSNKALPAPIEKTISKAKGQPREPQVYTLPPSRDELTKNQVSLTCLVKGFYPSDIAVEWESNGQPENNYKTTPPVLDSDGSFFLYSKLTVDKSRWQQGNVFSCSVMHEALHNHYTQKSLSLSPGK

SEQ ID NO: 201 - DNA, 1338 bp, Artificial Sequence
  IgG heavy chain 4_IgG1 mutant LALATA_DNA
gaggtgcagctgttggagtctgggggaggcttggtacagcctggggggtccctgagactctcctgtgcagcctctggattcacctttagcagttatgatatgagctgggtccgccaggctccagggaaggggctggagtgggtctcagcgatctctccgtattcgggtaggatttattacgctgattctgtaaaaggtcggttcaccatctccagagacaattccaagaacacgctgtatctgcaaatgaacagcctgagagccgaggacacggccgtgtattactctgcgagaatggcgcttgatttcgactactggggccagggtacactggtcaccgtgagctcagcctccaccaagggcccatcggtcttccccctggcaccctcctccaagagcacctctgggggcacagcggccctgggctgcctggtcaaggactacttccccgaaccggtgacggtgtcgtggaactcaggcgccctgaccagcggcgtgcacaccttcccggctgtcctacagtcctcaggactctactccctcagcagcgtggtgaccgtgccctccagcagcttgggcacccagacctacatctgcaacgtgaatcacaagcccagcaacaccaaggtggacaagaaagttgagcccaaatcttgtgacaaaactcacacatgcccaccgtgcccagcacctgaagccgccgggggaccgtcagtcttcctcttccccccaaaacccaaggacaccctcatgatctcccggacccctgaggtcacatgcgtggtggtggacgtgagccacgaagaccctgaggtcaagttcaactggtacgtggacggcgtggaggtgcataatgccaagacaaagccgcgggaggagcagtacaacagcgcctaccgtgtggtcagcgtcctcaccgtcctgcaccaggactggctgaatggcaaggagtacaagtgcaaggtctccaacaaagccctcccagcccccatcgagaaaaccatctccaaagccaaagggcagccccgagaaccacaggtgtataccctgcccccatcccgggatgagctgaccaagaaccaggtcagcctgacctgcctggtcaaaggcttctatcccagcgacatcgccgtggagtgggagagcaatgggcagccggagaacaactacaagaccacgcctcccgtgctggactccgacggctccttcttcctctacagcaagctcaccgtggacaagagcaggtggcagcaggggaacgtcttctcatgctccgtgatgcatgaggctctgcacaaccactacacgcagaagagcctctccctgtccccgggtaaa

SEQ ID NO: 202 - protein, 446 aa, Artificial Sequence
  IgG heavy chain 4_IgG1 mutant LALAPG_amino acid
EVQLLESGGGLVQPGGSLRLSCAASGFTFSSYDMSWVRQAPGKGLEWVSAISPYSGRIYYADSVKGRFTISRDNSKNTLYLQMNSLRAEDTAVYYSARMALDFDYWGQGTLVTVSSASTKGPSVFPLAPSSKSTSGGTAALGCLVKDYFPEPVTVSWNSGALTSGVHTFPAVLQSSGLYSLSSVVTVPSSSLGTQTYICNVNHKPSNTKVDKKVEPKSCDKTHTCPPCPAPEAAGGPSVFLFPPKPKDTLMISRTPEVTCVVVDVSHEDPEVKFNWYVDGVEVHNAKTKPREEQYNSTYRVVSVLTVLHQDWLNGKEYKCKVSNKALGAPIEKTISKAKGQPREPQVYTLPPSRDELTKNQVSLTCLVKGFYPSDIAVEWESNGQPENNYKTTPPVLDSDGSFFLYSKLTVDKSRWQQGNVFSCSVMHEALHNHYTQKSLSLSPGK

SEQ ID NO: 203 - DNA, 1338 bp, Artificial Sequence
  IgG heavy chain 4_IgG1 mutant LALAPG_DNA
gaggtgcagctgttggagtctgggggaggcttggtacagcctggggggtccctgagactctcctgtgcagcctctggattcacctttagcagttatgatatgagctgggtccgccaggctccagggaaggggctggagtgggtctcagcgatctctccgtattcgggtaggatttattacgctgattctgtaaaaggtcggttcaccatctccagagacaattccaagaacacgctgtatctgcaaatgaacagcctgagagccgaggacacggccgtgtattactctgcgagaatggcgcttgatttcgactactggggccagggtacactggtcaccgtgagctcagcctccaccaagggcccatcggtcttccccctggcaccctcctccaagagcacctctgggggcacagcggccctgggctgcctggtcaaggactacttccccgaaccggtgacggtgtcgtggaactcaggcgccctgaccagcggcgtgcacaccttcccggctgtcctacagtcctcaggactctactccctcagcagcgtggtgaccgtgccctccagcagcttgggcacccagacctacatctgcaacgtgaatcacaagcccagcaacaccaaggtggacaagaaagttgagcccaaatcttgtgacaaaactcacacatgcccaccgtgcccagcacctgaagccgccgggggaccgtcagtcttcctcttccccccaaaacccaaggacaccctcatgatctcccggacccctgaggtcacatgcgtggtggtggacgtgagccacgaagaccctgaggtcaagttcaactggtacgtggacggcgtggaggtgcataatgccaagacaaagccgcgggaggagcagtacaacagcacgtaccgtgtggtcagcgtcctcaccgtcctgcaccaggactggctgaatggcaaggagtacaagtgcaaggtctccaacaaagccctcggcgcccccatcgagaaaaccatctccaaagccaaagggcagccccgagaaccacaggtgtataccctgcccccatcccgggatgagctgaccaagaaccaggtcagcctgacctgcctggtcaaaggcttctatcccagcgacatcgccgtggagtgggagagcaatgggcagccggagaacaactacaagaccacgcctcccgtgctggactccgacggctccttcttcctctacagcaagctcaccgtggacaagagcaggtggcagcaggggaacgtcttctcatgctccgtgatgcatgaggctctgcacaaccactacacgcagaagagcctctccctgtccccgggtaaa

SEQ ID NO: 204 - protein, 446 aa, Artificial Sequence
  IgG heavy chain 4_IgG1 mutant LALAPGTA_amino acid
EVQLLESGGGLVQPGGSLRLSCAASGFTFSSYDMSWVRQAPGKGLEWVSAISPYSGRIYYADSVKGRFTISRDNSKNTLYLQMNSLRAEDTAVYYSARMALDFDYWGQGTLVTVSSASTKGPSVFPLAPSSKSTSGGTAALGCLVKDYFPEPVTVSWNSGALTSGVHTFPAVLQSSGLYSLSSVVTVPSSSLGTQTYICNVNHKPSNTKVDKKVEPKSCDKTHTCPPCPAPEAAGGPSVFLFPPKPKDTLMISRTPEVTCVVVDVSHEDPEVKFNWYVDGVEVHNAKTKPREEQYNSAYRVVSVLTVLHQDWLNGKEYKCKVSNKALGAPIEKTISKAKGQPREPQVYTLPPSRDELTKNQVSLTCLVKGFYPSDIAVEWESNGQPENNYKTTPPVLDSDGSFFLYSKLTVDKSRWQQGNVFSCSVMHEALHNHYTQKSLSLSPGK

SEQ ID NO: 205 - DNA, 1338 bp, Artificial Sequence
  IgG heavy chain 4_IgG1 mutant LALAPGTA_DNA
gaggtgcagctgttggagtctgggggaggcttggtacagcctggggggtccctgagactctcctgtgcagcctctggattcacctttagcagttatgatatgagctgggtccgccaggctccagggaaggggctggagtgggtctcagcgatctctccgtattcgggtaggatttattacgctgattctgtaaaaggtcggttcaccatctccagagacaattccaagaacacgctgtatctgcaaatgaacagcctgagagccgaggacacggccgtgtattactctgcgagaatggcgcttgatttcgactactggggccagggtacactggtcaccgtgagctcagcctccaccaagggcccatcggtcttccccctggcaccctcctccaagagcacctctgggggcacagcggccctgggctgcctggtcaaggactacttccccgaaccggtgacggtgtcgtggaactcaggcgccctgaccagcggcgtgcacaccttcccggctgtcctacagtcctcaggactctactccctcagcagcgtggtgaccgtgccctccagcagcttgggcacccagacctacatctgcaacgtgaatcacaagcccagcaacaccaaggtggacaagaaagttgagcccaaatcttgtgacaaaactcacacatgcccaccgtgcccagcacctgaagccgccgggggaccgtcagtcttcctcttccccccaaaacccaaggacaccctcatgatctcccggacccctgaggtcacatgcgtggtggtggacgtgagccacgaagaccctgaggtcaagttcaactggtacgtggacggcgtggaggtgcataatgccaagacaaagccgcgggaggagcagtacaacagcgcctaccgtgtggtcagcgtcctcaccgtcctgcaccaggactggctgaatggcaaggagtacaagtgcaaggtctccaacaaagccctcggcgcccccatcgagaaaaccatctccaaagccaaagggcagccccgagaaccacaggtgtataccctgcccccatcccgggatgagctgaccaagaaccaggtcagcctgacctgcctggtcaaaggcttctatcccagcgacatcgccgtggagtgggagagcaatgggcagccggagaacaactacaagaccacgcctcccgtgctggactccgacggctccttcttcctctacagcaagctcaccgtggacaagagcaggtggcagcaggggaacgtcttctcatgctccgtgatgcatgaggctctgcacaaccactacacgcagaagagcctctccctgtccccgggtaaa

SEQ ID NO: 206 - protein, 443 aa, Artificial Sequence
  IgG heavy chain 4_IgG4 wild type_amino acid
EVQLLESGGGLVQPGGSLRLSCAASGFTFSSYDMSWVRQAPGKGLEWVSAISPYSGRIYYADSVKGRFTISRDNSKNTLYLQMNSLRAEDTAVYYSARMALDFDYWGQGTLVTVSSASTKGPSVFPLAPCSRSTSESTAALGCLVKDYFPEPVTVSWNSGALTSGVHTFPAVLQSSGLYSLSSVVTVPSSSLGTKTYTCNVDHKPSNTKVDKRVESKYGPPCPSCPAPEFLGGPSVFLFPPKPKDTLMISRTPEVTCVVVDVSQEDPEVQFNWYVDGVEVHNAKTKPREEQFNSTYRVVSVLTVLHQDWLNGKEYKCKVSNKGLPSSIEKTISKAKGQPREPQVYTLPPSQEEMTKNQVSLTCLVKGFYPSDIAVEWESNGQPENNYKTTPPVLDSDGSFFLYSRLTVDKSRWQEGNVFSCSVMHEALHNHYTQKSLSLSLGK

SEQ ID NO: 207 - DNA, 1329 bp, Artificial Sequence
  IgG heavy chain 4_IgG4 wild type_DNA
gaggtgcagctgttggagtctgggggaggcttggtacagcctggggggtccctgagactctcctgtgcagcctctggattcacctttagcagttatgatatgagctgggtccgccaggctccagggaaggggctggagtgggtctcagcgatctctccgtattcgggtaggatttattacgctgattctgtaaaaggtcggttcaccatctccagagacaattccaagaacacgctgtatctgcaaatgaacagcctgagagccgaggacacggccgtgtattactctgcgagaatggcgcttgatttcgactactggggccagggtacactggtcaccgtgagctcagccagcaccaagggcccttccgtgtttcccctggccccttgctcccggtccacatctgagagcaccgccgccctgggctgtctggtgaaggactacttcccagagcccgtgaccgtgagctggaacagcggcgccctgacaagcggcgtgcacacatttcccgccgtgctgcagagctccggcctgtactccctgtctagcgtggtgacagtgccttcctctagcctgggcaccaagacatatacctgtaacgtggaccacaagccaagcaataccaaggtggataagcgggtggagtctaagtacggccctccttgccctagctgtcctgctccagagtttctgggcggcccttccgtgttcctgtttccacccaaaccaaaggacacactgatgatctctagaacaccagaggtgacctgcgtggtggtggacgtgagccaggaggatcccgaggtgcagttcaactggtacgtggatggcgtggaggtgcacaatgccaagaccaagccaagagaggagcagtttaactctacatacagggtggtgagcgtgctgaccgtgctgcaccaggattggctcaacggcaaggagtataagtgcaaggtgtccaataagggcctgccctcctctatcgagaagacaatctctaaggctaagggccagccaagagagcctcaggtgtacaccctgcctccaagccaggaggagatgacaaagaaccaggtgtccctgacatgtctggtgaagggcttctatccctccgacatcgccgtggagtgggagtctaatggccagcctgagaacaattacaagaccacaccccctgtgctggactctgatggcagcttctttctgtattccaggctgaccgtggataagtctcggtggcaggagggcaacgtgttcagctgctctgtgatgcacgaagccctgcataatcactatactcagaaaagtctgtcactgtcactgggaaag

SEQ ID NO: 208 - protein, 443 aa, Artificial Sequence
  IgG heavy chain 4_IgG4 mutant TA_amino acid
EVQLLESGGGLVQPGGSLRLSCAASGFTFSSYDMSWVRQAPGKGLEWVSAISPYSGRIYYADSVKGRFTISRDNSKNTLYLQMNSLRAEDTAVYYSARMALDFDYWGQGTLVTVSSASTKGPSVFPLAPCSRSTSESTAALGCLVKDYFPEPVTVSWNSGALTSGVHTFPAVLQSSGLYSLSSVVTVPSSSLGTKTYTCNVDHKPSNTKVDKRVESKYGPPCPSCPAPEFLGGPSVFLFPPKPKDTLMISRTPEVTCVVVDVSQEDPEVQFNWYVDGVEVHNAKTKPREEQFNSAYRVVSVLTVLHQDWLNGKEYKCKVSNKGLPSSIEKTISKAKGQPREPQVYTLPPSQEEMTKNQVSLTCLVKGFYPSDIAVEWESNGQPENNYKTTPPVLDSDGSFFLYSRLTVDKSRWQEGNVFSCSVMHEALHNHYTQKSLSLSLGK

SEQ ID NO: 209 - DNA, 1329 bp, Artificial Sequence
  IgG heavy chain 4_IgG4 mutant TA_DNA
gaggtgcagctgttggagtctgggggaggcttggtacagcctggggggtccctgagactctcctgtgcagcctctggattcacctttagcagttatgatatgagctgggtccgccaggctccagggaaggggctggagtgggtctcagcgatctctccgtattcgggtaggatttattacgctgattctgtaaaaggtcggttcaccatctccagagacaattccaagaacacgctgtatctgcaaatgaacagcctgagagccgaggacacggccgtgtattactctgcgagaatggcgcttgatttcgactactggggccagggtacactggtcaccgtgagctcagccagcaccaagggcccttccgtgtttcccctggccccttgctcccggtccacatctgagagcaccgccgccctgggctgtctggtgaaggactacttcccagagcccgtgaccgtgagctggaacagcggcgccctgacaagcggcgtgcacacatttcccgccgtgctgcagagctccggcctgtactccctgtctagcgtggtgacagtgccttcctctagcctgggcaccaagacatatacctgtaacgtggaccacaagccaagcaataccaaggtggataagcgggtggagtctaagtacggccctccttgccctagctgtcctgctccagagtttctgggcggcccttccgtgttcctgtttccacccaaaccaaaggacacactgatgatctctagaacaccagaggtgacctgcgtggtggtggacgtgagccaggaggatcccgaggtgcagttcaactggtacgtggatggcgtggaggtgcacaatgccaagaccaagccaagagaggagcagtttaactctgcctacagggtggtgagcgtgctgaccgtgctgcaccaggattggctcaacggcaaggagtataagtgcaaggtgtccaataagggcctgccctcctctatcgagaagacaatctctaaggctaagggccagccaagagagcctcaggtgtacaccctgcctccaagccaggaggagatgacaaagaaccaggtgtccctgacatgtctggtgaagggcttctatccctccgacatcgccgtggagtgggagtctaatggccagcctgagaacaattacaagaccacaccccctgtgctggactctgatggcagcttctttctgtattccaggctgaccgtggataagtctcggtggcaggagggcaacgtgttcagctgctctgtgatgcacgaagccctgcataatcactatactcagaaaagtctgtcactgtcactgggaaag

SEQ ID NO: 210 - protein, 446 aa, Artificial Sequence
  IgG heavy chain 5_IgG1 mutant TA_amino acid
EVQLLESGGGLVQPGGSLRLSCAASGFTFSSYDMSWVRQAPGKGLEWVSAIGADGGPSYYADSVKGRFTISRDNSKNTLYLQMNSLRAEDTAVYYCARMALDFDYWGQGTLVTVSSASTKGPSVFPLAPSSKSTSGGTAALGCLVKDYFPEPVTVSWNSGALTSGVHTFPAVLQSSGLYSLSSVVTVPSSSLGTQTYICNVNHKPSNTKVDKKVEPKSCDKTHTCPPCPAPELLGGPSVFLFPPKPKDTLMISRTPEVTCVVVDVSHEDPEVKFNWYVDGVEVHNAKTKPREEQYNSAYRVVSVLTVLHQDWLNGKEYKCKVSNKALPAPIEKTISKAKGQPREPQVYTLPPSRDELTKNQVSLTCLVKGFYPSDIAVEWESNGQPENNYKTTPPVLDSDGSFFLYSKLTVDKSRWQQGNVFSCSVMHEALHNHYTQKSLSLSPGK

SEQ ID NO: 211 - DNA, 1338 bp, Artificial Sequence
  IgG heavy chain 5_IgG1 mutant TA_DNA
gaggtgcagctgttggagtctgggggaggcttggtacagcctggggggtccctgagactctcctgtgcagcctctggattcacctttagcagttatgatatgagctgggtccgccaggctccagggaaggggctggagtgggtctcagcgatcggggctgatgggggtccgtcttattacgctgattctgtaaaaggtcggttcaccatctccagagacaattccaagaacacgctgtatctgcaaatgaacagcctgagagccgaggacacggccgtgtattactgtgcgagaatggcgcttgatttcgactactggggccagggtacactggtcaccgtgagctcagcctccaccaagggcccatcggtcttccccctggcaccctcctccaagagcacctctgggggcacagcggccctgggctgcctggtcaaggactacttccccgaaccggtgacggtgtcgtggaactcaggcgccctgaccagcggcgtgcacaccttcccggctgtcctacagtcctcaggactctactccctcagcagcgtggtgaccgtgccctccagcagcttgggcacccagacctacatctgcaacgtgaatcacaagcccagcaacaccaaggtggacaagaaagttgagcccaaatcttgtgacaaaactcacacatgcccaccgtgcccagcacctgaactcctggggggaccgtcagtcttcctcttccccccaaaacccaaggacaccctcatgatctcccggacccctgaggtcacatgcgtggtggtggacgtgagccacgaagaccctgaggtcaagttcaactggtacgtggacggcgtggaggtgcataatgccaagacaaagccgcgggaggagcagtacaacagcgcctaccgtgtggtcagcgtcctcaccgtcctgcaccaggactggctgaatggcaaggagtacaagtgcaaggtctccaacaaagccctcccagcccccatcgagaaaaccatctccaaagccaaagggcagccccgagaaccacaggtgtataccctgcccccatcccgggatgagctgaccaagaaccaggtcagcctgacctgcctggtcaaaggcttctatcccagcgacatcgccgtggagtgggagagcaatgggcagccggagaacaactacaagaccacgcctcccgtgctggactccgacggctccttcttcctctacagcaagctcaccgtggacaagagcaggtggcagcaggggaacgtcttctcatgctccgtgatgcatgaggctctgcacaaccactacacgcagaagagcctctccctgtccccgggtaaa

SEQ ID NO: 212 - protein, 446 aa, Artificial Sequence
  IgG heavy chain 5_IgG1 mutant LALA_amino acid
EVQLLESGGGLVQPGGSLRLSCAASGFTFSSYDMSWVRQAPGKGLEWVSAIGADGGPSYYADSVKGRFTISRDNSKNTLYLQMNSLRAEDTAVYYCARMALDFDYWGQGTLVTVSSASTKGPSVFPLAPSSKSTSGGTAALGCLVKDYFPEPVTVSWNSGALTSGVHTFPAVLQSSGLYSLSSVVTVPSSSLGTQTYICNVNHKPSNTKVDKKVEPKSCDKTHTCPPCPAPEAAGGPSVFLFPPKPKDTLMISRTPEVTCVVVDVSHEDPEVKFNWYVDGVEVHNAKTKPREEQYNSTYRVVSVLTVLHQDWLNGKEYKCKVSNKALPAPIEKTISKAKGQPREPQVYTLPPSRDELTKNQVSLTCLVKGFYPSDIAVEWESNGQPENNYKTTPPVLDSDGSFFLYSKLTVDKSRWQQGNVFSCSVMHEALHNHYTQKSLSLSPGK

SEQ ID NO: 213 - DNA, 1338 bp, Artificial Sequence
  IgG heavy chain 5_IgG1 mutant LALA_DNA
gaggtgcagctgttggagtctgggggaggcttggtacagcctggggggtccctgagactctcctgtgcagcctctggattcacctttagcagttatgatatgagctgggtccgccaggctccagggaaggggctggagtgggtctcagcgatcggggctgatgggggtccgtcttattacgctgattctgtaaaaggtcggttcaccatctccagagacaattccaagaacacgctgtatctgcaaatgaacagcctgagagccgaggacacggccgtgtattactgtgcgagaatggcgcttgatttcgactactggggccagggtacactggtcaccgtgagctcagcctccaccaagggcccatcggtcttccccctggcaccctcctccaagagcacctctgggggcacagcggccctgggctgcctggtcaaggactacttccccgaaccggtgacggtgtcgtggaactcaggcgccctgaccagcggcgtgcacaccttcccggctgtcctacagtcctcaggactctactccctcagcagcgtggtgaccgtgccctccagcagcttgggcacccagacctacatctgcaacgtgaatcacaagcccagcaacaccaaggtggacaagaaagttgagcccaaatcttgtgacaaaactcacacatgcccaccgtgcccagcacctgaagccgccgggggaccgtcagtcttcctcttccccccaaaacccaaggacaccctcatgatctcccggacccctgaggtcacatgcgtggtggtggacgtgagccacgaagaccctgaggtcaagttcaactggtacgtggacggcgtggaggtgcataatgccaagacaaagccgcgggaggagcagtacaacagcacgtaccgtgtggtcagcgtcctcaccgtcctgcaccaggactggctgaatggcaaggagtacaagtgcaaggtctccaacaaagccctcccagcccccatcgagaaaaccatctccaaagccaaagggcagccccgagaaccacaggtgtataccctgcccccatcccgggatgagctgaccaagaaccaggtcagcctgacctgcctggtcaaaggcttctatcccagcgacatcgccgtggagtgggagagcaatgggcagccggagaacaactacaagaccacgcctcccgtgctggactccgacggctccttcttcctctacagcaagctcaccgtggacaagagcaggtggcagcaggggaacgtcttctcatgctccgtgatgcatgaggctctgcacaaccactacacgcagaagagcctctccctgtccccgggtaaa

SEQ ID NO: 214 - protein, 446 aa, Artificial Sequence
  IgG heavy chain 5_IgG1 mutant LALATA_amino acid
EVQLLESGGGLVQPGGSLRLSCAASGFTFSSYDMSWVRQAPGKGLEWVSAIGADGGPSYYADSVKGRFTISRDNSKNTLYLQMNSLRAEDTAVYYCARMALDFDYWGQGTLVTVSSASTKGPSVFPLAPSSKSTSGGTAALGCLVKDYFPEPVTVSWNSGALTSGVHTFPAVLQSSGLYSLSSVVTVPSSSLGTQTYICNVNHKPSNTKVDKKVEPKSCDKTHTCPPCPAPEAAGGPSVFLFPPKPKDTLMISRTPEVTCVVVDVSHEDPEVKFNWYVDGVEVHNAKTKPREEQYNSAYRVVSVLTVLHQDWLNGKEYKCKVSNKALPAPIEKTISKAKGQPREPQVYTLPPSRDELTKNQVSLTCLVKGFYPSDIAVEWESNGQPENNYKTTPPVLDSDGSFFLYSKLTVDKSRWQQGNVFSCSVMHEALHNHYTQKSLSLSPGK

SEQ ID NO: 215 - DNA, 1338 bp, Artificial Sequence
  IgG heavy chain 5_IgG1 mutant LALATA_DNA
gaggtgcagctgttggagtctgggggaggcttggtacagcctggggggtccctgagactctcctgtgcagcctctggattcacctttagcagttatgatatgagctgggtccgccaggctccagggaaggggctggagtgggtctcagcgatcggggctgatgggggtccgtcttattacgctgattctgtaaaaggtcggttcaccatctccagagacaattccaagaacacgctgtatctgcaaatgaacagcctgagagccgaggacacggccgtgtattactgtgcgagaatggcgcttgatttcgactactggggccagggtacactggtcaccgtgagctcagcctccaccaagggcccatcggtcttccccctggcaccctcctccaagagcacctctgggggcacagcggccctgggctgcctggtcaaggactacttccccgaaccggtgacggtgtcgtggaactcaggcgccctgaccagcggcgtgcacaccttcccggctgtcctacagtcctcaggactctactccctcagcagcgtggtgaccgtgccctccagcagcttgggcacccagacctacatctgcaacgtgaatcacaagcccagcaacaccaaggtggacaagaaagttgagcccaaatcttgtgacaaaactcacacatgcccaccgtgcccagcacctgaagccgccgggggaccgtcagtcttcctcttccccccaaaacccaaggacaccctcatgatctcccggacccctgaggtcacatgcgtggtggtggacgtgagccacgaagaccctgaggtcaagttcaactggtacgtggacggcgtggaggtgcataatgccaagacaaagccgcgggaggagcagtacaacagcgcctaccgtgtggtcagcgtcctcaccgtcctgcaccaggactggctgaatggcaaggagtacaagtgcaaggtctccaacaaagccctcccagcccccatcgagaaaaccatctccaaagccaaagggcagccccgagaaccacaggtgtataccctgcccccatcccgggatgagctgaccaagaaccaggtcagcctgacctgcctggtcaaaggcttctatcccagcgacatcgccgtggagtgggagagcaatgggcagccggagaacaactacaagaccacgcctcccgtgctggactccgacggctccttcttcctctacagcaagctcaccgtggacaagagcaggtggcagcaggggaacgtcttctcatgctccgtgatgcatgaggctctgcacaaccactacacgcagaagagcctctccctgtccccgggtaaa

SEQ ID NO: 216 - protein, 446 aa, Artificial Sequence
  IgG heavy chain 5_IgG1 mutant LALAPG_amino acid
EVQLLESGGGLVQPGGSLRLSCAASGFTFSSYDMSWVRQAPGKGLEWVSAIGADGGPSYYADSVKGRFTISRDNSKNTLYLQMNSLRAEDTAVYYCARMALDFDYWGQGTLVTVSSASTKGPSVFPLAPSSKSTSGGTAALGCLVKDYFPEPVTVSWNSGALTSGVHTFPAVLQSSGLYSLSSVVTVPSSSLGTQTYICNVNHKPSNTKVDKKVEPKSCDKTHTCPPCPAPEAAGGPSVFLFPPKPKDTLMISRTPEVTCVVVDVSHEDPEVKFNWYVDGVEVHNAKTKPREEQYNSTYRVVSVLTVLHQDWLNGKEYKCKVSNKALGAPIEKTISKAKGQPREPQVYTLPPSRDELTKNQVSLTCLVKGFYPSDIAVEWESNGQPENNYKTTPPVLDSDGSFFLYSKLTVDKSRWQQGNVFSCSVMHEALHNHYTQKSLSLSPGK

SEQ ID NO: 217 - DNA, 1338 bp, Artificial Sequence
  IgG heavy chain 5_IgG1 mutant LALAPG_DNA
gaggtgcagctgttggagtctgggggaggcttggtacagcctggggggtccctgagactctcctgtgcagcctctggattcacctttagcagttatgatatgagctgggtccgccaggctccagggaaggggctggagtgggtctcagcgatcggggctgatgggggtccgtcttattacgctgattctgtaaaaggtcggttcaccatctccagagacaattccaagaacacgctgtatctgcaaatgaacagcctgagagccgaggacacggccgtgtattactgtgcgagaatggcgcttgatttcgactactggggccagggtacactggtcaccgtgagctcagcctccaccaagggcccatcggtcttccccctggcaccctcctccaagagcacctctgggggcacagcggccctgggctgcctggtcaaggactacttccccgaaccggtgacggtgtcgtggaactcaggcgccctgaccagcggcgtgcacaccttcccggctgtcctacagtcctcaggactctactccctcagcagcgtggtgaccgtgccctccagcagcttgggcacccagacctacatctgcaacgtgaatcacaagcccagcaacaccaaggtggacaagaaagttgagcccaaatcttgtgacaaaactcacacatgcccaccgtgcccagcacctgaagccgccgggggaccgtcagtcttcctcttccccccaaaacccaaggacaccctcatgatctcccggacccctgaggtcacatgcgtggtggtggacgtgagccacgaagaccctgaggtcaagttcaactggtacgtggacggcgtggaggtgcataatgccaagacaaagccgcgggaggagcagtacaacagcacgtaccgtgtggtcagcgtcctcaccgtcctgcaccaggactggctgaatggcaaggagtacaagtgcaaggtctccaacaaagccctcggcgcccccatcgagaaaaccatctccaaagccaaagggcagccccgagaaccacaggtgtataccctgcccccatcccgggatgagctgaccaagaaccaggtcagcctgacctgcctggtcaaaggcttctatcccagcgacatcgccgtggagtgggagagcaatgggcagccggagaacaactacaagaccacgcctcccgtgctggactccgacggctccttcttcctctacagcaagctcaccgtggacaagagcaggtggcagcaggggaacgtcttctcatgctccgtgatgcatgaggctctgcacaaccactacacgcagaagagcctctccctgtccccgggtaaa

SEQ ID NO: 218 - protein, 446 aa, Artificial Sequence
  IgG heavy chain 5_IgG1 mutant LALAPGTA_amino acid
EVQLLESGGGLVQPGGSLRLSCAASGFTFSSYDMSWVRQAPGKGLEWVSAIGADGGPSYYADSVKGRFTISRDNSKNTLYLQMNSLRAEDTAVYYCARMALDFDYWGQGTLVTVSSASTKGPSVFPLAPSSKSTSGGTAALGCLVKDYFPEPVTVSWNSGALTSGVHTFPAVLQSSGLYSLSSVVTVPSSSLGTQTYICNVNHKPSNTKVDKKVEPKSCDKTHTCPPCPAPEAAGGPSVFLFPPKPKDTLMISRTPEVTCVVVDVSHEDPEVKFNWYVDGVEVHNAKTKPREEQYNSAYRVVSVLTVLHQDWLNGKEYKCKVSNKALGAPIEKTISKAKGQPREPQVYTLPPSRDELTKNQVSLTCLVKGFYPSDIAVEWESNGQPENNYKTTPPVLDSDGSFFLYSKLTVDKSRWQQGNVFSCSVMHEALHNHYTQKSLSLSPGK

SEQ ID NO: 219 - DNA, 1338 bp, Artificial Sequence
  IgG heavy chain 5_IgG1 mutant LALAPGTA_DNA
gaggtgcagctgttggagtctgggggaggcttggtacagcctggggggtccctgagactctcctgtgcagcctctggattcacctttagcagttatgatatgagctgggtccgccaggctccagggaaggggctggagtgggtctcagcgatcggggctgatgggggtccgtcttattacgctgattctgtaaaaggtcggttcaccatctccagagacaattccaagaacacgctgtatctgcaaatgaacagcctgagagccgaggacacggccgtgtattactgtgcgagaatggcgcttgatttcgactactggggccagggtacactggtcaccgtgagctcagcctccaccaagggcccatcggtcttccccctggcaccctcctccaagagcacctctgggggcacagcggccctgggctgcctggtcaaggactacttccccgaaccggtgacggtgtcgtggaactcaggcgccctgaccagcggcgtgcacaccttcccggctgtcctacagtcctcaggactctactccctcagcagcgtggtgaccgtgccctccagcagcttgggcacccagacctacatctgcaacgtgaatcacaagcccagcaacaccaaggtggacaagaaagttgagcccaaatcttgtgacaaaactcacacatgcccaccgtgcccagcacctgaagccgccgggggaccgtcagtcttcctcttccccccaaaacccaaggacaccctcatgatctcccggacccctgaggtcacatgcgtggtggtggacgtgagccacgaagaccctgaggtcaagttcaactggtacgtggacggcgtggaggtgcataatgccaagacaaagccgcgggaggagcagtacaacagcgcctaccgtgtggtcagcgtcctcaccgtcctgcaccaggactggctgaatggcaaggagtacaagtgcaaggtctccaacaaagccctcggcgcccccatcgagaaaaccatctccaaagccaaagggcagccccgagaaccacaggtgtataccctgcccccatcccgggatgagctgaccaagaaccaggtcagcctgacctgcctggtcaaaggcttctatcccagcgacatcgccgtggagtgggagagcaatgggcagccggagaacaactacaagaccacgcctcccgtgctggactccgacggctccttcttcctctacagcaagctcaccgtggacaagagcaggtggcagcaggggaacgtcttctcatgctccgtgatgcatgaggctctgcacaaccactacacgcagaagagcctctccctgtccccgggtaaa

SEQ ID NO: 220 - protein, 443 aa, Artificial Sequence
  IgG heavy chain 5_IgG4 wild type_amino acid
EVQLLESGGGLVQPGGSLRLSCAASGFTFSSYDMSWVRQAPGKGLEWVSAIGADGGPSYYADSVKGRFTISRDNSKNTLYLQMNSLRAEDTAVYYCARMALDFDYWGQGTLVTVSSASTKGPSVFPLAPCSRSTSESTAALGCLVKDYFPEPVTVSWNSGALTSGVHTFPAVLQSSGLYSLSSVVTVPSSSLGTKTYTCNVDHKPSNTKVDKRVESKYGPPCPSCPAPEFLGGPSVFLFPPKPKDTLMISRTPEVTCVVVDVSQEDPEVQFNWYVDGVEVHNAKTKPREEQFNSTYRVVSVLTVLHQDWLNGKEYKCKVSNKGLPSSIEKTISKAKGQPREPQVYTLPPSQEEMTKNQVSLTCLVKGFYPSDIAVEWESNGQPENNYKTTPPVLDSDGSFFLYSRLTVDKSRWQEGNVFSCSVMHEALHNHYTQKSLSLSLGK

SEQ ID NO: 221 - DNA, 1329 bp, Artificial Sequence
  IgG heavy chain 5_IgG4 wild type_DNA
gaggtgcagctgttggagtctgggggaggcttggtacagcctggggggtccctgagactctcctgtgcagcctctggattcacctttagcagttatgatatgagctgggtccgccaggctccagggaaggggctggagtgggtctcagcgatcggggctgatgggggtccgtcttattacgctgattctgtaaaaggtcggttcaccatctccagagacaattccaagaacacgctgtatctgcaaatgaacagcctgagagccgaggacacggccgtgtattactgtgcgagaatggcgcttgatttcgactactggggccagggtacactggtcaccgtgagctcagccagcaccaagggcccttccgtgtttcccctggccccttgctcccggtccacatctgagagcaccgccgccctgggctgtctggtgaaggactacttcccagagcccgtgaccgtgagctggaacagcggcgccctgacaagcggcgtgcacacatttcccgccgtgctgcagagctccggcctgtactccctgtctagcgtggtgacagtgccttcctctagcctgggcaccaagacatatacctgtaacgtggaccacaagccaagcaataccaaggtggataagcgggtggagtctaagtacggccctccttgccctagctgtcctgctccagagtttctgggcggcccttccgtgttcctgtttccacccaaaccaaaggacacactgatgatctctagaacaccagaggtgacctgcgtggtggtggacgtgagccaggaggatcccgaggtgcagttcaactggtacgtggatggcgtggaggtgcacaatgccaagaccaagccaagagaggagcagtttaactctacatacagggtggtgagcgtgctgaccgtgctgcaccaggattggctcaacggcaaggagtataagtgcaaggtgtccaataagggcctgccctcctctatcgagaagacaatctctaaggctaagggccagccaagagagcctcaggtgtacaccctgcctccaagccaggaggagatgacaaagaaccaggtgtccctgacatgtctggtgaagggcttctatccctccgacatcgccgtggagtgggagtctaatggccagcctgagaacaattacaagaccacaccccctgtgctggactctgatggcagcttctttctgtattccaggctgaccgtggataagtctcggtggcaggagggcaacgtgttcagctgctctgtgatgcacgaagccctgcataatcactatactcagaaaagtctgtcactgtcactgggaaag

SEQ ID NO: 222 - protein, 443 aa, Artificial Sequence
  IgG heavy chain 5_IgG4 mutant TA_amino acid
EVQLLESGGGLVQPGGSLRLSCAASGFTFSSYDMSWVRQAPGKGLEWVSAIGADGGPSYYADSVKGRFTISRDNSKNTLYLQMNSLRAEDTAVYYCARMALDFDYWGQGTLVTVSSASTKGPSVFPLAPCSRSTSESTAALGCLVKDYFPEPVTVSWNSGALTSGVHTFPAVLQSSGLYSLSSVVTVPSSSLGTKTYTCNVDHKPSNTKVDKRVESKYGPPCPSCPAPEFLGGPSVFLFPPKPKDTLMISRTPEVTCVVVDVSQEDPEVQFNWYVDGVEVHNAKTKPREEQFNSAYRVVSVLTVLHQDWLNGKEYKCKVSNKGLPSSIEKTISKAKGQPREPQVYTLPPSQEEMTKNQVSLTCLVKGFYPSDIAVEWESNGQPENNYKTTPPVLDSDGSFFLYSRLTVDKSRWQEGNVFSCSVMHEALHNHYTQKSLSLSLGK

SEQ ID NO: 223 - DNA, 1329 bp, Artificial Sequence
  IgG heavy chain 5_IgG4 mutant TA_DNA
gaggtgcagctgttggagtctgggggaggcttggtacagcctggggggtccctgagactctcctgtgcagcctctggattcacctttagcagttatgatatgagctgggtccgccaggctccagggaaggggctggagtgggtctcagcgatcggggctgatgggggtccgtcttattacgctgattctgtaaaaggtcggttcaccatctccagagacaattccaagaacacgctgtatctgcaaatgaacagcctgagagccgaggacacggccgtgtattactgtgcgagaatggcgcttgatttcgactactggggccagggtacactggtcaccgtgagctcagccagcaccaagggcccttccgtgtttcccctggccccttgctcccggtccacatctgagagcaccgccgccctgggctgtctggtgaaggactacttcccagagcccgtgaccgtgagctggaacagcggcgccctgacaagcggcgtgcacacatttcccgccgtgctgcagagctccggcctgtactccctgtctagcgtggtgacagtgccttcctctagcctgggcaccaagacatatacctgtaacgtggaccacaagccaagcaataccaaggtggataagcgggtggagtctaagtacggccctccttgccctagctgtcctgctccagagtttctgggcggcccttccgtgttcctgtttccacccaaaccaaaggacacactgatgatctctagaacaccagaggtgacctgcgtggtggtggacgtgagccaggaggatcccgaggtgcagttcaactggtacgtggatggcgtggaggtgcacaatgccaagaccaagccaagagaggagcagtttaactctgcctacagggtggtgagcgtgctgaccgtgctgcaccaggattggctcaacggcaaggagtataagtgcaaggtgtccaataagggcctgccctcctctatcgagaagacaatctctaaggctaagggccagccaagagagcctcaggtgtacaccctgcctccaagccaggaggagatgacaaagaaccaggtgtccctgacatgtctggtgaagggcttctatccctccgacatcgccgtggagtgggagtctaatggccagcctgagaacaattacaagaccacaccccctgtgctggactctgatggcagcttctttctgtattccaggctgaccgtggataagtctcggtggcaggagggcaacgtgttcagctgctctgtgatgcacgaagccctgcataatcactatactcagaaaagtctgtcactgtcactgggaaag

SEQ ID NO: 224 - protein, 446 aa, Artificial Sequence
  IgG heavy chain 6_IgG1 mutant TA_amino acid
EVQLLESGGGLVQPGGSLRLSCAASGFTFSSYDMSWVRQAPGKGLEWVSAISPYSGRIYYADSVKGRFTISRDNSKNTLYLQMNSLRAEDTAVYYCARMALDFDYWGQGTLVTVSSASTKGPSVFPLAPSSKSTSGGTAALGCLVKDYFPEPVTVSWNSGALTSGVHTFPAVLQSSGLYSLSSVVTVPSSSLGTQTYICNVNHKPSNTKVDKKVEPKSCDKTHTCPPCPAPELLGGPSVFLFPPKPKDTLMISRTPEVTCVVVDVSHEDPEVKFNWYVDGVEVHNAKTKPREEQYNSAYRVVSVLTVLHQDWLNGKEYKCKVSNKALPAPIEKTISKAKGQPREPQVYTLPPSRDELTKNQVSLTCLVKGFYPSDIAVEWESNGQPENNYKTTPPVLDSDGSFFLYSKLTVDKSRWQQGNVFSCSVMHEALHNHYTQKSLSLSPGK

SEQ ID NO: 225 - DNA, 1338 bp, Artificial Sequence
  IgG heavy chain 6_IgG1 mutant TA_DNA
gaggtgcagctgttggagtctgggggaggcttggtacagcctggggggtccctgagactctcctgtgcagcctctggattcacctttagcagttatgatatgagctgggtccgccaggctccagggaaggggctggagtgggtctcagcgatctctccgtattcgggtaggatttattacgctgattctgtaaaaggtcggttcaccatctccagagacaattccaagaacacgctgtatctgcaaatgaacagcctgagagccgaggacacggccgtgtattactgtgcgagaatggcgcttgatttcgactactggggccagggtacactggtcaccgtgagctcagcctccaccaagggcccatcggtcttccccctggcaccctcctccaagagcacctctgggggcacagcggccctgggctgcctggtcaaggactacttccccgaaccggtgacggtgtcgtggaactcaggcgccctgaccagcggcgtgcacaccttcccggctgtcctacagtcctcaggactctactccctcagcagcgtggtgaccgtgccctccagcagcttgggcacccagacctacatctgcaacgtgaatcacaagcccagcaacaccaaggtggacaagaaagttgagcccaaatcttgtgacaaaactcacacatgcccaccgtgcccagcacctgaactcctggggggaccgtcagtcttcctcttccccccaaaacccaaggacaccctcatgatctcccggacccctgaggtcacatgcgtggtggtggacgtgagccacgaagaccctgaggtcaagttcaactggtacgtggacggcgtggaggtgcataatgccaagacaaagccgcgggaggagcagtacaacagcgcctaccgtgtggtcagcgtcctcaccgtcctgcaccaggactggctgaatggcaaggagtacaagtgcaaggtctccaacaaagccctcccagcccccatcgagaaaaccatctccaaagccaaagggcagccccgagaaccacaggtgtataccctgcccccatcccgggatgagctgaccaagaaccaggtcagcctgacctgcctggtcaaaggcttctatcccagcgacatcgccgtggagtgggagagcaatgggcagccggagaacaactacaagaccacgcctcccgtgctggactccgacggctccttcttcctctacagcaagctcaccgtggacaagagcaggtggcagcaggggaacgtcttctcatgctccgtgatgcatgaggctctgcacaaccactacacgcagaagagcctctccctgtccccgggtaaa

SEQ ID NO: 226 - protein, 446 aa, Artificial Sequence
  IgG heavy chain 6_IgG1 mutant LALA_amino acid
EVQLLESGGGLVQPGGSLRLSCAASGFTFSSYDMSWVRQAPGKGLEWVSAISPYSGRIYYADSVKGRFTISRDNSKNTLYLQMNSLRAEDTAVYYCARMALDFDYWGQGTLVTVSSASTKGPSVFPLAPSSKSTSGGTAALGCLVKDYFPEPVTVSWNSGALTSGVHTFPAVLQSSGLYSLSSVVTVPSSSLGTQTYICNVNHKPSNTKVDKKVEPKSCDKTHTCPPCPAPEAAGGPSVFLFPPKPKDTLMISRTPEVTCVVVDVSHEDPEVKFNWYVDGVEVHNAKTKPREEQYNSTYRVVSVLTVLHQDWLNGKEYKCKVSNKALPAPIEKTISKAKGQPREPQVYTLPPSRDELTKNQVSLTCLVKGFYPSDIAVEWESNGQPENNYKTTPPVLDSDGSFFLYSKLTVDKSRWQQGNVFSCSVMHEALHNHYTQKSLSLSPGK

SEQ ID NO: 227 - DNA, 1338 bp, Artificial Sequence
  IgG heavy chain 6_IgG1 mutant LALA_DNA
gaggtgcagctgttggagtctgggggaggcttggtacagcctggggggtccctgagactctcctgtgcagcctctggattcacctttagcagttatgatatgagctgggtccgccaggctccagggaaggggctggagtgggtctcagcgatctctccgtattcgggtaggatttattacgctgattctgtaaaaggtcggttcaccatctccagagacaattccaagaacacgctgtatctgcaaatgaacagcctgagagccgaggacacggccgtgtattactgtgcgagaatggcgcttgatttcgactactggggccagggtacactggtcaccgtgagctcagcctccaccaagggcccatcggtcttccccctggcaccctcctccaagagcacctctgggggcacagcggccctgggctgcctggtcaaggactacttccccgaaccggtgacggtgtcgtggaactcaggcgccctgaccagcggcgtgcacaccttcccggctgtcctacagtcctcaggactctactccctcagcagcgtggtgaccgtgccctccagcagcttgggcacccagacctacatctgcaacgtgaatcacaagcccagcaacaccaaggtggacaagaaagttgagcccaaatcttgtgacaaaactcacacatgcccaccgtgcccagcacctgaagccgccgggggaccgtcagtcttcctcttccccccaaaacccaaggacaccctcatgatctcccggacccctgaggtcacatgcgtggtggtggacgtgagccacgaagaccctgaggtcaagttcaactggtacgtggacggcgtggaggtgcataatgccaagacaaagccgcgggaggagcagtacaacagcacgtaccgtgtggtcagcgtcctcaccgtcctgcaccaggactggctgaatggcaaggagtacaagtgcaaggtctccaacaaagccctcccagcccccatcgagaaaaccatctccaaagccaaagggcagccccgagaaccacaggtgtataccctgcccccatcccgggatgagctgaccaagaaccaggtcagcctgacctgcctggtcaaaggcttctatcccagcgacatcgccgtggagtgggagagcaatgggcagccggagaacaactacaagaccacgcctcccgtgctggactccgacggctccttcttcctctacagcaagctcaccgtggacaagagcaggtggcagcaggggaacgtcttctcatgctccgtgatgcatgaggctctgcacaaccactacacgcagaagagcctctccctgtccccgggtaaa

SEQ ID NO: 228 - protein, 446 aa, Artificial Sequence
  IgG heavy chain 6_IgG1 mutant LALATA_amino acid
EVQLLESGGGLVQPGGSLRLSCAASGFTFSSYDMSWVRQAPGKGLEWVSAISPYSGRIYYADSVKGRFTISRDNSKNTLYLQMNSLRAEDTAVYYCARMALDFDYWGQGTLVTVSSASTKGPSVFPLAPSSKSTSGGTAALGCLVKDYFPEPVTVSWNSGALTSGVHTFPAVLQSSGLYSLSSVVTVPSSSLGTQTYICNVNHKPSNTKVDKKVEPKSCDKTHTCPPCPAPEAAGGPSVFLFPPKPKDTLMISRTPEVTCVVVDVSHEDPEVKFNWYVDGVEVHNAKTKPREEQYNSAYRVVSVLTVLHQDWLNGKEYKCKVSNKALPAPIEKTISKAKGQPREPQVYTLPPSRDELTKNQVSLTCLVKGFYPSDIAVEWESNGQPENNYKTTPPVLDSDGSFFLYSKLTVDKSRWQQGNVFSCSVMHEALHNHYTQKSLSLSPGK

SEQ ID NO: 229 - DNA, 1338 bp, Artificial Sequence
  IgG heavy chain 6_IgG1 mutant LALATA_DNA
gaggtgcagctgttggagtctgggggaggcttggtacagcctggggggtccctgagactctcctgtgcagcctctggattcacctttagcagttatgatatgagctgggtccgccaggctccagggaaggggctggagtgggtctcagcgatctctccgtattcgggtaggatttattacgctgattctgtaaaaggtcggttcaccatctccagagacaattccaagaacacgctgtatctgcaaatgaacagcctgagagccgaggacacggccgtgtattactgtgcgagaatggcgcttgatttcgactactggggccagggtacactggtcaccgtgagctcagcctccaccaagggcccatcggtcttccccctggcaccctcctccaagagcacctctgggggcacagcggccctgggctgcctggtcaaggactacttccccgaaccggtgacggtgtcgtggaactcaggcgccctgaccagcggcgtgcacaccttcccggctgtcctacagtcctcaggactctactccctcagcagcgtggtgaccgtgccctccagcagcttgggcacccagacctacatctgcaacgtgaatcacaagcccagcaacaccaaggtggacaagaaagttgagcccaaatcttgtgacaaaactcacacatgcccaccgtgcccagcacctgaagccgccgggggaccgtcagtcttcctcttccccccaaaacccaaggacaccctcatgatctcccggacccctgaggtcacatgcgtggtggtggacgtgagccacgaagaccctgaggtcaagttcaactggtacgtggacggcgtggaggtgcataatgccaagacaaagccgcgggaggagcagtacaacagcgcctaccgtgtggtcagcgtcctcaccgtcctgcaccaggactggctgaatggcaaggagtacaagtgcaaggtctccaacaaagccctcccagcccccatcgagaaaaccatctccaaagccaaagggcagccccgagaaccacaggtgtataccctgcccccatcccgggatgagctgaccaagaaccaggtcagcctgacctgcctggtcaaaggcttctatcccagcgacatcgccgtggagtgggagagcaatgggcagccggagaacaactacaagaccacgcctcccgtgctggactccgacggctccttcttcctctacagcaagctcaccgtggacaagagcaggtggcagcaggggaacgtcttctcatgctccgtgatgcatgaggctctgcacaaccactacacgcagaagagcctctccctgtccccgggtaaa

SEQ ID NO: 230 - protein, 446 aa, Artificial Sequence
  IgG heavy chain 6_IgG1 mutant LALAPG_amino acid
EVQLLESGGGLVQPGGSLRLSCAASGFTFSSYDMSWVRQAPGKGLEWVSAISPYSGRIYYADSVKGRFTISRDNSKNTLYLQMNSLRAEDTAVYYCARMALDFDYWGQGTLVTVSSASTKGPSVFPLAPSSKSTSGGTAALGCLVKDYFPEPVTVSWNSGALTSGVHTFPAVLQSSGLYSLSSVVTVPSSSLGTQTYICNVNHKPSNTKVDKKVEPKSCDKTHTCPPCPAPEAAGGPSVFLFPPKPKDTLMISRTPEVTCVVVDVSHEDPEVKFNWYVDGVEVHNAKTKPREEQYNSTYRVVSVLTVLHQDWLNGKEYKCKVSNKALGAPIEKTISKAKGQPREPQVYTLPPSRDELTKNQVSLTCLVKGFYPSDIAVEWESNGQPENNYKTTPPVLDSDGSFFLYSKLTVDKSRWQQGNVFSCSVMHEALHNHYTQKSLSLSPGK

SEQ ID NO: 231 - DNA, 1338 bp, Artificial Sequence
  IgG heavy chain 6_IgG1 mutant LALAPG_DNA
gaggtgcagctgttggagtctgggggaggcttggtacagcctggggggtccctgagactctcctgtgcagcctctggattcacctttagcagttatgatatgagctgggtccgccaggctccagggaaggggctggagtgggtctcagcgatctctccgtattcgggtaggatttattacgctgattctgtaaaaggtcggttcaccatctccagagacaattccaagaacacgctgtatctgcaaatgaacagcctgagagccgaggacacggccgtgtattactgtgcgagaatggcgcttgatttcgactactggggccagggtacactggtcaccgtgagctcagcctccaccaagggcccatcggtcttccccctggcaccctcctccaagagcacctctgggggcacagcggccctgggctgcctggtcaaggactacttccccgaaccggtgacggtgtcgtggaactcaggcgccctgaccagcggcgtgcacaccttcccggctgtcctacagtcctcaggactctactccctcagcagcgtggtgaccgtgccctccagcagcttgggcacccagacctacatctgcaacgtgaatcacaagcccagcaacaccaaggtggacaagaaagttgagcccaaatcttgtgacaaaactcacacatgcccaccgtgcccagcacctgaagccgccgggggaccgtcagtcttcctcttccccccaaaacccaaggacaccctcatgatctcccggacccctgaggtcacatgcgtggtggtggacgtgagccacgaagaccctgaggtcaagttcaactggtacgtggacggcgtggaggtgcataatgccaagacaaagccgcgggaggagcagtacaacagcacgtaccgtgtggtcagcgtcctcaccgtcctgcaccaggactggctgaatggcaaggagtacaagtgcaaggtctccaacaaagccctcggcgcccccatcgagaaaaccatctccaaagccaaagggcagccccgagaaccacaggtgtataccctgcccccatcccgggatgagctgaccaagaaccaggtcagcctgacctgcctggtcaaaggcttctatcccagcgacatcgccgtggagtgggagagcaatgggcagccggagaacaactacaagaccacgcctcccgtgctggactccgacggctccttcttcctctacagcaagctcaccgtggacaagagcaggtggcagcaggggaacgtcttctcatgctccgtgatgcatgaggctctgcacaaccactacacgcagaagagcctctccctgtccccgggtaaa

SEQ ID NO: 232 - protein, 446 aa, Artificial Sequence
  IgG heavy chain 6_IgG1 mutant LALAPGTA_amino acid
EVQLLESGGGLVQPGGSLRLSCAASGFTFSSYDMSWVRQAPGKGLEWVSAISPYSGRIYYADSVKGRFTISRDNSKNTLYLQMNSLRAEDTAVYYCARMALDFDYWGQGTLVTVSSASTKGPSVFPLAPSSKSTSGGTAALGCLVKDYFPEPVTVSWNSGALTSGVHTFPAVLQSSGLYSLSSVVTVPSSSLGTQTYICNVNHKPSNTKVDKKVEPKSCDKTHTCPPCPAPEAAGGPSVFLFPPKPKDTLMISRTPEVTCVVVDVSHEDPEVKFNWYVDGVEVHNAKTKPREEQYNSAYRVVSVLTVLHQDWLNGKEYKCKVSNKALGAPIEKTISKAKGQPREPQVYTLPPSRDELTKNQVSLTCLVKGFYPSDIAVEWESNGQPENNYKTTPPVLDSDGSFFLYSKLTVDKSRWQQGNVFSCSVMHEALHNHYTQKSLSLSPGK

SEQ ID NO: 233 - DNA, 1338 bp, Artificial Sequence
  IgG heavy chain 6_IgG1 mutant LALAPGTA_DNA
gaggtgcagctgttggagtctgggggaggcttggtacagcctggggggtccctgagactctcctgtgcagcctctggattcacctttagcagttatgatatgagctgggtccgccaggctccagggaaggggctggagtgggtctcagcgatctctccgtattcgggtaggatttattacgctgattctgtaaaaggtcggttcaccatctccagagacaattccaagaacacgctgtatctgcaaatgaacagcctgagagccgaggacacggccgtgtattactgtgcgagaatggcgcttgatttcgactactggggccagggtacactggtcaccgtgagctcagcctccaccaagggcccatcggtcttccccctggcaccctcctccaagagcacctctgggggcacagcggccctgggctgcctggtcaaggactacttccccgaaccggtgacggtgtcgtggaactcaggcgccctgaccagcggcgtgcacaccttcccggctgtcctacagtcctcaggactctactccctcagcagcgtggtgaccgtgccctccagcagcttgggcacccagacctacatctgcaacgtgaatcacaagcccagcaacaccaaggtggacaagaaagttgagcccaaatcttgtgacaaaactcacacatgcccaccgtgcccagcacctgaagccgccgggggaccgtcagtcttcctcttccccccaaaacccaaggacaccctcatgatctcccggacccctgaggtcacatgcgtggtggtggacgtgagccacgaagaccctgaggtcaagttcaactggtacgtggacggcgtggaggtgcataatgccaagacaaagccgcgggaggagcagtacaacagcgcctaccgtgtggtcagcgtcctcaccgtcctgcaccaggactggctgaatggcaaggagtacaagtgcaaggtctccaacaaagccctcggcgcccccatcgagaaaaccatctccaaagccaaagggcagccccgagaaccacaggtgtataccctgcccccatcccgggatgagctgaccaagaaccaggtcagcctgacctgcctggtcaaaggcttctatcccagcgacatcgccgtggagtgggagagcaatgggcagccggagaacaactacaagaccacgcctcccgtgctggactccgacggctccttcttcctctacagcaagctcaccgtggacaagagcaggtggcagcaggggaacgtcttctcatgctccgtgatgcatgaggctctgcacaaccactacacgcagaagagcctctccctgtccccgggtaaa

SEQ ID NO: 234 - protein, 443 aa, Artificial Sequence
  IgG heavy chain 6_IgG4 wild type_amino acid
EVQLLESGGGLVQPGGSLRLSCAASGFTFSSYDMSWVRQAPGKGLEWVSAISPYSGRIYYADSVKGRFTISRDNSKNTLYLQMNSLRAEDTAVYYCARMALDFDYWGQGTLVTVSSASTKGPSVFPLAPCSRSTSESTAALGCLVKDYFPEPVTVSWNSGALTSGVHTFPAVLQSSGLYSLSSVVTVPSSSLGTKTYTCNVDHKPSNTKVDKRVESKYGPPCPSCPAPEFLGGPSVFLFPPKPKDTLMISRTPEVTCVVVDVSQEDPEVQFNWYVDGVEVHNAKTKPREEQFNSTYRVVSVLTVLHQDWLNGKEYKCKVSNKGLPSSIEKTISKAKGQPREPQVYTLPPSQEEMTKNQVSLTCLVKGFYPSDIAVEWESNGQPENNYKTTPPVLDSDGSFFLYSRLTVDKSRWQEGNVFSCSVMHEALHNHYTQKSLSLSLGK

SEQ ID NO: 235 - DNA, 1329 bp, Artificial Sequence
  IgG heavy chain 6_IgG4 wild type_DNA
gaggtgcagctgttggagtctgggggaggcttggtacagcctggggggtccctgagactctcctgtgcagcctctggattcacctttagcagttatgatatgagctgggtccgccaggctccagggaaggggctggagtgggtctcagcgatctctccgtattcgggtaggatttattacgctgattctgtaaaaggtcggttcaccatctccagagacaattccaagaacacgctgtatctgcaaatgaacagcctgagagccgaggacacggccgtgtattactgtgcgagaatggcgcttgatttcgactactggggccagggtacactggtcaccgtgagctcagccagcaccaagggcccttccgtgtttcccctggccccttgctcccggtccacatctgagagcaccgccgccctgggctgtctggtgaaggactacttcccagagcccgtgaccgtgagctggaacagcggcgccctgacaagcggcgtgcacacatttcccgccgtgctgcagagctccggcctgtactccctgtctagcgtggtgacagtgccttcctctagcctgggcaccaagacatatacctgtaacgtggaccacaagccaagcaataccaaggtggataagcgggtggagtctaagtacggccctccttgccctagctgtcctgctccagagtttctgggcggcccttccgtgttcctgtttccacccaaaccaaaggacacactgatgatctctagaacaccagaggtgacctgcgtggtggtggacgtgagccaggaggatcccgaggtgcagttcaactggtacgtggatggcgtggaggtgcacaatgccaagaccaagccaagagaggagcagtttaactctacatacagggtggtgagcgtgctgaccgtgctgcaccaggattggctcaacggcaaggagtataagtgcaaggtgtccaataagggcctgccctcctctatcgagaagacaatctctaaggctaagggccagccaagagagcctcaggtgtacaccctgcctccaagccaggaggagatgacaaagaaccaggtgtccctgacatgtctggtgaagggcttctatccctccgacatcgccgtggagtgggagtctaatggccagcctgagaacaattacaagaccacaccccctgtgctggactctgatggcagcttctttctgtattccaggctgaccgtggataagtctcggtggcaggagggcaacgtgttcagctgctctgtgatgcacgaagccctgcataatcactatactcagaaaagtctgtcactgtcactgggaaag

SEQ ID NO: 236 - protein, 443 aa, Artificial Sequence
  IgG heavy chain 6_IgG4 mutant TA_amino acid
EVQLLESGGGLVQPGGSLRLSCAASGFTFSSYDMSWVRQAPGKGLEWVSAISPYSGRIYYADSVKGRFTISRDNSKNTLYLQMNSLRAEDTAVYYCARMALDFDYWGQGTLVTVSSASTKGPSVFPLAPCSRSTSESTAALGCLVKDYFPEPVTVSWNSGALTSGVHTFPAVLQSSGLYSLSSVVTVPSSSLGTKTYTCNVDHKPSNTKVDKRVESKYGPPCPSCPAPEFLGGPSVFLFPPKPKDTLMISRTPEVTCVVVDVSQEDPEVQFNWYVDGVEVHNAKTKPREEQFNSAYRVVSVLTVLHQDWLNGKEYKCKVSNKGLPSSIEKTISKAKGQPREPQVYTLPPSQEEMTKNQVSLTCLVKGFYPSDIAVEWESNGQPENNYKTTPPVLDSDGSFFLYSRLTVDKSRWQEGNVFSCSVMHEALHNHYTQKSLSLSLGK

SEQ ID NO: 237 - DNA, 1329 bp, Artificial Sequence
  IgG heavy chain 6_IgG4 mutant TA_DNA
gaggtgcagctgttggagtctgggggaggcttggtacagcctggggggtccctgagactctcctgtgcagcctctggattcacctttagcagttatgatatgagctgggtccgccaggctccagggaaggggctggagtgggtctcagcgatctctccgtattcgggtaggatttattacgctgattctgtaaaaggtcggttcaccatctccagagacaattccaagaacacgctgtatctgcaaatgaacagcctgagagccgaggacacggccgtgtattactgtgcgagaatggcgcttgatttcgactactggggccagggtacactggtcaccgtgagctcagccagcaccaagggcccttccgtgtttcccctggccccttgctcccggtccacatctgagagcaccgccgccctgggctgtctggtgaaggactacttcccagagcccgtgaccgtgagctggaacagcggcgccctgacaagcggcgtgcacacatttcccgccgtgctgcagagctccggcctgtactccctgtctagcgtggtgacagtgccttcctctagcctgggcaccaagacatatacctgtaacgtggaccacaagccaagcaataccaaggtggataagcgggtggagtctaagtacggccctccttgccctagctgtcctgctccagagtttctgggcggcccttccgtgttcctgtttccacccaaaccaaaggacacactgatgatctctagaacaccagaggtgacctgcgtggtggtggacgtgagccaggaggatcccgaggtgcagttcaactggtacgtggatggcgtggaggtgcacaatgccaagaccaagccaagagaggagcagtttaactctgcctacagggtggtgagcgtgctgaccgtgctgcaccaggattggctcaacggcaaggagtataagtgcaaggtgtccaataagggcctgccctcctctatcgagaagacaatctctaaggctaagggccagccaagagagcctcaggtgtacaccctgcctccaagccaggaggagatgacaaagaaccaggtgtccctgacatgtctggtgaagggcttctatccctccgacatcgccgtggagtgggagtctaatggccagcctgagaacaattacaagaccacaccccctgtgctggactctgatggcagcttctttctgtattccaggctgaccgtggataagtctcggtggcaggagggcaacgtgttcagctgctctgtgatgcacgaagccctgcataatcactatactcagaaaagtctgtcactgtcactgggaaag

SEQ ID NO: 238 - protein, 446 aa, Artificial Sequence
  IgG heavy chain 7_IgG1 mutant TA_amino acid
EVQLLESGGGLVQPGGSLRLSCAASGFTFSSYDMSWVRQAPGKGLEWVSAISPYSGRIYYADSVKGRFTISRDNSKNTLYLQMNSLRAEDTAVYYCARLALDFDYWGQGTLVTVSSASTKGPSVFPLAPSSKSTSGGTAALGCLVKDYFPEPVTVSWNSGALTSGVHTFPAVLQSSGLYSLSSVVTVPSSSLGTQTYICNVNHKPSNTKVDKKVEPKSCDKTHTCPPCPAPELLGGPSVFLFPPKPKDTLMISRTPEVTCVVVDVSHEDPEVKFNWYVDGVEVHNAKTKPREEQYNSAYRVVSVLTVLHQDWLNGKEYKCKVSNKALPAPIEKTISKAKGQPREPQVYTLPPSRDELTKNQVSLTCLVKGFYPSDIAVEWESNGQPENNYKTTPPVLDSDGSFFLYSKLTVDKSRWQQGNVFSCSVMHEALHNHYTQKSLSLSPGK

SEQ ID NO: 239 - DNA, 1338 bp, Artificial Sequence
  IgG heavy chain 7_IgG1 mutant TA_DNA
gaggtgcagctgttggagtctgggggaggcttggtacagcctggggggtccctgagactctcctgtgcagcctctggattcacctttagcagttatgatatgagctgggtccgccaggctccagggaaggggctggagtgggtctcagcgatctctccgtattcgggtaggatttattacgctgattctgtaaaaggtcggttcaccatctccagagacaattccaagaacacgctgtatctgcaaatgaacagcctgagagccgaggacacggccgtgtattactgtgcgagactggcgcttgatttcgactactggggccagggtacactggtcaccgtgagctcagcctccaccaagggcccatcggtcttccccctggcaccctcctccaagagcacctctgggggcacagcggccctgggctgcctggtcaaggactacttccccgaaccggtgacggtgtcgtggaactcaggcgccctgaccagcggcgtgcacaccttcccggctgtcctacagtcctcaggactctactccctcagcagcgtggtgaccgtgccctccagcagcttgggcacccagacctacatctgcaacgtgaatcacaagcccagcaacaccaaggtggacaagaaagttgagcccaaatcttgtgacaaaactcacacatgcccaccgtgcccagcacctgaactcctggggggaccgtcagtcttcctcttccccccaaaacccaaggacaccctcatgatctcccggacccctgaggtcacatgcgtggtggtggacgtgagccacgaagaccctgaggtcaagttcaactggtacgtggacggcgtggaggtgcataatgccaagacaaagccgcgggaggagcagtacaacagcgcctaccgtgtggtcagcgtcctcaccgtcctgcaccaggactggctgaatggcaaggagtacaagtgcaaggtctccaacaaagccctcccagcccccatcgagaaaaccatctccaaagccaaagggcagccccgagaaccacaggtgtataccctgcccccatcccgggatgagctgaccaagaaccaggtcagcctgacctgcctggtcaaaggcttctatcccagcgacatcgccgtggagtgggagagcaatgggcagccggagaacaactacaagaccacgcctcccgtgctggactccgacggctccttcttcctctacagcaagctcaccgtggacaagagcaggtggcagcaggggaacgtcttctcatgctccgtgatgcatgaggctctgcacaaccactacacgcagaagagcctctccctgtccccgggtaaa

SEQ ID NO: 240 - protein, 446 aa, Artificial Sequence
  IgG heavy chain 7_IgG1 mutant LALA_amino acid
EVQLLESGGGLVQPGGSLRLSCAASGFTFSSYDMSWVRQAPGKGLEWVSAISPYSGRIYYADSVKGRFTISRDNSKNTLYLQMNSLRAEDTAVYYCARLALDFDYWGQGTLVTVSSASTKGPSVFPLAPSSKSTSGGTAALGCLVKDYFPEPVTVSWNSGALTSGVHTFPAVLQSSGLYSLSSVVTVPSSSLGTQTYICNVNHKPSNTKVDKKVEPKSCDKTHTCPPCPAPEAAGGPSVFLFPPKPKDTLMISRTPEVTCVVVDVSHEDPEVKFNWYVDGVEVHNAKTKPREEQYNSTYRVVSVLTVLHQDWLNGKEYKCKVSNKALPAPIEKTISKAKGQPREPQVYTLPPSRDELTKNQVSLTCLVKGFYPSDIAVEWESNGQPENNYKTTPPVLDSDGSFFLYSKLTVDKSRWQQGNVFSCSVMHEALHNHYTQKSLSLSPGK

SEQ ID NO: 241 - DNA, 1338 bp, Artificial Sequence
  IgG heavy chain 7_IgG1 mutant LALA_DNA
gaggtgcagctgttggagtctgggggaggcttggtacagcctggggggtccctgagactctcctgtgcagcctctggattcacctttagcagttatgatatgagctgggtccgccaggctccagggaaggggctggagtgggtctcagcgatctctccgtattcgggtaggatttattacgctgattctgtaaaaggtcggttcaccatctccagagacaattccaagaacacgctgtatctgcaaatgaacagcctgagagccgaggacacggccgtgtattactgtgcgagactggcgcttgatttcgactactggggccagggtacactggtcaccgtgagctcagcctccaccaagggcccatcggtcttccccctggcaccctcctccaagagcacctctgggggcacagcggccctgggctgcctggtcaaggactacttccccgaaccggtgacggtgtcgtggaactcaggcgccctgaccagcggcgtgcacaccttcccggctgtcctacagtcctcaggactctactccctcagcagcgtggtgaccgtgccctccagcagcttgggcacccagacctacatctgcaacgtgaatcacaagcccagcaacaccaaggtggacaagaaagttgagcccaaatcttgtgacaaaactcacacatgcccaccgtgcccagcacctgaagccgccgggggaccgtcagtcttcctcttccccccaaaacccaaggacaccctcatgatctcccggacccctgaggtcacatgcgtggtggtggacgtgagccacgaagaccctgaggtcaagttcaactggtacgtggacggcgtggaggtgcataatgccaagacaaagccgcgggaggagcagtacaacagcacgtaccgtgtggtcagcgtcctcaccgtcctgcaccaggactggctgaatggcaaggagtacaagtgcaaggtctccaacaaagccctcccagcccccatcgagaaaaccatctccaaagccaaagggcagccccgagaaccacaggtgtataccctgcccccatcccgggatgagctgaccaagaaccaggtcagcctgacctgcctggtcaaaggcttctatcccagcgacatcgccgtggagtgggagagcaatgggcagccggagaacaactacaagaccacgcctcccgtgctggactccgacggctccttcttcctctacagcaagctcaccgtggacaagagcaggtggcagcaggggaacgtcttctcatgctccgtgatgcatgaggctctgcacaaccactacacgcagaagagcctctccctgtccccgggtaaa

SEQ ID NO: 242 - protein, 446 aa, Artificial Sequence
  IgG heavy chain 7_IgG1 mutant LALATA_amino acid
EVQLLESGGGLVQPGGSLRLSCAASGFTFSSYDMSWVRQAPGKGLEWVSAISPYSGRIYYADSVKGRFTISRDNSKNTLYLQMNSLRAEDTAVYYCARLALDFDYWGQGTLVTVSSASTKGPSVFPLAPSSKSTSGGTAALGCLVKDYFPEPVTVSWNSGALTSGVHTFPAVLQSSGLYSLSSVVTVPSSSLGTQTYICNVNHKPSNTKVDKKVEPKSCDKTHTCPPCPAPEAAGGPSVFLFPPKPKDTLMISRTPEVTCVVVDVSHEDPEVKFNWYVDGVEVHNAKTKPREEQYNSAYRVVSVLTVLHQDWLNGKEYKCKVSNKALPAPIEKTISKAKGQPREPQVYTLPPSRDELTKNQVSLTCLVKGFYPSDIAVEWESNGQPENNYKTTPPVLDSDGSFFLYSKLTVDKSRWQQGNVFSCSVMHEALHNHYTQKSLSLSPGK

SEQ ID NO: 243 - DNA, 1338 bp, Artificial Sequence
  IgG heavy chain 7_IgG1 mutant LALATA_DNA
gaggtgcagctgttggagtctgggggaggcttggtacagcctggggggtccctgagactctcctgtgcagcctctggattcacctttagcagttatgatatgagctgggtccgccaggctccagggaaggggctggagtgggtctcagcgatctctccgtattcgggtaggatttattacgctgattctgtaaaaggtcggttcaccatctccagagacaattccaagaacacgctgtatctgcaaatgaacagcctgagagccgaggacacggccgtgtattactgtgcgagactggcgcttgatttcgactactggggccagggtacactggtcaccgtgagctcagcctccaccaagggcccatcggtcttccccctggcaccctcctccaagagcacctctgggggcacagcggccctgggctgcctggtcaaggactacttccccgaaccggtgacggtgtcgtggaactcaggcgccctgaccagcggcgtgcacaccttcccggctgtcctacagtcctcaggactctactccctcagcagcgtggtgaccgtgccctccagcagcttgggcacccagacctacatctgcaacgtgaatcacaagcccagcaacaccaaggtggacaagaaagttgagcccaaatcttgtgacaaaactcacacatgcccaccgtgcccagcacctgaagccgccgggggaccgtcagtcttcctcttccccccaaaacccaaggacaccctcatgatctcccggacccctgaggtcacatgcgtggtggtggacgtgagccacgaagaccctgaggtcaagttcaactggtacgtggacggcgtggaggtgcataatgccaagacaaagccgcgggaggagcagtacaacagcgcctaccgtgtggtcagcgtcctcaccgtcctgcaccaggactggctgaatggcaaggagtacaagtgcaaggtctccaacaaagccctcccagcccccatcgagaaaaccatctccaaagccaaagggcagccccgagaaccacaggtgtataccctgcccccatcccgggatgagctgaccaagaaccaggtcagcctgacctgcctggtcaaaggcttctatcccagcgacatcgccgtggagtgggagagcaatgggcagccggagaacaactacaagaccacgcctcccgtgctggactccgacggctccttcttcctctacagcaagctcaccgtggacaagagcaggtggcagcaggggaacgtcttctcatgctccgtgatgcatgaggctctgcacaaccactacacgcagaagagcctctccctgtccccgggtaaa

SEQ ID NO: 244 - protein, 446 aa, Artificial Sequence
  IgG heavy chain 7_IgG1 mutant LALAPG_amino acid
EVQLLESGGGLVQPGGSLRLSCAASGFTFSSYDMSWVRQAPGKGLEWVSAISPYSGRIYYADSVKGRFTISRDNSKNTLYLQMNSLRAEDTAVYYCARLALDFDYWGQGTLVTVSSASTKGPSVFPLAPSSKSTSGGTAALGCLVKDYFPEPVTVSWNSGALTSGVHTFPAVLQSSGLYSLSSVVTVPSSSLGTQTYICNVNHKPSNTKVDKKVEPKSCDKTHTCPPCPAPEAAGGPSVFLFPPKPKDTLMISRTPEVTCVVVDVSHEDPEVKFNWYVDGVEVHNAKTKPREEQYNSTYRVVSVLTVLHQDWLNGKEYKCKVSNKALGAPIEKTISKAKGQPREPQVYTLPPSRDELTKNQVSLTCLVKGFYPSDIAVEWESNGQPENNYKTTPPVLDSDGSFFLYSKLTVDKSRWQQGNVFSCSVMHEALHNHYTQKSLSLSPGK

SEQ ID NO: 245 - DNA, 1338 bp, Artificial Sequence
  IgG heavy chain 7_IgG1 mutant LALAPG_DNA
gaggtgcagctgttggagtctgggggaggcttggtacagcctggggggtccctgagactctcctgtgcagcctctggattcacctttagcagttatgatatgagctgggtccgccaggctccagggaaggggctggagtgggtctcagcgatctctccgtattcgggtaggatttattacgctgattctgtaaaaggtcggttcaccatctccagagacaattccaagaacacgctgtatctgcaaatgaacagcctgagagccgaggacacggccgtgtattactgtgcgagactggcgcttgatttcgactactggggccagggtacactggtcaccgtgagctcagcctccaccaagggcccatcggtcttccccctggcaccctcctccaagagcacctctgggggcacagcggccctgggctgcctggtcaaggactacttccccgaaccggtgacggtgtcgtggaactcaggcgccctgaccagcggcgtgcacaccttcccggctgtcctacagtcctcaggactctactccctcagcagcgtggtgaccgtgccctccagcagcttgggcacccagacctacatctgcaacgtgaatcacaagcccagcaacaccaaggtggacaagaaagttgagcccaaatcttgtgacaaaactcacacatgcccaccgtgcccagcacctgaagccgccgggggaccgtcagtcttcctcttccccccaaaacccaaggacaccctcatgatctcccggacccctgaggtcacatgcgtggtggtggacgtgagccacgaagaccctgaggtcaagttcaactggtacgtggacggcgtggaggtgcataatgccaagacaaagccgcgggaggagcagtacaacagcacgtaccgtgtggtcagcgtcctcaccgtcctgcaccaggactggctgaatggcaaggagtacaagtgcaaggtctccaacaaagccctcggcgcccccatcgagaaaaccatctccaaagccaaagggcagccccgagaaccacaggtgtataccctgcccccatcccgggatgagctgaccaagaaccaggtcagcctgacctgcctggtcaaaggcttctatcccagcgacatcgccgtggagtgggagagcaatgggcagccggagaacaactacaagaccacgcctcccgtgctggactccgacggctccttcttcctctacagcaagctcaccgtggacaagagcaggtggcagcaggggaacgtcttctcatgctccgtgatgcatgaggctctgcacaaccactacacgcagaagagcctctccctgtccccgggtaaa

SEQ ID NO: 246 - protein, 446 aa, Artificial Sequence
  IgG heavy chain 7_IgG1 mutant LALAPGTA_amino acid
EVQLLESGGGLVQPGGSLRLSCAASGFTFSSYDMSWVRQAPGKGLEWVSAISPYSGRIYYADSVKGRFTISRDNSKNTLYLQMNSLRAEDTAVYYCARLALDFDYWGQGTLVTVSSASTKGPSVFPLAPSSKSTSGGTAALGCLVKDYFPEPVTVSWNSGALTSGVHTFPAVLQSSGLYSLSSVVTVPSSSLGTQTYICNVNHKPSNTKVDKKVEPKSCDKTHTCPPCPAPEAAGGPSVFLFPPKPKDTLMISRTPEVTCVVVDVSHEDPEVKFNWYVDGVEVHNAKTKPREEQYNSAYRVVSVLTVLHQDWLNGKEYKCKVSNKALGAPIEKTISKAKGQPREPQVYTLPPSRDELTKNQVSLTCLVKGFYPSDIAVEWESNGQPENNYKTTPPVLDSDGSFFLYSKLTVDKSRWQQGNVFSCSVMHEALHNHYTQKSLSLSPGK

SEQ ID NO: 247 - DNA, 1338 bp, Artificial Sequence
  IgG heavy chain 7_IgG1 mutant LALAPGTA_DNA
gaggtgcagctgttggagtctgggggaggcttggtacagcctggggggtccctgagactctcctgtgcagcctctggattcacctttagcagttatgatatgagctgggtccgccaggctccagggaaggggctggagtgggtctcagcgatctctccgtattcgggtaggatttattacgctgattctgtaaaaggtcggttcaccatctccagagacaattccaagaacacgctgtatctgcaaatgaacagcctgagagccgaggacacggccgtgtattactgtgcgagactggcgcttgatttcgactactggggccagggtacactggtcaccgtgagctcagcctccaccaagggcccatcggtcttccccctggcaccctcctccaagagcacctctgggggcacagcggccctgggctgcctggtcaaggactacttccccgaaccggtgacggtgtcgtggaactcaggcgccctgaccagcggcgtgcacaccttcccggctgtcctacagtcctcaggactctactccctcagcagcgtggtgaccgtgccctccagcagcttgggcacccagacctacatctgcaacgtgaatcacaagcccagcaacaccaaggtggacaagaaagttgagcccaaatcttgtgacaaaactcacacatgcccaccgtgcccagcacctgaagccgccgggggaccgtcagtcttcctcttccccccaaaacccaaggacaccctcatgatctcccggacccctgaggtcacatgcgtggtggtggacgtgagccacgaagaccctgaggtcaagttcaactggtacgtggacggcgtggaggtgcataatgccaagacaaagccgcgggaggagcagtacaacagcgcctaccgtgtggtcagcgtcctcaccgtcctgcaccaggactggctgaatggcaaggagtacaagtgcaaggtctccaacaaagccctcggcgcccccatcgagaaaaccatctccaaagccaaagggcagccccgagaaccacaggtgtataccctgcccccatcccgggatgagctgaccaagaaccaggtcagcctgacctgcctggtcaaaggcttctatcccagcgacatcgccgtggagtgggagagcaatgggcagccggagaacaactacaagaccacgcctcccgtgctggactccgacggctccttcttcctctacagcaagctcaccgtggacaagagcaggtggcagcaggggaacgtcttctcatgctccgtgatgcatgaggctctgcacaaccactacacgcagaagagcctctccctgtccccgggtaaa

SEQ ID NO: 248 - protein, 443 aa, Artificial Sequence
  IgG heavy chain 7_IgG4 wild type_amino acid
EVQLLESGGGLVQPGGSLRLSCAASGFTFSSYDMSWVRQAPGKGLEWVSAISPYSGRIYYADSVKGRFTISRDNSKNTLYLQMNSLRAEDTAVYYCARLALDFDYWGQGTLVTVSSASTKGPSVFPLAPCSRSTSESTAALGCLVKDYFPEPVTVSWNSGALTSGVHTFPAVLQSSGLYSLSSVVTVPSSSLGTKTYTCNVDHKPSNTKVDKRVESKYGPPCPSCPAPEFLGGPSVFLFPPKPKDTLMISRTPEVTCVVVDVSQEDPEVQFNWYVDGVEVHNAKTKPREEQFNSTYRVVSVLTVLHQDWLNGKEYKCKVSNKGLPSSIEKTISKAKGQPREPQVYTLPPSQEEMTKNQVSLTCLVKGFYPSDIAVEWESNGQPENNYKTTPPVLDSDGSFFLYSRLTVDKSRWQEGNVFSCSVMHEALHNHYTQKSLSLSLGK

SEQ ID NO: 249 - DNA, 1329 bp, Artificial Sequence
  IgG heavy chain 7_IgG4 wild type_DNA
gaggtgcagctgttggagtctgggggaggcttggtacagcctggggggtccctgagactctcctgtgcagcctctggattcacctttagcagttatgatatgagctgggtccgccaggctccagggaaggggctggagtgggtctcagcgatctctccgtattcgggtaggatttattacgctgattctgtaaaaggtcggttcaccatctccagagacaattccaagaacacgctgtatctgcaaatgaacagcctgagagccgaggacacggccgtgtattactgtgcgagactggcgcttgatttcgactactggggccagggtacactggtcaccgtgagctcagccagcaccaagggcccttccgtgtttcccctggccccttgctcccggtccacatctgagagcaccgccgccctgggctgtctggtgaaggactacttcccagagcccgtgaccgtgagctggaacagcggcgccctgacaagcggcgtgcacacatttcccgccgtgctgcagagctccggcctgtactccctgtctagcgtggtgacagtgccttcctctagcctgggcaccaagacatatacctgtaacgtggaccacaagccaagcaataccaaggtggataagcgggtggagtctaagtacggccctccttgccctagctgtcctgctccagagtttctgggcggcccttccgtgttcctgtttccacccaaaccaaaggacacactgatgatctctagaacaccagaggtgacctgcgtggtggtggacgtgagccaggaggatcccgaggtgcagttcaactggtacgtggatggcgtggaggtgcacaatgccaagaccaagccaagagaggagcagtttaactctacatacagggtggtgagcgtgctgaccgtgctgcaccaggattggctcaacggcaaggagtataagtgcaaggtgtccaataagggcctgccctcctctatcgagaagacaatctctaaggctaagggccagccaagagagcctcaggtgtacaccctgcctccaagccaggaggagatgacaaagaaccaggtgtccctgacatgtctggtgaagggcttctatccctccgacatcgccgtggagtgggagtctaatggccagcctgagaacaattacaagaccacaccccctgtgctggactctgatggcagcttctttctgtattccaggctgaccgtggataagtctcggtggcaggagggcaacgtgttcagctgctctgtgatgcacgaagccctgcataatcactatactcagaaaagtctgtcactgtcactgggaaag

SEQ ID NO: 250 - protein, 443 aa, Artificial Sequence
  IgG heavy chain 7_IgG4 mutant TA_amino acid
EVQLLESGGGLVQPGGSLRLSCAASGFTFSSYDMSWVRQAPGKGLEWVSAISPYSGRIYYADSVKGRFTISRDNSKNTLYLQMNSLRAEDTAVYYCARLALDFDYWGQGTLVTVSSASTKGPSVFPLAPCSRSTSESTAALGCLVKDYFPEPVTVSWNSGALTSGVHTFPAVLQSSGLYSLSSVVTVPSSSLGTKTYTCNVDHKPSNTKVDKRVESKYGPPCPSCPAPEFLGGPSVFLFPPKPKDTLMISRTPEVTCVVVDVSQEDPEVQFNWYVDGVEVHNAKTKPREEQFNSAYRVVSVLTVLHQDWLNGKEYKCKVSNKGLPSSIEKTISKAKGQPREPQVYTLPPSQEEMTKNQVSLTCLVKGFYPSDIAVEWESNGQPENNYKTTPPVLDSDGSFFLYSRLTVDKSRWQEGNVFSCSVMHEALHNHYTQKSLSLSLGK

SEQ ID NO: 251 - DNA, 1329 bp, Artificial Sequence
  IgG heavy chain 7_IgG4 mutant TA_DNA
gaggtgcagctgttggagtctgggggaggcttggtacagcctggggggtccctgagactctcctgtgcagcctctggattcacctttagcagttatgatatgagctgggtccgccaggctccagggaaggggctggagtgggtctcagcgatctctccgtattcgggtaggatttattacgctgattctgtaaaaggtcggttcaccatctccagagacaattccaagaacacgctgtatctgcaaatgaacagcctgagagccgaggacacggccgtgtattactgtgcgagactggcgcttgatttcgactactggggccagggtacactggtcaccgtgagctcagccagcaccaagggcccttccgtgtttcccctggccccttgctcccggtccacatctgagagcaccgccgccctgggctgtctggtgaaggactacttcccagagcccgtgaccgtgagctggaacagcggcgccctgacaagcggcgtgcacacatttcccgccgtgctgcagagctccggcctgtactccctgtctagcgtggtgacagtgccttcctctagcctgggcaccaagacatatacctgtaacgtggaccacaagccaagcaataccaaggtggataagcgggtggagtctaagtacggccctccttgccctagctgtcctgctccagagtttctgggcggcccttccgtgttcctgtttccacccaaaccaaaggacacactgatgatctctagaacaccagaggtgacctgcgtggtggtggacgtgagccaggaggatcccgaggtgcagttcaactggtacgtggatggcgtggaggtgcacaatgccaagaccaagccaagagaggagcagtttaactctgcctacagggtggtgagcgtgctgaccgtgctgcaccaggattggctcaacggcaaggagtataagtgcaaggtgtccaataagggcctgccctcctctatcgagaagacaatctctaaggctaagggccagccaagagagcctcaggtgtacaccctgcctccaagccaggaggagatgacaaagaaccaggtgtccctgacatgtctggtgaagggcttctatccctccgacatcgccgtggagtgggagtctaatggccagcctgagaacaattacaagaccacaccccctgtgctggactctgatggcagcttctttctgtattccaggctgaccgtggataagtctcggtggcaggagggcaacgtgttcagctgctctgtgatgcacgaagccctgcataatcactatactcagaaaagtctgtcactgtcactgggaaag